European Patent Specification EP 4 105 341 B1, published May 1, 2024. Title: A primer for Next Generation Sequencer and a method for producing the same, a DNA library obtained through the use of a primer for Next Generation Sequencer and a method for producing the same, and a DNA analyzing method using a DNA library. Applicant: TOYOTA JIDOSHA KABUSHKI KAISHA. The sequence listing filed with the application follows.

SEQUENCE LISTING (1515 sequences)

SEQ ID NO: 1 - DNA, 24 bp, Artificial
  synthetic
caagcagaagacggcatacgagat

SEQ ID NO: 2 - DNA, 34 bp, Artificial
  synthetic
gtctcgtgggctcggagatgtgtataagagacag

SEQ ID NO: 3 - DNA, 13 bp, Artificial
  synthetic
taagagacagaaa

SEQ ID NO: 4 - DNA, 13 bp, Artificial
  synthetic
taagagacagaac

SEQ ID NO: 5 - DNA, 13 bp, Artificial
  synthetic
taagagacagaag

SEQ ID NO: 6 - DNA, 13 bp, Artificial
  synthetic
taagagacagaat

SEQ ID NO: 7 - DNA, 13 bp, Artificial
  synthetic
taagagacagaca

SEQ ID NO: 8 - DNA, 13 bp, Artificial
  synthetic
taagagacagacc

SEQ ID NO: 9 - DNA, 13 bp, Artificial
  synthetic
taagagacagacg

SEQ ID NO: 10 - DNA, 13 bp, Artificial
  synthetic
taagagacagact

SEQ ID NO: 11 - DNA, 13 bp, Artificial
  synthetic
taagagacagaga

SEQ ID NO: 12 - DNA, 13 bp, Artificial
  synthetic
taagagacagagc

SEQ ID NO: 13 - DNA, 13 bp, Artificial
  synthetic
taagagacagagg

SEQ ID NO: 14 - DNA, 13 bp, Artificial
  synthetic
taagagacagagt

SEQ ID NO: 15 - DNA, 13 bp, Artificial
  synthetic
taagagacagata

SEQ ID NO: 16 - DNA, 13 bp, Artificial
  synthetic
taagagacagatc

SEQ ID NO: 17 - DNA, 13 bp, Artificial
  synthetic
taagagacagatg

SEQ ID NO: 18 - DNA, 13 bp, Artificial
  synthetic
taagagacagatt

SEQ ID NO: 19 - DNA, 13 bp, Artificial
  synthetic
taagagacagcaa

SEQ ID NO: 20 - DNA, 13 bp, Artificial
  synthetic
taagagacagcac

SEQ ID NO: 21 - DNA, 13 bp, Artificial
  synthetic
taagagacagcag

SEQ ID NO: 22 - DNA, 13 bp, Artificial
  synthetic
taagagacagcat

SEQ ID NO: 23 - DNA, 13 bp, Artificial
  synthetic
taagagacagcca

SEQ ID NO: 24 - DNA, 13 bp, Artificial
  synthetic
taagagacagccc

SEQ ID NO: 25 - DNA, 13 bp, Artificial
  synthetic
taagagacagccg

SEQ ID NO: 26 - DNA, 13 bp, Artificial
  synthetic
taagagacagcct

SEQ ID NO: 27 - DNA, 13 bp, Artificial
  synthetic
taagagacagcga

SEQ ID NO: 28 - DNA, 13 bp, Artificial
  synthetic
taagagacagcgc

SEQ ID NO: 29 - DNA, 13 bp, Artificial
  synthetic
taagagacagcgg

SEQ ID NO: 30 - DNA, 13 bp, Artificial
  synthetic
taagagacagcgt

SEQ ID NO: 31 - DNA, 13 bp, Artificial
  synthetic
taagagacagcta

SEQ ID NO: 32 - DNA, 13 bp, Artificial
  synthetic
taagagacagctc

SEQ ID NO: 33 - DNA, 13 bp, Artificial
  synthetic
taagagacagctg

SEQ ID NO: 34 - DNA, 13 bp, Artificial
  synthetic
taagagacagctt

SEQ ID NO: 35 - DNA, 13 bp, Artificial
  synthetic
taagagacaggaa

SEQ ID NO: 36 - DNA, 13 bp, Artificial
  synthetic
taagagacaggac

SEQ ID NO: 37 - DNA, 13 bp, Artificial
  synthetic
taagagacaggag

SEQ ID NO: 38 - DNA, 13 bp, Artificial
  synthetic
taagagacaggat

SEQ ID NO: 39 - DNA, 13 bp, Artificial
  synthetic
taagagacaggca

SEQ ID NO: 40 - DNA, 13 bp, Artificial
  synthetic
taagagacaggcc

SEQ ID NO: 41 - DNA, 13 bp, Artificial
  synthetic
taagagacaggcg

SEQ ID NO: 42 - DNA, 13 bp, Artificial
  synthetic
taagagacaggct

SEQ ID NO: 43 - DNA, 13 bp, Artificial
  synthetic
taagagacaggga

SEQ ID NO: 44 - DNA, 13 bp, Artificial
  synthetic
taagagacagggc

SEQ ID NO: 45 - DNA, 13 bp, Artificial
  synthetic
taagagacagggg

SEQ ID NO: 46 - DNA, 13 bp, Artificial
  synthetic
taagagacagggt

SEQ ID NO: 47 - DNA, 13 bp, Artificial
  synthetic
taagagacaggta

SEQ ID NO: 48 - DNA, 13 bp, Artificial
  synthetic
taagagacaggtc

SEQ ID NO: 49 - DNA, 13 bp, Artificial
  synthetic
taagagacaggtg

SEQ ID NO: 50 - DNA, 13 bp, Artificial
  synthetic
taagagacaggtt

SEQ ID NO: 51 - DNA, 13 bp, Artificial
  synthetic
taagagacagtaa

SEQ ID NO: 52 - DNA, 13 bp, Artificial
  synthetic
taagagacagtac

SEQ ID NO: 53 - DNA, 13 bp, Artificial
  synthetic
taagagacagtag

SEQ ID NO: 54 - DNA, 13 bp, Artificial
  synthetic
taagagacagtat

SEQ ID NO: 55 - DNA, 13 bp, Artificial
  synthetic
taagagacagtca

SEQ ID NO: 56 - DNA, 13 bp, Artificial
  synthetic
taagagacagtcc

SEQ ID NO: 57 - DNA, 13 bp, Artificial
  synthetic
taagagacagtcg

SEQ ID NO: 58 - DNA, 13 bp, Artificial
  synthetic
taagagacagtct

SEQ ID NO: 59 - DNA, 13 bp, Artificial
  synthetic
taagagacagtga

SEQ ID NO: 60 - DNA, 13 bp, Artificial
  synthetic
taagagacagtgg

SEQ ID NO: 61 - DNA, 13 bp, Artificial
  synthetic
taagagacagtgt

SEQ ID NO: 62 - DNA, 13 bp, Artificial
  synthetic
taagagacagtta

SEQ ID NO: 63 - DNA, 13 bp, Artificial
  synthetic
taagagacagttc

SEQ ID NO: 64 - DNA, 13 bp, Artificial
  synthetic
taagagacagttg

SEQ ID NO: 65 - DNA, 13 bp, Artificial
  synthetic
taagagacagttt

SEQ ID NO: 66 - DNA, 70 bp, Artificial
  synthetic
  misc_feature (30)..(37): n is a, c, g, or t
aatgatacggcgaccaccgagatctacacnnnnnnnntcgtcggcagcgtcagatgtgtataagagacag

SEQ ID NO: 67 - DNA, 66 bp, Artificial
  synthetic
  misc_feature (25)..(32): n is a, c, g, or t
caagcagaagacggcatacgagatnnnnnnnngtctcgtgggctcggagatgtgtataagagacag

SEQ ID NO: 68 - DNA, 66 bp, Artificial
  synthetic
caagcagaagacggcatacgagatgtgatactgtctcgtgggctcggagatgtgtataagagacag

SEQ ID NO: 69 - DNA, 66 bp, Artificial
  synthetic
caagcagaagacggcatacgagatgagcgcgtgtctcgtgggctcggagatgtgtataagagacag

SEQ ID NO: 70 - DNA, 66 bp, Artificial
  synthetic
caagcagaagacggcatacgagatgcatctcggtctcgtgggctcggagatgtgtataagagacag

SEQ ID NO: 71 - DNA, 66 bp, Artificial
  synthetic
caagcagaagacggcatacgagattcgtacgtgtctcgtgggctcggagatgtgtataagagacag

SEQ ID NO: 72 - DNA, 66 bp, Artificial
  synthetic
caagcagaagacggcatacgagattatcgtcggtctcgtgggctcggagatgtgtataagagacag

SEQ ID NO: 73 - DNA, 66 bp, Artificial
  synthetic
caagcagaagacggcatacgagattgcacagagtctcgtgggctcggagatgtgtataagagacag

SEQ ID NO: 74 - DNA, 66 bp, Artificial
  synthetic
caagcagaagacggcatacgagatcgtatgacgtctcgtgggctcggagatgtgtataagagacag

SEQ ID NO: 75 - DNA, 66 bp, Artificial
  synthetic
caagcagaagacggcatacgagattcgatctcgtctcgtgggctcggagatgtgtataagagacag

SEQ ID NO: 76 - DNA, 66 bp, Artificial
  synthetic
caagcagaagacggcatacgagatatatgacagtctcgtgggctcggagatgtgtataagagacag

SEQ ID NO: 77 - DNA, 66 bp, Artificial
  synthetic
caagcagaagacggcatacgagatgctatcgtgtctcgtgggctcggagatgtgtataagagacag

SEQ ID NO: 78 - DNA, 66 bp, Artificial
  synthetic
caagcagaagacggcatacgagatctgtgtgtgtctcgtgggctcggagatgtgtataagagacag

SEQ ID NO: 79 - DNA, 66 bp, Artificial
  synthetic
caagcagaagacggcatacgagattatactgcgtctcgtgggctcggagatgtgtataagagacag

SEQ ID NO: 80 - DNA, 66 bp, Artificial
  synthetic
caagcagaagacggcatacgagatactgtcgtgtctcgtgggctcggagatgtgtataagagacag

SEQ ID NO: 81 - DNA, 66 bp, Artificial
  synthetic
caagcagaagacggcatacgagatgagctatagtctcgtgggctcggagatgtgtataagagacag

SEQ ID NO: 82 - DNA, 66 bp, Artificial
  synthetic
caagcagaagacggcatacgagattgtgtcgtgtctcgtgggctcggagatgtgtataagagacag

SEQ ID NO: 83 - DNA, 66 bp, Artificial
  synthetic
caagcagaagacggcatacgagatgtgactatgtctcgtgggctcggagatgtgtataagagacag

SEQ ID NO: 84 - DNA, 66 bp, Artificial
  synthetic
caagcagaagacggcatacgagattatacagtgtctcgtgggctcggagatgtgtataagagacag

SEQ ID NO: 85 - DNA, 66 bp, Artificial
  synthetic
caagcagaagacggcatacgagatatgagcgagtctcgtgggctcggagatgtgtataagagacag

SEQ ID NO: 86 - DNA, 66 bp, Artificial
  synthetic
caagcagaagacggcatacgagatagatcagagtctcgtgggctcggagatgtgtataagagacag

SEQ ID NO: 87 - DNA, 66 bp, Artificial
  synthetic
caagcagaagacggcatacgagatagtctgcagtctcgtgggctcggagatgtgtataagagacag

SEQ ID NO: 88 - DNA, 66 bp, Artificial
  synthetic
caagcagaagacggcatacgagatcgctgtgagtctcgtgggctcggagatgtgtataagagacag

SEQ ID NO: 89 - DNA, 66 bp, Artificial
  synthetic
caagcagaagacggcatacgagatgtctatgtgtctcgtgggctcggagatgtgtataagagacag

SEQ ID NO: 90 - DNA, 66 bp, Artificial
  synthetic
caagcagaagacggcatacgagatctgatgtggtctcgtgggctcggagatgtgtataagagacag

SEQ ID NO: 91 - DNA, 66 bp, Artificial
  synthetic
caagcagaagacggcatacgagatcgcactatgtctcgtgggctcggagatgtgtataagagacag

SEQ ID NO: 92 - DNA, 66 bp, Artificial
  synthetic
caagcagaagacggcatacgagatagtgtgcggtctcgtgggctcggagatgtgtataagagacag

SEQ ID NO: 93 - DNA, 66 bp, Artificial
  synthetic
caagcagaagacggcatacgagatcgtatcgcgtctcgtgggctcggagatgtgtataagagacag

SEQ ID NO: 94 - DNA, 66 bp, Artificial
  synthetic
caagcagaagacggcatacgagatgcactctagtctcgtgggctcggagatgtgtataagagacag

SEQ ID NO: 95 - DNA, 66 bp, Artificial
  synthetic
caagcagaagacggcatacgagattacgacacgtctcgtgggctcggagatgtgtataagagacag

SEQ ID NO: 96 - DNA, 66 bp, Artificial
  synthetic
caagcagaagacggcatacgagattctgctcagtctcgtgggctcggagatgtgtataagagacag

SEQ ID NO: 97 - DNA, 66 bp, Artificial
  synthetic
caagcagaagacggcatacgagattcgtgactgtctcgtgggctcggagatgtgtataagagacag

SEQ ID NO: 98 - DNA, 66 bp, Artificial
  synthetic
caagcagaagacggcatacgagattgtatctagtctcgtgggctcggagatgtgtataagagacag

SEQ ID NO: 99 - DNA, 66 bp, Artificial
  synthetic
caagcagaagacggcatacgagatgtgcgtacgtctcgtgggctcggagatgtgtataagagacag

SEQ ID NO: 100 - DNA, 66 bp, Artificial
  synthetic
caagcagaagacggcatacgagatcactactcgtctcgtgggctcggagatgtgtataagagacag

SEQ ID NO: 101 - DNA, 66 bp, Artificial
  synthetic
caagcagaagacggcatacgagattgagcgtcgtctcgtgggctcggagatgtgtataagagacag

SEQ ID NO: 102 - DNA, 66 bp, Artificial
  synthetic
caagcagaagacggcatacgagattgacgtctgtctcgtgggctcggagatgtgtataagagacag

SEQ ID NO: 103 - DNA, 66 bp, Artificial
  synthetic
caagcagaagacggcatacgagatacagtgaggtctcgtgggctcggagatgtgtataagagacag

SEQ ID NO: 104 - DNA, 66 bp, Artificial
  synthetic
caagcagaagacggcatacgagatgactctcagtctcgtgggctcggagatgtgtataagagacag

SEQ ID NO: 105 - DNA, 66 bp, Artificial
  synthetic
caagcagaagacggcatacgagatagcgcgctgtctcgtgggctcggagatgtgtataagagacag

SEQ ID NO: 106 - DNA, 66 bp, Artificial
  synthetic
caagcagaagacggcatacgagatctgtagaggtctcgtgggctcggagatgtgtataagagacag

SEQ ID NO: 107 - DNA, 66 bp, Artificial
  synthetic
caagcagaagacggcatacgagatatgcgatagtctcgtgggctcggagatgtgtataagagacag

SEQ ID NO: 108 - DNA, 66 bp, Artificial
  synthetic
caagcagaagacggcatacgagatgagacatggtctcgtgggctcggagatgtgtataagagacag

SEQ ID NO: 109 - DNA, 66 bp, Artificial
  synthetic
caagcagaagacggcatacgagatgtcatgtggtctcgtgggctcggagatgtgtataagagacag

SEQ ID NO: 110 - DNA, 66 bp, Artificial
  synthetic
caagcagaagacggcatacgagattcatgatagtctcgtgggctcggagatgtgtataagagacag

SEQ ID NO: 111 - DNA, 66 bp, Artificial
  synthetic
caagcagaagacggcatacgagatgtcatctcgtctcgtgggctcggagatgtgtataagagacag

SEQ ID NO: 112 - DNA, 66 bp, Artificial
  synthetic
caagcagaagacggcatacgagatagtgtcgcgtctcgtgggctcggagatgtgtataagagacag

SEQ ID NO: 113 - DNA, 66 bp, Artificial
  synthetic
caagcagaagacggcatacgagatgctgacgtgtctcgtgggctcggagatgtgtataagagacag

SEQ ID NO: 114 - DNA, 66 bp, Artificial
  synthetic
caagcagaagacggcatacgagatgatcagctgtctcgtgggctcggagatgtgtataagagacag

SEQ ID NO: 115 - DNA, 66 bp, Artificial
  synthetic
caagcagaagacggcatacgagattatctctagtctcgtgggctcggagatgtgtataagagacag

SEQ ID NO: 116 - DNA, 66 bp, Artificial
  synthetic
caagcagaagacggcatacgagatgcagagctgtctcgtgggctcggagatgtgtataagagacag

SEQ ID NO: 117 - DNA, 66 bp, Artificial
  synthetic
caagcagaagacggcatacgagattgctagcggtctcgtgggctcggagatgtgtataagagacag

SEQ ID NO: 118 - DNA, 66 bp, Artificial
  synthetic
caagcagaagacggcatacgagatcgtatctcgtctcgtgggctcggagatgtgtataagagacag

SEQ ID NO: 119 - DNA, 66 bp, Artificial
  synthetic
caagcagaagacggcatacgagatctgatatagtctcgtgggctcggagatgtgtataagagacag

SEQ ID NO: 120 - DNA, 66 bp, Artificial
  synthetic
caagcagaagacggcatacgagattagtgcgcgtctcgtgggctcggagatgtgtataagagacag

SEQ ID NO: 121 - DNA, 66 bp, Artificial
  synthetic
caagcagaagacggcatacgagatctagtgcagtctcgtgggctcggagatgtgtataagagacag

SEQ ID NO: 122 - DNA, 66 bp, Artificial
  synthetic
caagcagaagacggcatacgagatgatgtcacgtctcgtgggctcggagatgtgtataagagacag

SEQ ID NO: 123 - DNA, 66 bp, Artificial
  synthetic
caagcagaagacggcatacgagatatagagcggtctcgtgggctcggagatgtgtataagagacag

SEQ ID NO: 124 - DNA, 66 bp, Artificial
  synthetic
caagcagaagacggcatacgagatagacatatgtctcgtgggctcggagatgtgtataagagacag

SEQ ID NO: 125 - DNA, 66 bp, Artificial
  synthetic
caagcagaagacggcatacgagatcgatcatggtctcgtgggctcggagatgtgtataagagacag

SEQ ID NO: 126 - DNA, 66 bp, Artificial
  synthetic
caagcagaagacggcatacgagatacatagcggtctcgtgggctcggagatgtgtataagagacag

SEQ ID NO: 127 - DNA, 66 bp, Artificial
  synthetic
caagcagaagacggcatacgagatatcgacacgtctcgtgggctcggagatgtgtataagagacag

SEQ ID NO: 128 - DNA, 66 bp, Artificial
  synthetic
caagcagaagacggcatacgagattacacacggtctcgtgggctcggagatgtgtataagagacag

SEQ ID NO: 129 - DNA, 66 bp, Artificial
  synthetic
caagcagaagacggcatacgagattacgcatggtctcgtgggctcggagatgtgtataagagacag

SEQ ID NO: 130 - DNA, 66 bp, Artificial
  synthetic
caagcagaagacggcatacgagatcgtgagtggtctcgtgggctcggagatgtgtataagagacag

SEQ ID NO: 131 - DNA, 66 bp, Artificial
  synthetic
caagcagaagacggcatacgagatgtctgcatgtctcgtgggctcggagatgtgtataagagacag

SEQ ID NO: 132 - DNA, 66 bp, Artificial
  synthetic
caagcagaagacggcatacgagatgcatatgagtctcgtgggctcggagatgtgtataagagacag

SEQ ID NO: 133 - DNA, 66 bp, Artificial
  synthetic
caagcagaagacggcatacgagattgctctctgtctcgtgggctcggagatgtgtataagagacag

SEQ ID NO: 134 - DNA, 66 bp, Artificial
  synthetic
caagcagaagacggcatacgagatgacacatggtctcgtgggctcggagatgtgtataagagacag

SEQ ID NO: 135 - DNA, 66 bp, Artificial
  synthetic
caagcagaagacggcatacgagatctgagcaggtctcgtgggctcggagatgtgtataagagacag

SEQ ID NO: 136 - DNA, 66 bp, Artificial
  synthetic
caagcagaagacggcatacgagatgacatgcggtctcgtgggctcggagatgtgtataagagacag

SEQ ID NO: 137 - DNA, 66 bp, Artificial
  synthetic
caagcagaagacggcatacgagattctgacgagtctcgtgggctcggagatgtgtataagagacag

SEQ ID NO: 138 - DNA, 66 bp, Artificial
  synthetic
caagcagaagacggcatacgagattacagtgtgtctcgtgggctcggagatgtgtataagagacag

SEQ ID NO: 139 - DNA, 66 bp, Artificial
  synthetic
caagcagaagacggcatacgagatgatcgcaggtctcgtgggctcggagatgtgtataagagacag

SEQ ID NO: 140 - DNA, 66 bp, Artificial
  synthetic
caagcagaagacggcatacgagatacatgacggtctcgtgggctcggagatgtgtataagagacag

SEQ ID NO: 141 - DNA, 66 bp, Artificial
  synthetic
caagcagaagacggcatacgagatctagatgagtctcgtgggctcggagatgtgtataagagacag

SEQ ID NO: 142 - DNA, 66 bp, Artificial
  synthetic
caagcagaagacggcatacgagatgcgtctaggtctcgtgggctcggagatgtgtataagagacag

SEQ ID NO: 143 - DNA, 66 bp, Artificial
  synthetic
caagcagaagacggcatacgagatactcgtgcgtctcgtgggctcggagatgtgtataagagacag

SEQ ID NO: 144 - DNA, 66 bp, Artificial
  synthetic
caagcagaagacggcatacgagattcacgctggtctcgtgggctcggagatgtgtataagagacag

SEQ ID NO: 145 - DNA, 66 bp, Artificial
  synthetic
caagcagaagacggcatacgagatctagatctgtctcgtgggctcggagatgtgtataagagacag

SEQ ID NO: 146 - DNA, 66 bp, Artificial
  synthetic
caagcagaagacggcatacgagatcgatagcagtctcgtgggctcggagatgtgtataagagacag

SEQ ID NO: 147 - DNA, 66 bp, Artificial
  synthetic
caagcagaagacggcatacgagatatcgtactgtctcgtgggctcggagatgtgtataagagacag

SEQ ID NO: 148 - DNA, 66 bp, Artificial
  synthetic
caagcagaagacggcatacgagattcatgtacgtctcgtgggctcggagatgtgtataagagacag

SEQ ID NO: 149 - DNA, 66 bp, Artificial
  synthetic
caagcagaagacggcatacgagattagtgacggtctcgtgggctcggagatgtgtataagagacag

SEQ ID NO: 150 - DNA, 66 bp, Artificial
  synthetic
caagcagaagacggcatacgagatcacgataggtctcgtgggctcggagatgtgtataagagacag

SEQ ID NO: 151 - DNA, 66 bp, Artificial
  synthetic
caagcagaagacggcatacgagatacacactggtctcgtgggctcggagatgtgtataagagacag

SEQ ID NO: 152 - DNA, 66 bp, Artificial
  synthetic
caagcagaagacggcatacgagatcgtctagcgtctcgtgggctcggagatgtgtataagagacag

SEQ ID NO: 153 - DNA, 66 bp, Artificial
  synthetic
caagcagaagacggcatacgagattagctagcgtctcgtgggctcggagatgtgtataagagacag

SEQ ID NO: 154 - DNA, 66 bp, Artificial
  synthetic
caagcagaagacggcatacgagattcgacgtcgtctcgtgggctcggagatgtgtataagagacag

SEQ ID NO: 155 - DNA, 66 bp, Artificial
  synthetic
caagcagaagacggcatacgagatagcatcacgtctcgtgggctcggagatgtgtataagagacag

SEQ ID NO: 156 - DNA, 66 bp, Artificial
  synthetic
caagcagaagacggcatacgagatcgagacgcgtctcgtgggctcggagatgtgtataagagacag

SEQ ID NO: 157 - DNA, 66 bp, Artificial
  synthetic
caagcagaagacggcatacgagatcgcgagcagtctcgtgggctcggagatgtgtataagagacag

SEQ ID NO: 158 - DNA, 66 bp, Artificial
  synthetic
caagcagaagacggcatacgagattagtcgtagtctcgtgggctcggagatgtgtataagagacag

SEQ ID NO: 159 - DNA, 66 bp, Artificial
  synthetic
caagcagaagacggcatacgagatcgtagtatgtctcgtgggctcggagatgtgtataagagacag

SEQ ID NO: 160 - DNA, 66 bp, Artificial
  synthetic
caagcagaagacggcatacgagattcacgtacgtctcgtgggctcggagatgtgtataagagacag

SEQ ID NO: 161 - DNA, 66 bp, Artificial
  synthetic
caagcagaagacggcatacgagatgcatcgcggtctcgtgggctcggagatgtgtataagagacag

SEQ ID NO: 162 - DNA, 66 bp, Artificial
  synthetic
caagcagaagacggcatacgagatatcatgtcgtctcgtgggctcggagatgtgtataagagacag

SEQ ID NO: 163 - DNA, 66 bp, Artificial
  synthetic
caagcagaagacggcatacgagatctatgcatgtctcgtgggctcggagatgtgtataagagacag

SEQ ID NO: 164 - DNA, 70 bp, Artificial
  synthetic
aatgatacggcgaccaccgagatctacacctgctcgttcgtcggcagcgtcagatgtgtataagagacag

SEQ ID NO: 165 - DNA, 70 bp, Artificial
  synthetic
aatgatacggcgaccaccgagatctacactgcgacgatcgtcggcagcgtcagatgtgtataagagacag

SEQ ID NO: 166 - DNA, 70 bp, Artificial
  synthetic
aatgatacggcgaccaccgagatctacaccacatgcttcgtcggcagcgtcagatgtgtataagagacag

SEQ ID NO: 167 - DNA, 70 bp, Artificial
  synthetic
aatgatacggcgaccaccgagatctacacatactcattcgtcggcagcgtcagatgtgtataagagacag

SEQ ID NO: 168 - DNA, 70 bp, Artificial
  synthetic
aatgatacggcgaccaccgagatctacacgatgcacgtcgtcggcagcgtcagatgtgtataagagacag

SEQ ID NO: 169 - DNA, 70 bp, Artificial
  synthetic
aatgatacggcgaccaccgagatctacacgtagtgcttcgtcggcagcgtcagatgtgtataagagacag

SEQ ID NO: 170 - DNA, 70 bp, Artificial
  synthetic
aatgatacggcgaccaccgagatctacacatgatagttcgtcggcagcgtcagatgtgtataagagacag

SEQ ID NO: 171 - DNA, 70 bp, Artificial
  synthetic
aatgatacggcgaccaccgagatctacacctcgctagtcgtcggcagcgtcagatgtgtataagagacag

SEQ ID NO: 172 - DNA, 70 bp, Artificial
  synthetic
aatgatacggcgaccaccgagatctacacgctgagagtcgtcggcagcgtcagatgtgtataagagacag

SEQ ID NO: 173 - DNA, 70 bp, Artificial
  synthetic
aatgatacggcgaccaccgagatctacacagcacgagtcgtcggcagcgtcagatgtgtataagagacag

SEQ ID NO: 174 - DNA, 70 bp, Artificial
  synthetic
aatgatacggcgaccaccgagatctacactgtcagagtcgtcggcagcgtcagatgtgtataagagacag

SEQ ID NO: 175 - DNA, 70 bp, Artificial
  synthetic
aatgatacggcgaccaccgagatctacacgcgcagtatcgtcggcagcgtcagatgtgtataagagacag

SEQ ID NO: 176 - DNA, 70 bp, Artificial
  synthetic
aatgatacggcgaccaccgagatctacaccatcagcgtcgtcggcagcgtcagatgtgtataagagacag

SEQ ID NO: 177 - DNA, 70 bp, Artificial
  synthetic
aatgatacggcgaccaccgagatctacactacgagcatcgtcggcagcgtcagatgtgtataagagacag

SEQ ID NO: 178 - DNA, 70 bp, Artificial
  synthetic
aatgatacggcgaccaccgagatctacacagcagacttcgtcggcagcgtcagatgtgtataagagacag

SEQ ID NO: 179 - DNA, 70 bp, Artificial
  synthetic
aatgatacggcgaccaccgagatctacaccagtacattcgtcggcagcgtcagatgtgtataagagacag

SEQ ID NO: 180 - DNA, 70 bp, Artificial
  synthetic
aatgatacggcgaccaccgagatctacacgagtatgatcgtcggcagcgtcagatgtgtataagagacag

SEQ ID NO: 181 - DNA, 70 bp, Artificial
  synthetic
aatgatacggcgaccaccgagatctacactatcacattcgtcggcagcgtcagatgtgtataagagacag

SEQ ID NO: 182 - DNA, 70 bp, Artificial
  synthetic
aatgatacggcgaccaccgagatctacaccacagtcatcgtcggcagcgtcagatgtgtataagagacag

SEQ ID NO: 183 - DNA, 70 bp, Artificial
  synthetic
aatgatacggcgaccaccgagatctacactgcagctatcgtcggcagcgtcagatgtgtataagagacag

SEQ ID NO: 184 - DNA, 70 bp, Artificial
  synthetic
aatgatacggcgaccaccgagatctacacgcgagcagtcgtcggcagcgtcagatgtgtataagagacag

SEQ ID NO: 185 - DNA, 70 bp, Artificial
  synthetic
aatgatacggcgaccaccgagatctacacgacagcgttcgtcggcagcgtcagatgtgtataagagacag

SEQ ID NO: 186 - DNA, 70 bp, Artificial
  synthetic
aatgatacggcgaccaccgagatctacacagctcgagtcgtcggcagcgtcagatgtgtataagagacag

SEQ ID NO: 187 - DNA, 70 bp, Artificial
  synthetic
aatgatacggcgaccaccgagatctacactagatcattcgtcggcagcgtcagatgtgtataagagacag

SEQ ID NO: 188 - DNA, 70 bp, Artificial
  synthetic
aatgatacggcgaccaccgagatctacaccgcagtgatcgtcggcagcgtcagatgtgtataagagacag

SEQ ID NO: 189 - DNA, 70 bp, Artificial
  synthetic
aatgatacggcgaccaccgagatctacaccgtactgatcgtcggcagcgtcagatgtgtataagagacag

SEQ ID NO: 190 - DNA, 70 bp, Artificial
  synthetic
aatgatacggcgaccaccgagatctacactcagatgttcgtcggcagcgtcagatgtgtataagagacag

SEQ ID NO: 191 - DNA, 70 bp, Artificial
  synthetic
aatgatacggcgaccaccgagatctacacctctctgatcgtcggcagcgtcagatgtgtataagagacag

SEQ ID NO: 192 - DNA, 70 bp, Artificial
  synthetic
aatgatacggcgaccaccgagatctacactcagcatatcgtcggcagcgtcagatgtgtataagagacag

SEQ ID NO: 193 - DNA, 70 bp, Artificial
  synthetic
aatgatacggcgaccaccgagatctacaccatacagatcgtcggcagcgtcagatgtgtataagagacag

SEQ ID NO: 194 - DNA, 70 bp, Artificial
  synthetic
aatgatacggcgaccaccgagatctacaccgagacgatcgtcggcagcgtcagatgtgtataagagacag

SEQ ID NO: 195 - DNA, 70 bp, Artificial
  synthetic
aatgatacggcgaccaccgagatctacacctcgacagtcgtcggcagcgtcagatgtgtataagagacag

SEQ ID NO: 196 - DNA, 70 bp, Artificial
  synthetic
aatgatacggcgaccaccgagatctacacgtagatgatcgtcggcagcgtcagatgtgtataagagacag

SEQ ID NO: 197 - DNA, 70 bp, Artificial
  synthetic
aatgatacggcgaccaccgagatctacaccatctcagtcgtcggcagcgtcagatgtgtataagagacag

SEQ ID NO: 198 - DNA, 70 bp, Artificial
  synthetic
aatgatacggcgaccaccgagatctacactgagctcatcgtcggcagcgtcagatgtgtataagagacag

SEQ ID NO: 199 - DNA, 70 bp, Artificial
  synthetic
aatgatacggcgaccaccgagatctacactagagcgttcgtcggcagcgtcagatgtgtataagagacag

SEQ ID NO: 200 - DNA, 70 bp, Artificial
  synthetic
aatgatacggcgaccaccgagatctacacagatagcatcgtcggcagcgtcagatgtgtataagagacag

SEQ ID NO: 201 - DNA, 70 bp, Artificial
  synthetic
aatgatacggcgaccaccgagatctacacagactgagtcgtcggcagcgtcagatgtgtataagagacag

SEQ ID NO: 202 - DNA, 70 bp, Artificial
  synthetic
aatgatacggcgaccaccgagatctacacgctacatatcgtcggcagcgtcagatgtgtataagagacag

SEQ ID NO: 203 - DNA, 70 bp, Artificial
  synthetic
aatgatacggcgaccaccgagatctacacatagctattcgtcggcagcgtcagatgtgtataagagacag

SEQ ID NO: 204 - DNA, 70 bp, Artificial
  synthetic
aatgatacggcgaccaccgagatctacacatcgagtatcgtcggcagcgtcagatgtgtataagagacag

SEQ ID NO: 205 - DNA, 70 bp, Artificial
  synthetic
aatgatacggcgaccaccgagatctacacgatgtgattcgtcggcagcgtcagatgtgtataagagacag

SEQ ID NO: 206 - DNA, 70 bp, Artificial
  synthetic
aatgatacggcgaccaccgagatctacacgatcagtatcgtcggcagcgtcagatgtgtataagagacag

SEQ ID NO: 207 - DNA, 70 bp, Artificial
  synthetic
aatgatacggcgaccaccgagatctacactatgtacttcgtcggcagcgtcagatgtgtataagagacag

SEQ ID NO: 208 - DNA, 70 bp, Artificial
  synthetic
aatgatacggcgaccaccgagatctacactcactgcatcgtcggcagcgtcagatgtgtataagagacag

SEQ ID NO: 209 - DNA, 70 bp, Artificial
  synthetic
aatgatacggcgaccaccgagatctacacacacatattcgtcggcagcgtcagatgtgtataagagacag

SEQ ID NO: 210 - DNA, 70 bp, Artificial
  synthetic
aatgatacggcgaccaccgagatctacacctctctagtcgtcggcagcgtcagatgtgtataagagacag

SEQ ID NO: 211 - DNA, 70 bp, Artificial
  synthetic
aatgatacggcgaccaccgagatctacacgtgagtgttcgtcggcagcgtcagatgtgtataagagacag

SEQ ID NO: 212 - DNA, 70 bp, Artificial
  synthetic
aatgatacggcgaccaccgagatctacaccatcgatgtcgtcggcagcgtcagatgtgtataagagacag

SEQ ID NO: 213 - DNA, 70 bp, Artificial
  synthetic
aatgatacggcgaccaccgagatctacacgatgcacttcgtcggcagcgtcagatgtgtataagagacag

SEQ ID NO: 214 - DNA, 70 bp, Artificial
  synthetic
aatgatacggcgaccaccgagatctacaccgtactcgtcgtcggcagcgtcagatgtgtataagagacag

SEQ ID NO: 215 - DNA, 70 bp, Artificial
  synthetic
aatgatacggcgaccaccgagatctacactgagtgcatcgtcggcagcgtcagatgtgtataagagacag

SEQ ID NO: 216 - DNA, 70 bp, Artificial
  synthetic
aatgatacggcgaccaccgagatctacaccgcgatgatcgtcggcagcgtcagatgtgtataagagacag

SEQ ID NO: 217 - DNA, 70 bp, Artificial
  synthetic
aatgatacggcgaccaccgagatctacactgatcgcatcgtcggcagcgtcagatgtgtataagagacag

SEQ ID NO: 218 - DNA, 70 bp, Artificial
  synthetic
aatgatacggcgaccaccgagatctacaccgcgactatcgtcggcagcgtcagatgtgtataagagacag

SEQ ID NO: 219 - DNA, 70 bp, Artificial
  synthetic
aatgatacggcgaccaccgagatctacacatacgcattcgtcggcagcgtcagatgtgtataagagacag

SEQ ID NO: 220 - DNA, 70 bp, Artificial
  synthetic
aatgatacggcgaccaccgagatctacaccgagcgcttcgtcggcagcgtcagatgtgtataagagacag

SEQ ID NO: 221 - DNA, 70 bp, Artificial
  synthetic
aatgatacggcgaccaccgagatctacacactacgattcgtcggcagcgtcagatgtgtataagagacag

SEQ ID NO: 222 - DNA, 70 bp, Artificial
  synthetic
aatgatacggcgaccaccgagatctacactgcagcagtcgtcggcagcgtcagatgtgtataagagacag

SEQ ID NO: 223 - DNA, 70 bp, Artificial
  synthetic
aatgatacggcgaccaccgagatctacacagtactcgtcgtcggcagcgtcagatgtgtataagagacag

SEQ ID NO: 224 - DNA, 70 bp, Artificial
  synthetic
aatgatacggcgaccaccgagatctacacctgagtgttcgtcggcagcgtcagatgtgtataagagacag

SEQ ID NO: 225 - DNA, 70 bp, Artificial
  synthetic
aatgatacggcgaccaccgagatctacacgtgagtgatcgtcggcagcgtcagatgtgtataagagacag

SEQ ID NO: 226 - DNA, 70 bp, Artificial
  synthetic
aatgatacggcgaccaccgagatctacactgtcgtcatcgtcggcagcgtcagatgtgtataagagacag

SEQ ID NO: 227 - DNA, 70 bp, Artificial
  synthetic
aatgatacggcgaccaccgagatctacaccacgagcttcgtcggcagcgtcagatgtgtataagagacag

SEQ ID NO: 228 - DNA, 70 bp, Artificial
  synthetic
aatgatacggcgaccaccgagatctacacgagactcttcgtcggcagcgtcagatgtgtataagagacag

SEQ ID NO: 229 - DNA, 70 bp, Artificial
  synthetic
aatgatacggcgaccaccgagatctacaccatgtcactcgtcggcagcgtcagatgtgtataagagacag

SEQ ID NO: 230 - DNA, 70 bp, Artificial
  synthetic
aatgatacggcgaccaccgagatctacaccgtgtacgtcgtcggcagcgtcagatgtgtataagagacag

SEQ ID NO: 231 - DNA, 70 bp, Artificial
  synthetic
aatgatacggcgaccaccgagatctacactcgtagattcgtcggcagcgtcagatgtgtataagagacag

SEQ ID NO: 232 - DNA, 70 bp, Artificial
  synthetic
aatgatacggcgaccaccgagatctacacagctgacatcgtcggcagcgtcagatgtgtataagagacag

SEQ ID NO: 233 - DNA, 70 bp, Artificial
  synthetic
aatgatacggcgaccaccgagatctacaccgtcatcatcgtcggcagcgtcagatgtgtataagagacag

SEQ ID NO: 234 - DNA, 70 bp, Artificial
  synthetic
aatgatacggcgaccaccgagatctacactactcacgtcgtcggcagcgtcagatgtgtataagagacag

SEQ ID NO: 235 - DNA, 70 bp, Artificial
  synthetic
aatgatacggcgaccaccgagatctacaccagtagcgtcgtcggcagcgtcagatgtgtataagagacag

SEQ ID NO: 236 - DNA, 70 bp, Artificial
  synthetic
aatgatacggcgaccaccgagatctacaccatgtagttcgtcggcagcgtcagatgtgtataagagacag

SEQ ID NO: 237 - DNA, 70 bp, Artificial
  synthetic
aatgatacggcgaccaccgagatctacactagagacgtcgtcggcagcgtcagatgtgtataagagacag

SEQ ID NO: 238 - DNA, 70 bp, Artificial
  synthetic
aatgatacggcgaccaccgagatctacaccgtctcagtcgtcggcagcgtcagatgtgtataagagacag

SEQ ID NO: 239 - DNA, 70 bp, Artificial
  synthetic
aatgatacggcgaccaccgagatctacactacatgcatcgtcggcagcgtcagatgtgtataagagacag

SEQ ID NO: 240 - DNA, 70 bp, Artificial
  synthetic
aatgatacggcgaccaccgagatctacactactagcatcgtcggcagcgtcagatgtgtataagagacag

SEQ ID NO: 241 - DNA, 70 bp, Artificial
  synthetic
aatgatacggcgaccaccgagatctacacatgacagatcgtcggcagcgtcagatgtgtataagagacag

SEQ ID NO: 242 - DNA, 70 bp, Artificial
  synthetic
aatgatacggcgaccaccgagatctacacacagcgtatcgtcggcagcgtcagatgtgtataagagacag

SEQ ID NO: 243 - DNA, 70 bp, Artificial
  synthetic
aatgatacggcgaccaccgagatctacaccatgcacttcgtcggcagcgtcagatgtgtataagagacag

SEQ ID NO: 244 - DNA, 70 bp, Artificial
  synthetic
aatgatacggcgaccaccgagatctacactcgagcgttcgtcggcagcgtcagatgtgtataagagacag

SEQ ID NO: 245 - DNA, 70 bp, Artificial
  synthetic
aatgatacggcgaccaccgagatctacaccgcacgagtcgtcggcagcgtcagatgtgtataagagacag

SEQ ID NO: 246 - DNA, 70 bp, Artificial
  synthetic
aatgatacggcgaccaccgagatctacaccacagtattcgtcggcagcgtcagatgtgtataagagacag

SEQ ID NO: 247 - DNA, 70 bp, Artificial
  synthetic
aatgatacggcgaccaccgagatctacacagtcatcatcgtcggcagcgtcagatgtgtataagagacag

SEQ ID NO: 248 - DNA, 70 bp, Artificial
  synthetic
aatgatacggcgaccaccgagatctacactgactatatcgtcggcagcgtcagatgtgtataagagacag

SEQ ID NO: 249 - DNA, 70 bp, Artificial
  synthetic
aatgatacggcgaccaccgagatctacactcgcatattcgtcggcagcgtcagatgtgtataagagacag

SEQ ID NO: 250 - DNA, 70 bp, Artificial
  synthetic
aatgatacggcgaccaccgagatctacacatcgatgttcgtcggcagcgtcagatgtgtataagagacag

SEQ ID NO: 251 - DNA, 70 bp, Artificial
  synthetic
aatgatacggcgaccaccgagatctacaccgacagcgtcgtcggcagcgtcagatgtgtataagagacag

SEQ ID NO: 252 - DNA, 70 bp, Artificial
  synthetic
aatgatacggcgaccaccgagatctacacatcgtgtatcgtcggcagcgtcagatgtgtataagagacag

SEQ ID NO: 253 - DNA, 70 bp, Artificial
  synthetic
aatgatacggcgaccaccgagatctacacgcatgtagtcgtcggcagcgtcagatgtgtataagagacag

SEQ ID NO: 254 - DNA, 70 bp, Artificial
  synthetic
aatgatacggcgaccaccgagatctacacagagatcatcgtcggcagcgtcagatgtgtataagagacag

SEQ ID NO: 255 - DNA, 70 bp, Artificial
  synthetic
aatgatacggcgaccaccgagatctacaccgtcagtatcgtcggcagcgtcagatgtgtataagagacag

SEQ ID NO: 256 - DNA, 70 bp, Artificial
  synthetic
aatgatacggcgaccaccgagatctacacgcgtagattcgtcggcagcgtcagatgtgtataagagacag

SEQ ID NO: 257 - DNA, 70 bp, Artificial
  synthetic
aatgatacggcgaccaccgagatctacacgtactacatcgtcggcagcgtcagatgtgtataagagacag

SEQ ID NO: 258 - DNA, 70 bp, Artificial
  synthetic
aatgatacggcgaccaccgagatctacacgcgagacatcgtcggcagcgtcagatgtgtataagagacag

SEQ ID NO: 259 - DNA, 70 bp, Artificial
  synthetic
aatgatacggcgaccaccgagatctacacgatagacgtcgtcggcagcgtcagatgtgtataagagacag

SEQ ID NO: 260 - DNA, 70 bp, Artificial
  synthetic
aatgatacggcgaccaccgagatctacactatactagtcgtcggcagcgtcagatgtgtataagagacag

SEQ ID NO: 261 - DNA, 70 bp, Artificial
  synthetic
aatgatacggcgaccaccgagatctacactgctcgcatcgtcggcagcgtcagatgtgtataagagacag

SEQ ID NO: 262 - DNA, 66 bp, Artificial
  synthetic
  misc_feature (26)..(27): n is a, c, g, or t
caagcagaagacggcatacgagatcnncttttgtctcgtgggctcggagatgtgtataagagacag

SEQ ID NO: 263 - DNA, 66 bp, Artificial
  synthetic
caagcagaagacggcatacgagatcctcgtttgtctcgtgggctcggagatgtgtataagagacag

SEQ ID NO: 264 - DNA, 66 bp, Artificial
  synthetic
caagcagaagacggcatacgagatccccgtttgtctcgtgggctcggagatgtgtataagagacag

SEQ ID NO: 265 - DNA, 66 bp, Artificial
  synthetic
caagcagaagacggcatacgagatccacgtttgtctcgtgggctcggagatgtgtataagagacag

SEQ ID NO: 266 - DNA, 66 bp, Artificial
  synthetic
  misc_feature (25)..(27): n is a, c, g, or t
  misc_feature (29)..(29): n is a, c, g, or t
caagcagaagacggcatacgagatnnntntttgtctcgtgggctcggagatgtgtataagagacag

SEQ ID NO: 267 - DNA, 66 bp, Artificial
  synthetic
  misc_feature (25)..(27): n is a, c, g, or t
  misc_feature (29)..(29): n is a, c, g, or t
caagcagaagacggcatacgagatnnngntttgtctcgtgggctcggagatgtgtataagagacag

SEQ ID NO: 268 - DNA, 66 bp, Artificial
  synthetic
  misc_feature (26)..(27): n is a, c, g, or t
  misc_feature (29)..(29): n is a, c, g, or t
caagcagaagacggcatacgagattnncntttgtctcgtgggctcggagatgtgtataagagacag

SEQ ID NO: 269 - DNA, 66 bp, Artificial
  synthetic
  misc_feature (26)..(27): n is a, c, g, or t
  misc_feature (29)..(29): n is a, c, g, or t
caagcagaagacggcatacgagatgnncntttgtctcgtgggctcggagatgtgtataagagacag

SEQ ID NO: 270 - DNA, 66 bp, Artificial
  synthetic
  misc_feature (26)..(27): n is a, c, g, or t
  misc_feature (29)..(29): n is a, c, g, or t
caagcagaagacggcatacgagatanncntttgtctcgtgggctcggagatgtgtataagagacag

SEQ ID NO: 271 - DNA, 66 bp, Artificial
  synthetic
  misc_feature (25)..(27): n is a, c, g, or t
  misc_feature (29)..(29): n is a, c, g, or t
caagcagaagacggcatacgagatnnnantttgtctcgtgggctcggagatgtgtataagagacag

SEQ ID NO: 272 - DNA, 66 bp, Artificial
  synthetic
  misc_feature (26)..(27): n is a, c, g, or t
caagcagaagacggcatacgagatcnncatttgtctcgtgggctcggagatgtgtataagagacag

SEQ ID NO: 273 - DNA, 66 bp, Artificial
  synthetic
  misc_feature (26)..(27): n is a, c, g, or t
caagcagaagacggcatacgagatcnnttgttgtctcgtgggctcggagatgtgtataagagacag

SEQ ID NO: 274 - DNA, 66 bp, Artificial
  synthetic
  misc_feature (26)..(27): n is a, c, g, or t
caagcagaagacggcatacgagattnngtgttgtctcgtgggctcggagatgtgtataagagacag

SEQ ID NO: 275 - DNA, 66 bp, Artificial
  synthetic
  misc_feature (26)..(27): n is a, c, g, or t
caagcagaagacggcatacgagatgnngtgttgtctcgtgggctcggagatgtgtataagagacag

SEQ ID NO: 276 - DNA, 66 bp, Artificial
  synthetic
  misc_feature (26)..(27): n is a, c, g, or t
caagcagaagacggcatacgagatcnngtgttgtctcgtgggctcggagatgtgtataagagacag

SEQ ID NO: 277 - DNA, 66 bp, Artificial
  synthetic
  misc_feature (27)..(27): n is a, c, g, or t
caagcagaagacggcatacgagatccnctgttgtctcgtgggctcggagatgtgtataagagacag

SEQ ID NO: 278 - DNA, 66 bp, Artificial
  synthetic
  misc_feature (26)..(27): n is a, c, g, or t
caagcagaagacggcatacgagattnnctgttgtctcgtgggctcggagatgtgtataagagacag

SEQ ID NO: 279 - DNA, 66 bp, Artificial
  synthetic
  misc_feature (26)..(27): n is a, c, g, or t
caagcagaagacggcatacgagatgnnctgttgtctcgtgggctcggagatgtgtataagagacag

SEQ ID NO: 280 - DNA, 66 bp, Artificial
  synthetic
  misc_feature (26)..(27): n is a, c, g, or t
caagcagaagacggcatacgagatannctgttgtctcgtgggctcggagatgtgtataagagacag

SEQ ID NO: 281 - DNA, 66 bp, Artificial
  synthetic
  misc_feature (26)..(27): n is a, c, g, or t
caagcagaagacggcatacgagattnnatgttgtctcgtgggctcggagatgtgtataagagacag

SEQ ID NO: 282 - DNA, 66 bp, Artificial
  synthetic
  misc_feature (26)..(27): n is a, c, g, or t
caagcagaagacggcatacgagatgnnatgttgtctcgtgggctcggagatgtgtataagagacag

SEQ ID NO: 283 - DNA, 66 bp, Artificial
  synthetic
  misc_feature (26)..(27): n is a, c, g, or t
caagcagaagacggcatacgagatcnnatgttgtctcgtgggctcggagatgtgtataagagacag

SEQ ID NO: 284 - DNA, 66 bp, Artificial
  synthetic
  misc_feature (27)..(27): n is a, c, g, or t
caagcagaagacggcatacgagatcgntggttgtctcgtgggctcggagatgtgtataagagacag

SEQ ID NO: 285 - DNA, 66 bp, Artificial
  synthetic
  misc_feature (27)..(27): n is a, c, g, or t
caagcagaagacggcatacgagatccntggttgtctcgtgggctcggagatgtgtataagagacag

SEQ ID NO: 286 - DNA, 66 bp, Artificial
  synthetic
  misc_feature (27)..(27): n is a, c, g, or t
caagcagaagacggcatacgagatcantggttgtctcgtgggctcggagatgtgtataagagacag

SEQ ID NO: 287 - DNA, 66 bp, Artificial
  synthetic
  misc_feature (27)..(27): n is a, c, g, or t
caagcagaagacggcatacgagattgngggttgtctcgtgggctcggagatgtgtataagagacag

SEQ ID NO: 288 - DNA, 66 bp, Artificial
  synthetic
  misc_feature (27)..(27): n is a, c, g, or t
caagcagaagacggcatacgagatggngggttgtctcgtgggctcggagatgtgtataagagacag

SEQ ID NO: 289 - DNA, 66 bp, Artificial
  synthetic
  misc_feature (27)..(27): n is a, c, g, or t
caagcagaagacggcatacgagattcngggttgtctcgtgggctcggagatgtgtataagagacag

SEQ ID NO: 290 - DNA, 66 bp, Artificial
  synthetic
  misc_feature (27)..(27): n is a, c, g, or t
caagcagaagacggcatacgagatgcngggttgtctcgtgggctcggagatgtgtataagagacag

SEQ ID NO: 291 - DNA, 66 bp, Artificial
  synthetic
  misc_feature (27)..(27): n is a, c, g, or t
caagcagaagacggcatacgagattangggttgtctcgtgggctcggagatgtgtataagagacag

SEQ ID NO: 292 - DNA, 66 bp, Artificial
  synthetic
  misc_feature (27)..(27): n is a, c, g, or t
caagcagaagacggcatacgagatgangggttgtctcgtgggctcggagatgtgtataagagacag

SEQ ID NO: 293 - DNA, 66 bp, Artificial
  synthetic
  misc_feature (27)..(27): n is a, c, g, or t
caagcagaagacggcatacgagatagncggttgtctcgtgggctcggagatgtgtataagagacag

SEQ ID NO: 294 - DNA, 66 bp, Artificial
  synthetic
  misc_feature (27)..(27): n is a, c, g, or t
caagcagaagacggcatacgagatacncggttgtctcgtgggctcggagatgtgtataagagacag

SEQ ID NO: 295 - DNA, 66 bp, Artificial
  synthetic
  misc_feature (27)..(27): n is a, c, g, or t
caagcagaagacggcatacgagataancggttgtctcgtgggctcggagatgtgtataagagacag

SEQ ID NO: 296 - DNA, 66 bp, Artificial
  synthetic
  misc_feature (27)..(27): n is a, c, g, or t
caagcagaagacggcatacgagattgnaggttgtctcgtgggctcggagatgtgtataagagacag

SEQ ID NO: 297 - DNA, 66 bp, Artificial
  synthetic
  misc_feature (27)..(27): n is a, c, g, or t
caagcagaagacggcatacgagatggnaggttgtctcgtgggctcggagatgtgtataagagacag

SEQ ID NO: 298 - DNA, 66 bp, Artificial
  synthetic
  misc_feature (27)..(27): n is a, c, g, or t
caagcagaagacggcatacgagattcnaggttgtctcgtgggctcggagatgtgtataagagacag

SEQ ID NO: 299 - DNA, 66 bp, Artificial
  synthetic
  misc_feature (27)..(27): n is a, c, g, or t
caagcagaagacggcatacgagatgcnaggttgtctcgtgggctcggagatgtgtataagagacag

SEQ ID NO: 300 - DNA, 66 bp, Artificial
  synthetic
  misc_feature (27)..(27): n is a, c, g, or t
caagcagaagacggcatacgagattanaggttgtctcgtgggctcggagatgtgtataagagacag

SEQ ID NO: 301 - DNA, 66 bp, Artificial
  synthetic
  misc_feature (27)..(27): n is a, c, g, or t
caagcagaagacggcatacgagatganaggttgtctcgtgggctcggagatgtgtataagagacag

SEQ ID NO: 302 - DNA, 66 bp, Artificial
  synthetic
  misc_feature (27)..(27): n is a, c, g, or t
caagcagaagacggcatacgagatcgntcgttgtctcgtgggctcggagatgtgtataagagacag

SEQ ID NO: 303 - DNA, 66 bp, Artificial
  synthetic
  misc_feature (27)..(27): n is a, c, g, or t
caagcagaagacggcatacgagatccntcgttgtctcgtgggctcggagatgtgtataagagacag

SEQ ID NO: 304 - DNA, 66 bp, Artificial
  synthetic
  misc_feature (27)..(27): n is a, c, g, or t
caagcagaagacggcatacgagatcantcgttgtctcgtgggctcggagatgtgtataagagacag

SEQ ID NO: 305 - DNA, 66 bp, Artificial
  synthetic
  misc_feature (27)..(27): n is a, c, g, or t
caagcagaagacggcatacgagattgngcgttgtctcgtgggctcggagatgtgtataagagacag

SEQ ID NO: 306 - DNA, 66 bp, Artificial
  synthetic
  misc_feature (27)..(27): n is a, c, g, or t
caagcagaagacggcatacgagatggngcgttgtctcgtgggctcggagatgtgtataagagacag

SEQ ID NO: 307 - DNA, 66 bp, Artificial
  synthetic
  misc_feature (27)..(27): n is a, c, g, or t
caagcagaagacggcatacgagattcngcgttgtctcgtgggctcggagatgtgtataagagacag

SEQ ID NO: 308 - DNA, 66 bp, Artificial
  synthetic
  misc_feature (27)..(27): n is a, c, g, or t
caagcagaagacggcatacgagatgcngcgttgtctcgtgggctcggagatgtgtataagagacag

SEQ ID NO: 309 - DNA, 66 bp, Artificial
  synthetic
  misc_feature (27)..(27): n is a, c, g, or t
caagcagaagacggcatacgagattangcgttgtctcgtgggctcggagatgtgtataagagacag

SEQ ID NO: 310 - DNA, 66 bp, Artificial
  synthetic
  misc_feature (27)..(27): n is a, c, g, or t
caagcagaagacggcatacgagatgangcgttgtctcgtgggctcggagatgtgtataagagacag

SEQ ID NO: 311 - DNA, 66 bp, Artificial
  synthetic
  misc_feature (27)..(27): n is a, c, g, or t
caagcagaagacggcatacgagatagnccgttgtctcgtgggctcggagatgtgtataagagacag

SEQ ID NO: 312 - DNA, 66 bp, Artificial
  synthetic
  misc_feature (27)..(27): n is a, c, g, or t
caagcagaagacggcatacgagatacnccgttgtctcgtgggctcggagatgtgtataagagacag

SEQ ID NO: 313 - DNA, 66 bp, Artificial
  synthetic
  misc_feature (27)..(27): n is a, c, g, or t
caagcagaagacggcatacgagataanccgttgtctcgtgggctcggagatgtgtataagagacag

SEQ ID NO: 314 - DNA, 66 bp, Artificial
  synthetic
  misc_feature (27)..(27): n is a, c, g, or t
caagcagaagacggcatacgagattgnacgttgtctcgtgggctcggagatgtgtataagagacag

SEQ ID NO: 315 - DNA, 66 bp, Artificial
  synthetic
  misc_feature (27)..(27): n is a, c, g, or t
caagcagaagacggcatacgagatggnacgttgtctcgtgggctcggagatgtgtataagagacag

SEQ ID NO: 316 - DNA, 66 bp, Artificial
  synthetic
  misc_feature (27)..(27): n is a, c, g, or t
caagcagaagacggcatacgagattcnacgttgtctcgtgggctcggagatgtgtataagagacag

SEQ ID NO: 317 - DNA, 66 bp, Artificial
  synthetic
  misc_feature (27)..(27): n is a, c, g, or t
caagcagaagacggcatacgagatgcnacgttgtctcgtgggctcggagatgtgtataagagacag

SEQ ID NO: 318 - DNA, 66 bp, Artificial
  synthetic
  misc_feature (27)..(27): n is a, c, g, or t
caagcagaagacggcatacgagattanacgttgtctcgtgggctcggagatgtgtataagagacag

SEQ ID NO: 319 - DNA, 66 bp, Artificial
  synthetic
  misc_feature (27)..(27): n is a, c, g, or t
caagcagaagacggcatacgagatganacgttgtctcgtgggctcggagatgtgtataagagacag

SEQ ID NO: 320 - DNA, 66 bp, Artificial
  synthetic
  misc_feature (26)..(27): n is a, c, g, or t
  misc_feature (29)..(29): n is a, c, g, or t
caagcagaagacggcatacgagattnntngttgtctcgtgggctcggagatgtgtataagagacag

SEQ ID NO: 321 - DNA, 66 bp, Artificial
  synthetic
  misc_feature (26)..(27): n is a, c, g, or t
  misc_feature (29)..(29): n is a, c, g, or t
caagcagaagacggcatacgagatgnntngttgtctcgtgggctcggagatgtgtataagagacag

SEQ ID NO: 322 - DNA, 66 bp, Artificial
  synthetic
  misc_feature (26)..(27): n is a, c, g, or t
  misc_feature (29)..(29): n is a, c, g, or t
caagcagaagacggcatacgagatanntngttgtctcgtgggctcggagatgtgtataagagacag

SEQ ID NO: 323 - DNA, 66 bp, Artificial
  synthetic
  misc_feature (26)..(27): n is a, c, g, or t
  misc_feature (29)..(29): n is a, c, g, or t
caagcagaagacggcatacgagatanngngttgtctcgtgggctcggagatgtgtataagagacag

SEQ ID NO: 324 - DNA, 66 bp, Artificial
  synthetic
  misc_feature (26)..(27): n is a, c, g, or t
  misc_feature (29)..(29): n is a, c, g, or t
caagcagaagacggcatacgagatannangttgtctcgtgggctcggagatgtgtataagagacag

SEQ ID NO: 325 - DNA, 66 bp, Artificial
  synthetic
  misc_feature (26)..(27): n is a, c, g, or t
caagcagaagacggcatacgagatcnntagttgtctcgtgggctcggagatgtgtataagagacag

SEQ ID NO: 326 - DNA, 66 bp, Artificial
  synthetic
  misc_feature (26)..(27): n is a, c, g, or t
caagcagaagacggcatacgagattnngagttgtctcgtgggctcggagatgtgtataagagacag

SEQ ID NO: 327 - DNA, 66 bp, Artificial
  synthetic
  misc_feature (26)..(27): n is a, c, g, or t
caagcagaagacggcatacgagatgnngagttgtctcgtgggctcggagatgtgtataagagacag

SEQ ID NO: 328 - DNA, 66 bp, Artificial
  synthetic
  misc_feature (27)..(27): n is a, c, g, or t
caagcagaagacggcatacgagattgncagttgtctcgtgggctcggagatgtgtataagagacag

SEQ ID NO: 329 - DNA, 66 bp, Artificial
  synthetic
  misc_feature (27)..(27): n is a, c, g, or t
caagcagaagacggcatacgagatggncagttgtctcgtgggctcggagatgtgtataagagacag

SEQ ID NO: 330 - DNA, 66 bp, Artificial
  synthetic
  misc_feature (27)..(27): n is a, c, g, or t
caagcagaagacggcatacgagattcncagttgtctcgtgggctcggagatgtgtataagagacag

SEQ ID NO: 331 - DNA, 66 bp, Artificial
  synthetic
  misc_feature (27)..(27): n is a, c, g, or t
caagcagaagacggcatacgagatgcncagttgtctcgtgggctcggagatgtgtataagagacag

SEQ ID NO: 332 - DNA, 66 bp, Artificial
  synthetic
  misc_feature (26)..(27): n is a, c, g, or t
caagcagaagacggcatacgagatanncagttgtctcgtgggctcggagatgtgtataagagacag

SEQ ID NO: 333 - DNA, 66 bp, Artificial
  synthetic
  misc_feature (27)..(27): n is a, c, g, or t
caagcagaagacggcatacgagattancagttgtctcgtgggctcggagatgtgtataagagacag

SEQ ID NO: 334 - DNA, 66 bp, Artificial
  synthetic
  misc_feature (27)..(27): n is a, c, g, or t
caagcagaagacggcatacgagatgancagttgtctcgtgggctcggagatgtgtataagagacag

SEQ ID NO: 335 - DNA, 66 bp, Artificial
  synthetic
  misc_feature (26)..(27): n is a, c, g, or t
caagcagaagacggcatacgagattnnaagttgtctcgtgggctcggagatgtgtataagagacag

SEQ ID NO: 336 - DNA, 66 bp, Artificial
  synthetic
  misc_feature (26)..(27): n is a, c, g, or t
caagcagaagacggcatacgagatgnnaagttgtctcgtgggctcggagatgtgtataagagacag

SEQ ID NO: 337 - DNA, 66 bp, Artificial
  synthetic
  misc_feature (26)..(27): n is a, c, g, or t
caagcagaagacggcatacgagatcnnttcttgtctcgtgggctcggagatgtgtataagagacag

SEQ ID NO: 338 - DNA, 66 bp, Artificial
  synthetic
  misc_feature (26)..(27): n is a, c, g, or t
caagcagaagacggcatacgagattnngtcttgtctcgtgggctcggagatgtgtataagagacag

SEQ ID NO: 339 - DNA, 66 bp, Artificial
  synthetic
  misc_feature (26)..(27): n is a, c, g, or t
caagcagaagacggcatacgagatgnngtcttgtctcgtgggctcggagatgtgtataagagacag

SEQ ID NO: 340 - DNA, 66 bp, Artificial
  synthetic
  misc_feature (26)..(27): n is a, c, g, or t
caagcagaagacggcatacgagatcnngtcttgtctcgtgggctcggagatgtgtataagagacag

SEQ ID NO: 341 - DNA, 66 bp, Artificial
  synthetic
caagcagaagacggcatacgagatcctctcttgtctcgtgggctcggagatgtgtataagagacag

SEQ ID NO: 342 - DNA, 66 bp, Artificial
  synthetic
caagcagaagacggcatacgagatcccctcttgtctcgtgggctcggagatgtgtataagagacag

SEQ ID NO: 343 - DNA, 66 bp, Artificial
  synthetic
  misc_feature (26)..(27): n is a, c, g, or t
caagcagaagacggcatacgagattnnctcttgtctcgtgggctcggagatgtgtataagagacag

SEQ ID NO: 344 - DNA, 66 bp, Artificial
  synthetic
  misc_feature (26)..(27): n is a, c, g, or t
caagcagaagacggcatacgagatgnnctcttgtctcgtgggctcggagatgtgtataagagacag

SEQ ID NO: 345 - DNA, 66 bp, Artificial
  synthetic
  misc_feature (26)..(27): n is a, c, g, or t
caagcagaagacggcatacgagatannctcttgtctcgtgggctcggagatgtgtataagagacag

SEQ ID NO: 346 - DNA, 66 bp, Artificial
  synthetic
caagcagaagacggcatacgagatccactcttgtctcgtgggctcggagatgtgtataagagacag

SEQ ID NO: 347 - DNA, 66 bp, Artificial
  synthetic
  misc_feature (26)..(27): n is a, c, g, or t
caagcagaagacggcatacgagattnnatcttgtctcgtgggctcggagatgtgtataagagacag

SEQ ID NO: 348 - DNA, 66 bp, Artificial
  synthetic
  misc_feature (26)..(27): n is a, c, g, or t
caagcagaagacggcatacgagatgnnatcttgtctcgtgggctcggagatgtgtataagagacag

SEQ ID NO: 349 - DNA, 66 bp, Artificial
  synthetic
  misc_feature (26)..(27): n is a, c, g, or t
caagcagaagacggcatacgagatcnnatcttgtctcgtgggctcggagatgtgtataagagacag

SEQ ID NO: 350 - DNA, 66 bp, Artificial
  synthetic
  misc_feature (27)..(27): n is a, c, g, or t
caagcagaagacggcatacgagatcgntgcttgtctcgtgggctcggagatgtgtataagagacag

SEQ ID NO: 351 - DNA, 66 bp, Artificial
  synthetic
  misc_feature (27)..(27): n is a, c, g, or t
caagcagaagacggcatacgagatccntgcttgtctcgtgggctcggagatgtgtataagagacag

SEQ ID NO: 352 - DNA, 66 bp, Artificial
  synthetic
  misc_feature (27)..(27): n is a, c, g, or t
caagcagaagacggcatacgagatcantgcttgtctcgtgggctcggagatgtgtataagagacag

SEQ ID NO: 353 - DNA, 66 bp, Artificial
  synthetic
  misc_feature (27)..(27): n is a, c, g, or t
caagcagaagacggcatacgagattgnggcttgtctcgtgggctcggagatgtgtataagagacag

SEQ ID NO: 354 - DNA, 66 bp, Artificial
  synthetic
  misc_feature (27)..(27): n is a, c, g, or t
caagcagaagacggcatacgagatggnggcttgtctcgtgggctcggagatgtgtataagagacag

SEQ ID NO: 355 - DNA, 66 bp, Artificial
  synthetic
  misc_feature (27)..(27): n is a, c, g, or t
caagcagaagacggcatacgagattcnggcttgtctcgtgggctcggagatgtgtataagagacag

SEQ ID NO: 356 - DNA, 66 bp, Artificial
  synthetic
  misc_feature (27)..(27): n is a, c, g, or t
caagcagaagacggcatacgagatgcnggcttgtctcgtgggctcggagatgtgtataagagacag

SEQ ID NO: 357 - DNA, 66 bp, Artificial
  synthetic
  misc_feature (27)..(27): n is a, c, g, or t
caagcagaagacggcatacgagattanggcttgtctcgtgggctcggagatgtgtataagagacag

SEQ ID NO: 358 - DNA, 66 bp, Artificial
  synthetic
  misc_feature (27)..(27): n is a, c, g, or t
caagcagaagacggcatacgagatganggcttgtctcgtgggctcggagatgtgtataagagacag

SEQ ID NO: 359 - DNA, 66 bp, Artificial
  synthetic
  misc_feature (27)..(27): n is a, c, g, or t
caagcagaagacggcatacgagatagncgcttgtctcgtgggctcggagatgtgtataagagacag

SEQ ID NO: 360 - DNA, 66 bp, Artificial
  synthetic
  misc_feature (27)..(27): n is a, c, g, or t
caagcagaagacggcatacgagatacncgcttgtctcgtgggctcggagatgtgtataagagacag

SEQ ID NO: 361 - DNA, 66 bp, Artificial
  synthetic
  misc_feature (27)..(27): n is a, c, g, or t
caagcagaagacggcatacgagataancgcttgtctcgtgggctcggagatgtgtataagagacag

SEQ ID NO: 362 - DNA, 66 bp, Artificial
  synthetic
  misc_feature (27)..(27): n is a, c, g, or t
caagcagaagacggcatacgagattgnagcttgtctcgtgggctcggagatgtgtataagagacag

SEQ ID NO: 363 - DNA, 66 bp, Artificial
  synthetic
  misc_feature (27)..(27): n is a, c, g, or t
caagcagaagacggcatacgagatggnagcttgtctcgtgggctcggagatgtgtataagagacag

SEQ ID NO: 364 - DNA, 66 bp, Artificial
  synthetic
  misc_feature (27)..(27): n is a, c, g, or t
caagcagaagacggcatacgagattcnagcttgtctcgtgggctcggagatgtgtataagagacag

SEQ ID NO: 365 - DNA, 66 bp, Artificial
  synthetic
  misc_feature (27)..(27): n is a, c, g, or t
caagcagaagacggcatacgagatgcnagcttgtctcgtgggctcggagatgtgtataagagacag

SEQ ID NO: 366 - DNA, 66 bp, Artificial
  synthetic
  misc_feature (27)..(27): n is a, c, g, or t
caagcagaagacggcatacgagattanagcttgtctcgtgggctcggagatgtgtataagagacag

SEQ ID NO: 367 - DNA, 66 bp, Artificial
  synthetic
  misc_feature (27)..(27): n is a, c, g, or t
caagcagaagacggcatacgagatganagcttgtctcgtgggctcggagatgtgtataagagacag

SEQ ID NO: 368 - DNA, 66 bp, Artificial
  synthetic
  misc_feature (27)..(27): n is a, c, g, or t
caagcagaagacggcatacgagatcgntccttgtctcgtgggctcggagatgtgtataagagacag

SEQ ID NO: 369 - DNA, 66 bp, Artificial
  synthetic
  misc_feature (27)..(27): n is a, c, g, or t
caagcagaagacggcatacgagatccntccttgtctcgtgggctcggagatgtgtataagagacag

SEQ ID NO: 370 - DNA, 66 bp, Artificial
  synthetic
  misc_feature (27)..(27): n is a, c, g, or t
caagcagaagacggcatacgagatcantccttgtctcgtgggctcggagatgtgtataagagacag

SEQ ID NO: 371 - DNA, 66 bp, Artificial
  synthetic
  misc_feature (27)..(27): n is a, c, g, or t
caagcagaagacggcatacgagattgngccttgtctcgtgggctcggagatgtgtataagagacag

SEQ ID NO: 372 - DNA, 66 bp, Artificial
  synthetic
  misc_feature (27)..(27): n is a, c, g, or t
caagcagaagacggcatacgagatggngccttgtctcgtgggctcggagatgtgtataagagacag

SEQ ID NO: 373 - DNA, 66 bp, Artificial
  synthetic
  misc_feature (27)..(27): n is a, c, g, or t
caagcagaagacggcatacgagattcngccttgtctcgtgggctcggagatgtgtataagagacag

SEQ ID NO: 374 - DNA, 66 bp, Artificial
  synthetic
  misc_feature (27)..(27): n is a, c, g, or t
caagcagaagacggcatacgagatgcngccttgtctcgtgggctcggagatgtgtataagagacag

SEQ ID NO: 375 - DNA, 66 bp, Artificial
  synthetic
  misc_feature (27)..(27): n is a, c, g, or t
caagcagaagacggcatacgagattangccttgtctcgtgggctcggagatgtgtataagagacag

SEQ ID NO: 376 - DNA, 66 bp, Artificial
  synthetic
  misc_feature (27)..(27): n is a, c, g, or t
caagcagaagacggcatacgagatgangccttgtctcgtgggctcggagatgtgtataagagacag

SEQ ID NO: 377 - DNA, 66 bp, Artificial
  synthetic
  misc_feature (27)..(27): n is a, c, g, or t
caagcagaagacggcatacgagatagncccttgtctcgtgggctcggagatgtgtataagagacag

SEQ ID NO: 378 - DNA, 66 bp, Artificial
  synthetic
  misc_feature (27)..(27): n is a, c, g, or t
caagcagaagacggcatacgagatacncccttgtctcgtgggctcggagatgtgtataagagacag

SEQ ID NO: 379 - DNA, 66 bp, Artificial
  synthetic
  misc_feature (27)..(27): n is a, c, g, or t
caagcagaagacggcatacgagataancccttgtctcgtgggctcggagatgtgtataagagacag

SEQ ID NO: 380 - DNA, 66 bp, Artificial
  synthetic
  misc_feature (27)..(27): n is a, c, g, or t
caagcagaagacggcatacgagattgnaccttgtctcgtgggctcggagatgtgtataagagacag

SEQ ID NO: 381 - DNA, 66 bp, Artificial
  synthetic
  misc_feature (27)..(27): n is a, c, g, or t
caagcagaagacggcatacgagatggnaccttgtctcgtgggctcggagatgtgtataagagacag

SEQ ID NO: 382 - DNA, 66 bp, Artificial
  synthetic
  misc_feature (27)..(27): n is a, c, g, or t
caagcagaagacggcatacgagattcnaccttgtctcgtgggctcggagatgtgtataagagacag

SEQ ID NO: 383 - DNA, 66 bp, Artificial
  synthetic
  misc_feature (27)..(27): n is a, c, g, or t
caagcagaagacggcatacgagatgcnaccttgtctcgtgggctcggagatgtgtataagagacag

SEQ ID NO: 384 - DNA, 66 bp, Artificial
  synthetic
  misc_feature (27)..(27): n is a, c, g, or t
caagcagaagacggcatacgagattanaccttgtctcgtgggctcggagatgtgtataagagacag

SEQ ID NO: 385 - DNA, 66 bp, Artificial
  synthetic
  misc_feature (27)..(27): n is a, c, g, or t
caagcagaagacggcatacgagatganaccttgtctcgtgggctcggagatgtgtataagagacag

SEQ ID NO: 386 - DNA, 66 bp, Artificial
  synthetic
  misc_feature (26)..(27): n is a, c, g, or t
  misc_feature (29)..(29): n is a, c, g, or t
caagcagaagacggcatacgagattnntncttgtctcgtgggctcggagatgtgtataagagacag

SEQ ID NO: 387 - DNA, 66 bp, Artificial
  synthetic
  misc_feature (26)..(27): n is a, c, g, or t
  misc_feature (29)..(29): n is a, c, g, or t
caagcagaagacggcatacgagatgnntncttgtctcgtgggctcggagatgtgtataagagacag

SEQ ID NO: 388 - DNA, 66 bp, Artificial
  synthetic
  misc_feature (26)..(27): n is a, c, g, or t
  misc_feature (29)..(29): n is a, c, g, or t
caagcagaagacggcatacgagatanntncttgtctcgtgggctcggagatgtgtataagagacag

SEQ ID NO: 389 - DNA, 66 bp, Artificial
  synthetic
  misc_feature (26)..(27): n is a, c, g, or t
  misc_feature (29)..(29): n is a, c, g, or t
caagcagaagacggcatacgagatanngncttgtctcgtgggctcggagatgtgtataagagacag

SEQ ID NO: 390 - DNA, 66 bp, Artificial
  synthetic
  misc_feature (26)..(27): n is a, c, g, or t
  misc_feature (29)..(29): n is a, c, g, or t
caagcagaagacggcatacgagatannancttgtctcgtgggctcggagatgtgtataagagacag

SEQ ID NO: 391 - DNA, 66 bp, Artificial
  synthetic
  misc_feature (26)..(27): n is a, c, g, or t
caagcagaagacggcatacgagatcnntacttgtctcgtgggctcggagatgtgtataagagacag

SEQ ID NO: 392 - DNA, 66 bp, Artificial
  synthetic
  misc_feature (26)..(27): n is a, c, g, or t
caagcagaagacggcatacgagattnngacttgtctcgtgggctcggagatgtgtataagagacag

SEQ ID NO: 393 - DNA, 66 bp, Artificial
  synthetic
  misc_feature (26)..(27): n is a, c, g, or t
caagcagaagacggcatacgagatgnngacttgtctcgtgggctcggagatgtgtataagagacag

SEQ ID NO: 394 - DNA, 66 bp, Artificial
  synthetic
  misc_feature (27)..(27): n is a, c, g, or t
caagcagaagacggcatacgagattgncacttgtctcgtgggctcggagatgtgtataagagacag

SEQ ID NO: 395 - DNA, 66 bp, Artificial
  synthetic
  misc_feature (27)..(27): n is a, c, g, or t
caagcagaagacggcatacgagatggncacttgtctcgtgggctcggagatgtgtataagagacag

SEQ ID NO: 396 - DNA, 66 bp, Artificial
  synthetic
  misc_feature (27)..(27): n is a, c, g, or t
caagcagaagacggcatacgagattcncacttgtctcgtgggctcggagatgtgtataagagacag

SEQ ID NO: 397 - DNA, 66 bp, Artificial
  synthetic
  misc_feature (27)..(27): n is a, c, g, or t
caagcagaagacggcatacgagatgcncacttgtctcgtgggctcggagatgtgtataagagacag

SEQ ID NO: 398 - DNA, 66 bp, Artificial
  synthetic
  misc_feature (26)..(27): n is a, c, g, or t
caagcagaagacggcatacgagatanncacttgtctcgtgggctcggagatgtgtataagagacag

SEQ ID NO: 399 - DNA, 66 bp, Artificial
  synthetic
  misc_feature (27)..(27): n is a, c, g, or t
caagcagaagacggcatacgagattancacttgtctcgtgggctcggagatgtgtataagagacag

SEQ ID NO: 400 - DNA, 66 bp, Artificial
  synthetic
  misc_feature (27)..(27): n is a, c, g, or t
caagcagaagacggcatacgagatgancacttgtctcgtgggctcggagatgtgtataagagacag

SEQ ID NO: 401 - DNA, 66 bp, Artificial
  synthetic
  misc_feature (26)..(27): n is a, c, g, or t
caagcagaagacggcatacgagattnnaacttgtctcgtgggctcggagatgtgtataagagacag

SEQ ID NO: 402 - DNA, 66 bp, Artificial
  synthetic
  misc_feature (26)..(27): n is a, c, g, or t
caagcagaagacggcatacgagatgnnaacttgtctcgtgggctcggagatgtgtataagagacag

SEQ ID NO: 403 - DNA, 66 bp, Artificial
  synthetic
  misc_feature (26)..(27): n is a, c, g, or t
caagcagaagacggcatacgagatcnngtattgtctcgtgggctcggagatgtgtataagagacag

SEQ ID NO: 404 - DNA, 66 bp, Artificial
  synthetic
  misc_feature (26)..(27): n is a, c, g, or t
caagcagaagacggcatacgagattnnctattgtctcgtgggctcggagatgtgtataagagacag

SEQ ID NO: 405 - DNA, 66 bp, Artificial
  synthetic
  misc_feature (26)..(27): n is a, c, g, or t
caagcagaagacggcatacgagatgnnctattgtctcgtgggctcggagatgtgtataagagacag

SEQ ID NO: 406 - DNA, 66 bp, Artificial
  synthetic
  misc_feature (26)..(27): n is a, c, g, or t
caagcagaagacggcatacgagatcnnctattgtctcgtgggctcggagatgtgtataagagacag

SEQ ID NO: 407 - DNA, 66 bp, Artificial
  synthetic
  misc_feature (26)..(27): n is a, c, g, or t
caagcagaagacggcatacgagatcnnatattgtctcgtgggctcggagatgtgtataagagacag

SEQ ID NO: 408 - DNA, 66 bp, Artificial
  synthetic
caagcagaagacggcatacgagatcctggattgtctcgtgggctcggagatgtgtataagagacag

SEQ ID NO: 409 - DNA, 66 bp, Artificial
  synthetic
caagcagaagacggcatacgagatcccggattgtctcgtgggctcggagatgtgtataagagacag

SEQ ID NO: 410 - DNA, 66 bp, Artificial
  synthetic
caagcagaagacggcatacgagatccaggattgtctcgtgggctcggagatgtgtataagagacag

SEQ ID NO: 411 - DNA, 66 bp, Artificial
  synthetic
  misc_feature (27)..(27): n is a, c, g, or t
caagcagaagacggcatacgagattgncgattgtctcgtgggctcggagatgtgtataagagacag

SEQ ID NO: 412 - DNA, 66 bp, Artificial
  synthetic
  misc_feature (27)..(27): n is a, c, g, or t
caagcagaagacggcatacgagatggncgattgtctcgtgggctcggagatgtgtataagagacag

SEQ ID NO: 413 - DNA, 66 bp, Artificial
  synthetic
  misc_feature (27)..(27): n is a, c, g, or t
caagcagaagacggcatacgagattcncgattgtctcgtgggctcggagatgtgtataagagacag

SEQ ID NO: 414 - DNA, 66 bp, Artificial
  synthetic
  misc_feature (27)..(27): n is a, c, g, or t
caagcagaagacggcatacgagatgcncgattgtctcgtgggctcggagatgtgtataagagacag

SEQ ID NO: 415 - DNA, 66 bp, Artificial
  synthetic
  misc_feature (27)..(27): n is a, c, g, or t
caagcagaagacggcatacgagattancgattgtctcgtgggctcggagatgtgtataagagacag

SEQ ID NO: 416 - DNA, 66 bp, Artificial
  synthetic
  misc_feature (27)..(27): n is a, c, g, or t
caagcagaagacggcatacgagatgancgattgtctcgtgggctcggagatgtgtataagagacag

SEQ ID NO: 417 - DNA, 66 bp, Artificial
  synthetic
caagcagaagacggcatacgagatcctagattgtctcgtgggctcggagatgtgtataagagacag

SEQ ID NO: 418 - DNA, 66 bp, Artificial
  synthetic
caagcagaagacggcatacgagatcccagattgtctcgtgggctcggagatgtgtataagagacag

SEQ ID NO: 419 - DNA, 66 bp, Artificial
  synthetic
caagcagaagacggcatacgagatccaagattgtctcgtgggctcggagatgtgtataagagacag

SEQ ID NO: 420 - DNA, 66 bp, Artificial
  synthetic
  misc_feature (27)..(27): n is a, c, g, or t
caagcagaagacggcatacgagattgnccattgtctcgtgggctcggagatgtgtataagagacag

SEQ ID NO: 421 - DNA, 66 bp, Artificial
  synthetic
  misc_feature (27)..(27): n is a, c, g, or t
caagcagaagacggcatacgagatggnccattgtctcgtgggctcggagatgtgtataagagacag

SEQ ID NO: 422 - DNA, 66 bp, Artificial
  synthetic
  misc_feature (27)..(27): n is a, c, g, or t
caagcagaagacggcatacgagattcnccattgtctcgtgggctcggagatgtgtataagagacag

SEQ ID NO: 423 - DNA, 66 bp, Artificial
  synthetic
  misc_feature (27)..(27): n is a, c, g, or t
caagcagaagacggcatacgagatgcnccattgtctcgtgggctcggagatgtgtataagagacag

SEQ ID NO: 424 - DNA, 66 bp, Artificial
  synthetic
  misc_feature (27)..(27): n is a, c, g, or t
caagcagaagacggcatacgagattanccattgtctcgtgggctcggagatgtgtataagagacag

SEQ ID NO: 425 - DNA, 66 bp, Artificial
  synthetic
  misc_feature (27)..(27): n is a, c, g, or t
caagcagaagacggcatacgagatganccattgtctcgtgggctcggagatgtgtataagagacag

SEQ ID NO: 426 - DNA, 66 bp, Artificial
  synthetic
  misc_feature (25)..(27): n is a, c, g, or t
  misc_feature (29)..(29): n is a, c, g, or t
caagcagaagacggcatacgagatnnntnattgtctcgtgggctcggagatgtgtataagagacag

SEQ ID NO: 427 - DNA, 66 bp, Artificial
  synthetic
  misc_feature (26)..(27): n is a, c, g, or t
  misc_feature (29)..(29): n is a, c, g, or t
caagcagaagacggcatacgagattnngnattgtctcgtgggctcggagatgtgtataagagacag

SEQ ID NO: 428 - DNA, 66 bp, Artificial
  synthetic
  misc_feature (26)..(27): n is a, c, g, or t
  misc_feature (29)..(29): n is a, c, g, or t
caagcagaagacggcatacgagatgnngnattgtctcgtgggctcggagatgtgtataagagacag

SEQ ID NO: 429 - DNA, 66 bp, Artificial
  synthetic
  misc_feature (26)..(27): n is a, c, g, or t
  misc_feature (29)..(29): n is a, c, g, or t
caagcagaagacggcatacgagatanngnattgtctcgtgggctcggagatgtgtataagagacag

SEQ ID NO: 430 - DNA, 66 bp, Artificial
  synthetic
  misc_feature (26)..(27): n is a, c, g, or t
  misc_feature (29)..(29): n is a, c, g, or t
caagcagaagacggcatacgagatanncnattgtctcgtgggctcggagatgtgtataagagacag

SEQ ID NO: 431 - DNA, 66 bp, Artificial
  synthetic
  misc_feature (26)..(27): n is a, c, g, or t
  misc_feature (29)..(29): n is a, c, g, or t
caagcagaagacggcatacgagattnnanattgtctcgtgggctcggagatgtgtataagagacag

SEQ ID NO: 432 - DNA, 66 bp, Artificial
  synthetic
  misc_feature (26)..(27): n is a, c, g, or t
  misc_feature (29)..(29): n is a, c, g, or t
caagcagaagacggcatacgagatgnnanattgtctcgtgggctcggagatgtgtataagagacag

SEQ ID NO: 433 - DNA, 66 bp, Artificial
  synthetic
  misc_feature (26)..(27): n is a, c, g, or t
  misc_feature (29)..(29): n is a, c, g, or t
caagcagaagacggcatacgagatannanattgtctcgtgggctcggagatgtgtataagagacag

SEQ ID NO: 434 - DNA, 66 bp, Artificial
  synthetic
  misc_feature (26)..(27): n is a, c, g, or t
caagcagaagacggcatacgagatcnngaattgtctcgtgggctcggagatgtgtataagagacag

SEQ ID NO: 435 - DNA, 66 bp, Artificial
  synthetic
  misc_feature (26)..(27): n is a, c, g, or t
caagcagaagacggcatacgagattnncaattgtctcgtgggctcggagatgtgtataagagacag

SEQ ID NO: 436 - DNA, 66 bp, Artificial
  synthetic
  misc_feature (26)..(27): n is a, c, g, or t
caagcagaagacggcatacgagatgnncaattgtctcgtgggctcggagatgtgtataagagacag

SEQ ID NO: 437 - DNA, 66 bp, Artificial
  synthetic
  misc_feature (26)..(27): n is a, c, g, or t
caagcagaagacggcatacgagatcnnaaattgtctcgtgggctcggagatgtgtataagagacag

SEQ ID NO: 438 - DNA, 66 bp, Artificial
  synthetic
  misc_feature (26)..(27): n is a, c, g, or t
caagcagaagacggcatacgagatcnntttgtgtctcgtgggctcggagatgtgtataagagacag

SEQ ID NO: 439 - DNA, 66 bp, Artificial
  synthetic
  misc_feature (26)..(27): n is a, c, g, or t
caagcagaagacggcatacgagattnngttgtgtctcgtgggctcggagatgtgtataagagacag

SEQ ID NO: 440 - DNA, 66 bp, Artificial
  synthetic
  misc_feature (26)..(27): n is a, c, g, or t
caagcagaagacggcatacgagatgnngttgtgtctcgtgggctcggagatgtgtataagagacag

SEQ ID NO: 441 - DNA, 66 bp, Artificial
  synthetic
  misc_feature (26)..(27): n is a, c, g, or t
caagcagaagacggcatacgagatcnngttgtgtctcgtgggctcggagatgtgtataagagacag

SEQ ID NO: 442 - DNA, 66 bp, Artificial
  synthetic
  misc_feature (27)..(27): n is a, c, g, or t
caagcagaagacggcatacgagatcgncttgtgtctcgtgggctcggagatgtgtataagagacag

SEQ ID NO: 443 - DNA, 66 bp, Artificial
  synthetic
  misc_feature (27)..(27): n is a, c, g, or t
caagcagaagacggcatacgagatccncttgtgtctcgtgggctcggagatgtgtataagagacag

SEQ ID NO: 444 - DNA, 66 bp, Artificial
  synthetic
  misc_feature (26)..(27): n is a, c, g, or t
caagcagaagacggcatacgagattnncttgtgtctcgtgggctcggagatgtgtataagagacag

SEQ ID NO: 445 - DNA, 66 bp, Artificial
  synthetic
  misc_feature (26)..(27): n is a, c, g, or t
caagcagaagacggcatacgagatgnncttgtgtctcgtgggctcggagatgtgtataagagacag

SEQ ID NO: 446 - DNA, 66 bp, Artificial
  synthetic
  misc_feature (26)..(27): n is a, c, g, or t
caagcagaagacggcatacgagatanncttgtgtctcgtgggctcggagatgtgtataagagacag

SEQ ID NO: 447 - DNA, 66 bp, Artificial
  synthetic
  misc_feature (27)..(27): n is a, c, g, or t
caagcagaagacggcatacgagatcancttgtgtctcgtgggctcggagatgtgtataagagacag

SEQ ID NO: 448 - DNA, 66 bp, Artificial
  synthetic
  misc_feature (26)..(27): n is a, c, g, or t
caagcagaagacggcatacgagattnnattgtgtctcgtgggctcggagatgtgtataagagacag

SEQ ID NO: 449 - DNA, 66 bp, Artificial
  synthetic
  misc_feature (26)..(27): n is a, c, g, or t
caagcagaagacggcatacgagatgnnattgtgtctcgtgggctcggagatgtgtataagagacag

SEQ ID NO: 450 - DNA, 66 bp, Artificial
  synthetic
  misc_feature (26)..(27): n is a, c, g, or t
caagcagaagacggcatacgagatcnnattgtgtctcgtgggctcggagatgtgtataagagacag

SEQ ID NO: 451 - DNA, 66 bp, Artificial
  synthetic
caagcagaagacggcatacgagatctttgtgtgtctcgtgggctcggagatgtgtataagagacag

SEQ ID NO: 452 - DNA, 66 bp, Artificial
  synthetic
caagcagaagacggcatacgagatctctgtgtgtctcgtgggctcggagatgtgtataagagacag

SEQ ID NO: 453 - DNA, 66 bp, Artificial
  synthetic
  misc_feature (27)..(27): n is a, c, g, or t
caagcagaagacggcatacgagatcgntgtgtgtctcgtgggctcggagatgtgtataagagacag

SEQ ID NO: 454 - DNA, 66 bp, Artificial
  synthetic
  misc_feature (27)..(27): n is a, c, g, or t
caagcagaagacggcatacgagatccntgtgtgtctcgtgggctcggagatgtgtataagagacag

SEQ ID NO: 455 - DNA, 66 bp, Artificial
  synthetic
  misc_feature (27)..(27): n is a, c, g, or t
caagcagaagacggcatacgagatcantgtgtgtctcgtgggctcggagatgtgtataagagacag

SEQ ID NO: 456 - DNA, 66 bp, Artificial
  synthetic
caagcagaagacggcatacgagatctatgtgtgtctcgtgggctcggagatgtgtataagagacag

SEQ ID NO: 457 - DNA, 66 bp, Artificial
  synthetic
  misc_feature (27)..(27): n is a, c, g, or t
caagcagaagacggcatacgagattgnggtgtgtctcgtgggctcggagatgtgtataagagacag

SEQ ID NO: 458 - DNA, 66 bp, Artificial
  synthetic
  misc_feature (27)..(27): n is a, c, g, or t
caagcagaagacggcatacgagatggnggtgtgtctcgtgggctcggagatgtgtataagagacag

SEQ ID NO: 459 - DNA, 66 bp, Artificial
  synthetic
  misc_feature (27)..(27): n is a, c, g, or t
caagcagaagacggcatacgagattcnggtgtgtctcgtgggctcggagatgtgtataagagacag

SEQ ID NO: 460 - DNA, 66 bp, Artificial
  synthetic
  misc_feature (27)..(27): n is a, c, g, or t
caagcagaagacggcatacgagatgcnggtgtgtctcgtgggctcggagatgtgtataagagacag

SEQ ID NO: 461 - DNA, 66 bp, Artificial
  synthetic
  misc_feature (27)..(27): n is a, c, g, or t
caagcagaagacggcatacgagattanggtgtgtctcgtgggctcggagatgtgtataagagacag

SEQ ID NO: 462 - DNA, 66 bp, Artificial
  synthetic
  misc_feature (27)..(27): n is a, c, g, or t
caagcagaagacggcatacgagatganggtgtgtctcgtgggctcggagatgtgtataagagacag

SEQ ID NO: 463 - DNA, 66 bp, Artificial
  synthetic
  misc_feature (27)..(27): n is a, c, g, or t
caagcagaagacggcatacgagatagncgtgtgtctcgtgggctcggagatgtgtataagagacag

SEQ ID NO: 464 - DNA, 66 bp, Artificial
  synthetic
  misc_feature (27)..(27): n is a, c, g, or t
caagcagaagacggcatacgagatacncgtgtgtctcgtgggctcggagatgtgtataagagacag

SEQ ID NO: 465 - DNA, 66 bp, Artificial
  synthetic
  misc_feature (27)..(27): n is a, c, g, or t
caagcagaagacggcatacgagataancgtgtgtctcgtgggctcggagatgtgtataagagacag

SEQ ID NO: 466 - DNA, 66 bp, Artificial
  synthetic
  misc_feature (27)..(27): n is a, c, g, or t
caagcagaagacggcatacgagattgnagtgtgtctcgtgggctcggagatgtgtataagagacag

SEQ ID NO: 467 - DNA, 66 bp, Artificial
  synthetic
  misc_feature (27)..(27): n is a, c, g, or t
caagcagaagacggcatacgagatggnagtgtgtctcgtgggctcggagatgtgtataagagacag

SEQ ID NO: 468 - DNA, 66 bp, Artificial
  synthetic
  misc_feature (27)..(27): n is a, c, g, or t
caagcagaagacggcatacgagattcnagtgtgtctcgtgggctcggagatgtgtataagagacag

SEQ ID NO: 469 - DNA, 66 bp, Artificial
  synthetic
  misc_feature (27)..(27): n is a, c, g, or t
caagcagaagacggcatacgagatgcnagtgtgtctcgtgggctcggagatgtgtataagagacag

SEQ ID NO: 470 - DNA, 66 bp, Artificial
  synthetic
  misc_feature (27)..(27): n is a, c, g, or t
caagcagaagacggcatacgagattanagtgtgtctcgtgggctcggagatgtgtataagagacag

SEQ ID NO: 471 - DNA, 66 bp, Artificial
  synthetic
  misc_feature (27)..(27): n is a, c, g, or t
caagcagaagacggcatacgagatganagtgtgtctcgtgggctcggagatgtgtataagagacag

SEQ ID NO: 472 - DNA, 66 bp, Artificial
  synthetic
  misc_feature (27)..(27): n is a, c, g, or t
caagcagaagacggcatacgagatcgntctgtgtctcgtgggctcggagatgtgtataagagacag

SEQ ID NO: 473 - DNA, 66 bp, Artificial
  synthetic
  misc_feature (27)..(27): n is a, c, g, or t
caagcagaagacggcatacgagatccntctgtgtctcgtgggctcggagatgtgtataagagacag

SEQ ID NO: 474 - DNA, 66 bp, Artificial
  synthetic
  misc_feature (27)..(27): n is a, c, g, or t
caagcagaagacggcatacgagatcantctgtgtctcgtgggctcggagatgtgtataagagacag

SEQ ID NO: 475 - DNA, 66 bp, Artificial
  synthetic
  misc_feature (27)..(27): n is a, c, g, or t
caagcagaagacggcatacgagattgngctgtgtctcgtgggctcggagatgtgtataagagacag

SEQ ID NO: 476 - DNA, 66 bp, Artificial
  synthetic
  misc_feature (27)..(27): n is a, c, g, or t
caagcagaagacggcatacgagatggngctgtgtctcgtgggctcggagatgtgtataagagacag

SEQ ID NO: 477 - DNA, 66 bp, Artificial
  synthetic
  misc_feature (27)..(27): n is a, c, g, or t
caagcagaagacggcatacgagattcngctgtgtctcgtgggctcggagatgtgtataagagacag

SEQ ID NO: 478 - DNA, 66 bp, Artificial
  synthetic
  misc_feature (27)..(27): n is a, c, g, or t
caagcagaagacggcatacgagatgcngctgtgtctcgtgggctcggagatgtgtataagagacag

SEQ ID NO: 479 - DNA, 66 bp, Artificial
  synthetic
  misc_feature (27)..(27): n is a, c, g, or t
caagcagaagacggcatacgagattangctgtgtctcgtgggctcggagatgtgtataagagacag

SEQ ID NO: 480 - DNA, 66 bp, Artificial
  synthetic
  misc_feature (27)..(27): n is a, c, g, or t
caagcagaagacggcatacgagatgangctgtgtctcgtgggctcggagatgtgtataagagacag

SEQ ID NO: 481 - DNA, 66 bp, Artificial
  synthetic
  misc_feature (27)..(27): n is a, c, g, or t
caagcagaagacggcatacgagatagncctgtgtctcgtgggctcggagatgtgtataagagacag

SEQ ID NO: 482 - DNA, 66 bp, Artificial
  synthetic
  misc_feature (27)..(27): n is a, c, g, or t
caagcagaagacggcatacgagatacncctgtgtctcgtgggctcggagatgtgtataagagacag

SEQ ID NO: 483 - DNA, 66 bp, Artificial
  synthetic
  misc_feature (27)..(27): n is a, c, g, or t
caagcagaagacggcatacgagataancctgtgtctcgtgggctcggagatgtgtataagagacag

SEQ ID NO: 484 - DNA, 66 bp, Artificial
  synthetic
  misc_feature (27)..(27): n is a, c, g, or t
caagcagaagacggcatacgagattgnactgtgtctcgtgggctcggagatgtgtataagagacag

SEQ ID NO: 485 - DNA, 66 bp, Artificial
  synthetic
  misc_feature (27)..(27): n is a, c, g, or t
caagcagaagacggcatacgagatggnactgtgtctcgtgggctcggagatgtgtataagagacag

SEQ ID NO: 486 - DNA, 66 bp, Artificial
  synthetic
  misc_feature (27)..(27): n is a, c, g, or t
caagcagaagacggcatacgagattcnactgtgtctcgtgggctcggagatgtgtataagagacag

SEQ ID NO: 487 - DNA, 66 bp, Artificial
  synthetic
  misc_feature (27)..(27): n is a, c, g, or t
caagcagaagacggcatacgagatgcnactgtgtctcgtgggctcggagatgtgtataagagacag

SEQ ID NO: 488 - DNA, 66 bp, Artificial
  synthetic
  misc_feature (27)..(27): n is a, c, g, or t
caagcagaagacggcatacgagattanactgtgtctcgtgggctcggagatgtgtataagagacag

SEQ ID NO: 489 - DNA, 66 bp, Artificial
  synthetic
  misc_feature (27)..(27): n is a, c, g, or t
caagcagaagacggcatacgagatganactgtgtctcgtgggctcggagatgtgtataagagacag

SEQ ID NO: 490 - DNA, 66 bp, Artificial
  synthetic
  misc_feature (26)..(27): n is a, c, g, or t
  misc_feature (29)..(29): n is a, c, g, or t
caagcagaagacggcatacgagattnntntgtgtctcgtgggctcggagatgtgtataagagacag

SEQ ID NO: 491 - DNA, 66 bp, Artificial
  synthetic
  misc_feature (26)..(27): n is a, c, g, or t
  misc_feature (29)..(29): n is a, c, g, or t
caagcagaagacggcatacgagatgnntntgtgtctcgtgggctcggagatgtgtataagagacag

SEQ ID NO: 492 - DNA, 66 bp, Artificial
  synthetic
  misc_feature (26)..(27): n is a, c, g, or t
  misc_feature (29)..(29): n is a, c, g, or t
caagcagaagacggcatacgagatanngntgtgtctcgtgggctcggagatgtgtataagagacag

SEQ ID NO: 493 - DNA, 66 bp, Artificial
  synthetic
  misc_feature (26)..(27): n is a, c, g, or t
  misc_feature (29)..(29): n is a, c, g, or t
caagcagaagacggcatacgagatannantgtgtctcgtgggctcggagatgtgtataagagacag

SEQ ID NO: 494 - DNA, 66 bp, Artificial
  synthetic
  misc_feature (26)..(27): n is a, c, g, or t
caagcagaagacggcatacgagatcnntatgtgtctcgtgggctcggagatgtgtataagagacag

SEQ ID NO: 495 - DNA, 66 bp, Artificial
  synthetic
caagcagaagacggcatacgagatcgtgatgtgtctcgtgggctcggagatgtgtataagagacag

SEQ ID NO: 496 - DNA, 66 bp, Artificial
  synthetic
caagcagaagacggcatacgagatcatgatgtgtctcgtgggctcggagatgtgtataagagacag

SEQ ID NO: 497 - DNA, 66 bp, Artificial
  synthetic
caagcagaagacggcatacgagatcgcgatgtgtctcgtgggctcggagatgtgtataagagacag

SEQ ID NO: 498 - DNA, 66 bp, Artificial
  synthetic
caagcagaagacggcatacgagatcacgatgtgtctcgtgggctcggagatgtgtataagagacag

SEQ ID NO: 499 - DNA, 66 bp, Artificial
  synthetic
  misc_feature (27)..(27): n is a, c, g, or t
caagcagaagacggcatacgagatccngatgtgtctcgtgggctcggagatgtgtataagagacag

SEQ ID NO: 500 - DNA, 66 bp, Artificial
  synthetic
  misc_feature (26)..(27): n is a, c, g, or t
caagcagaagacggcatacgagattnngatgtgtctcgtgggctcggagatgtgtataagagacag

SEQ ID NO: 501 - DNA, 66 bp, Artificial
  synthetic
  misc_feature (26)..(27): n is a, c, g, or t
caagcagaagacggcatacgagatgnngatgtgtctcgtgggctcggagatgtgtataagagacag

SEQ ID NO: 502 - DNA, 66 bp, Artificial
  synthetic
caagcagaagacggcatacgagatcgagatgtgtctcgtgggctcggagatgtgtataagagacag

SEQ ID NO: 503 - DNA, 66 bp, Artificial
  synthetic
caagcagaagacggcatacgagatcaagatgtgtctcgtgggctcggagatgtgtataagagacag

SEQ ID NO: 504 - DNA, 66 bp, Artificial
  synthetic
  misc_feature (27)..(27): n is a, c, g, or t
caagcagaagacggcatacgagattgncatgtgtctcgtgggctcggagatgtgtataagagacag

SEQ ID NO: 505 - DNA, 66 bp, Artificial
  synthetic
  misc_feature (27)..(27): n is a, c, g, or t
caagcagaagacggcatacgagatggncatgtgtctcgtgggctcggagatgtgtataagagacag

SEQ ID NO: 506 - DNA, 66 bp, Artificial
  synthetic
  misc_feature (27)..(27): n is a, c, g, or t
caagcagaagacggcatacgagattcncatgtgtctcgtgggctcggagatgtgtataagagacag

SEQ ID NO: 507 - DNA, 66 bp, Artificial
  synthetic
  misc_feature (27)..(27): n is a, c, g, or t
caagcagaagacggcatacgagatgcncatgtgtctcgtgggctcggagatgtgtataagagacag

SEQ ID NO: 508 - DNA, 66 bp, Artificial
  synthetic
  misc_feature (26)..(27): n is a, c, g, or t
caagcagaagacggcatacgagatanncatgtgtctcgtgggctcggagatgtgtataagagacag

SEQ ID NO: 509 - DNA, 66 bp, Artificial
  synthetic
  misc_feature (27)..(27): n is a, c, g, or t
caagcagaagacggcatacgagattancatgtgtctcgtgggctcggagatgtgtataagagacag

SEQ ID NO: 510 - DNA, 66 bp, Artificial
  synthetic
  misc_feature (27)..(27): n is a, c, g, or t
caagcagaagacggcatacgagatgancatgtgtctcgtgggctcggagatgtgtataagagacag

SEQ ID NO: 511 - DNA, 66 bp, Artificial
  synthetic
caagcagaagacggcatacgagatcgtaatgtgtctcgtgggctcggagatgtgtataagagacag

SEQ ID NO: 512 - DNA, 66 bp, Artificial
  synthetic
caagcagaagacggcatacgagatcataatgtgtctcgtgggctcggagatgtgtataagagacag

SEQ ID NO: 513 - DNA, 66 bp, Artificial
  synthetic
caagcagaagacggcatacgagatcgcaatgtgtctcgtgggctcggagatgtgtataagagacag

SEQ ID NO: 514 - DNA, 66 bp, Artificial
  synthetic
caagcagaagacggcatacgagatcacaatgtgtctcgtgggctcggagatgtgtataagagacag

SEQ ID NO: 515 - DNA, 66 bp, Artificial
  synthetic
  misc_feature (27)..(27): n is a, c, g, or t
caagcagaagacggcatacgagatccnaatgtgtctcgtgggctcggagatgtgtataagagacag

SEQ ID NO: 516 - DNA, 66 bp, Artificial
  synthetic
  misc_feature (26)..(27): n is a, c, g, or t
caagcagaagacggcatacgagattnnaatgtgtctcgtgggctcggagatgtgtataagagacag

SEQ ID NO: 517 - DNA, 66 bp, Artificial
  synthetic
  misc_feature (26)..(27): n is a, c, g, or t
caagcagaagacggcatacgagatgnnaatgtgtctcgtgggctcggagatgtgtataagagacag

SEQ ID NO: 518 - DNA, 66 bp, Artificial
  synthetic
caagcagaagacggcatacgagatcgaaatgtgtctcgtgggctcggagatgtgtataagagacag

SEQ ID NO: 519 - DNA, 66 bp, Artificial
  synthetic
caagcagaagacggcatacgagatcaaaatgtgtctcgtgggctcggagatgtgtataagagacag

SEQ ID NO: 520 - DNA, 66 bp, Artificial
  synthetic
caagcagaagacggcatacgagatcttttggtgtctcgtgggctcggagatgtgtataagagacag

SEQ ID NO: 521 - DNA, 66 bp, Artificial
  synthetic
caagcagaagacggcatacgagatctcttggtgtctcgtgggctcggagatgtgtataagagacag

SEQ ID NO: 522 - DNA, 66 bp, Artificial
  synthetic
  misc_feature (27)..(27): n is a, c, g, or t
caagcagaagacggcatacgagatcgnttggtgtctcgtgggctcggagatgtgtataagagacag

SEQ ID NO: 523 - DNA, 66 bp, Artificial
  synthetic
  misc_feature (27)..(27): n is a, c, g, or t
caagcagaagacggcatacgagatccnttggtgtctcgtgggctcggagatgtgtataagagacag

SEQ ID NO: 524 - DNA, 66 bp, Artificial
  synthetic
  misc_feature (26)..(27): n is a, c, g, or t
caagcagaagacggcatacgagattnnttggtgtctcgtgggctcggagatgtgtataagagacag

SEQ ID NO: 525 - DNA, 66 bp, Artificial
  synthetic
  misc_feature (26)..(27): n is a, c, g, or t
caagcagaagacggcatacgagatgnnttggtgtctcgtgggctcggagatgtgtataagagacag

SEQ ID NO: 526 - DNA, 66 bp, Artificial
  synthetic
  misc_feature (27)..(27): n is a, c, g, or t
caagcagaagacggcatacgagatcanttggtgtctcgtgggctcggagatgtgtataagagacag

SEQ ID NO: 527 - DNA, 66 bp, Artificial
  synthetic
caagcagaagacggcatacgagatctattggtgtctcgtgggctcggagatgtgtataagagacag

SEQ ID NO: 528 - DNA, 66 bp, Artificial
  synthetic
  misc_feature (27)..(27): n is a, c, g, or t
caagcagaagacggcatacgagattgngtggtgtctcgtgggctcggagatgtgtataagagacag

SEQ ID NO: 529 - DNA, 66 bp, Artificial
  synthetic
  misc_feature (27)..(27): n is a, c, g, or t
caagcagaagacggcatacgagatggngtggtgtctcgtgggctcggagatgtgtataagagacag

SEQ ID NO: 530 - DNA, 66 bp, Artificial
  synthetic
  misc_feature (27)..(27): n is a, c, g, or t
caagcagaagacggcatacgagattcngtggtgtctcgtgggctcggagatgtgtataagagacag

SEQ ID NO: 531 - DNA, 66 bp, Artificial
  synthetic
  misc_feature (27)..(27): n is a, c, g, or t
caagcagaagacggcatacgagatgcngtggtgtctcgtgggctcggagatgtgtataagagacag

SEQ ID NO: 532 - DNA, 66 bp, Artificial
  synthetic
  misc_feature (26)..(27): n is a, c, g, or t
caagcagaagacggcatacgagatanngtggtgtctcgtgggctcggagatgtgtataagagacag

SEQ ID NO: 533 - DNA, 66 bp, Artificial
  synthetic
  misc_feature (27)..(27): n is a, c, g, or t
caagcagaagacggcatacgagattangtggtgtctcgtgggctcggagatgtgtataagagacag

SEQ ID NO: 534 - DNA, 66 bp, Artificial
  synthetic
  misc_feature (27)..(27): n is a, c, g, or t
caagcagaagacggcatacgagatgangtggtgtctcgtgggctcggagatgtgtataagagacag

SEQ ID NO: 535 - DNA, 66 bp, Artificial
  synthetic
caagcagaagacggcatacgagatattctggtgtctcgtgggctcggagatgtgtataagagacag

SEQ ID NO: 536 - DNA, 66 bp, Artificial
  synthetic
caagcagaagacggcatacgagatatcctggtgtctcgtgggctcggagatgtgtataagagacag

SEQ ID NO: 537 - DNA, 66 bp, Artificial
  synthetic
  misc_feature (27)..(27): n is a, c, g, or t
caagcagaagacggcatacgagatagnctggtgtctcgtgggctcggagatgtgtataagagacag

SEQ ID NO: 538 - DNA, 66 bp, Artificial
  synthetic
  misc_feature (27)..(27): n is a, c, g, or t
caagcagaagacggcatacgagatacnctggtgtctcgtgggctcggagatgtgtataagagacag

SEQ ID NO: 539 - DNA, 66 bp, Artificial
  synthetic
  misc_feature (27)..(27): n is a, c, g, or t
caagcagaagacggcatacgagataanctggtgtctcgtgggctcggagatgtgtataagagacag

SEQ ID NO: 540 - DNA, 66 bp, Artificial
  synthetic
caagcagaagacggcatacgagatatactggtgtctcgtgggctcggagatgtgtataagagacag

SEQ ID NO: 541 - DNA, 66 bp, Artificial
  synthetic
  misc_feature (27)..(27): n is a, c, g, or t
caagcagaagacggcatacgagattgnatggtgtctcgtgggctcggagatgtgtataagagacag

SEQ ID NO: 542 - DNA, 66 bp, Artificial
  synthetic
  misc_feature (27)..(27): n is a, c, g, or t
caagcagaagacggcatacgagatggnatggtgtctcgtgggctcggagatgtgtataagagacag

SEQ ID NO: 543 - DNA, 66 bp, Artificial
  synthetic
  misc_feature (27)..(27): n is a, c, g, or t
caagcagaagacggcatacgagattcnatggtgtctcgtgggctcggagatgtgtataagagacag

SEQ ID NO: 544 - DNA, 66 bp, Artificial
  synthetic
  misc_feature (27)..(27): n is a, c, g, or t
caagcagaagacggcatacgagatgcnatggtgtctcgtgggctcggagatgtgtataagagacag

SEQ ID NO: 545 - DNA, 66 bp, Artificial
  synthetic
  misc_feature (26)..(27): n is a, c, g, or t
caagcagaagacggcatacgagatannatggtgtctcgtgggctcggagatgtgtataagagacag

SEQ ID NO: 546 - DNA, 66 bp, Artificial
  synthetic
  misc_feature (27)..(27): n is a, c, g, or t
caagcagaagacggcatacgagattanatggtgtctcgtgggctcggagatgtgtataagagacag

SEQ ID NO: 547 - DNA, 66 bp, Artificial
  synthetic
  misc_feature (27)..(27): n is a, c, g, or t
caagcagaagacggcatacgagatganatggtgtctcgtgggctcggagatgtgtataagagacag

SEQ ID NO: 548 - DNA, 66 bp, Artificial
  synthetic
caagcagaagacggcatacgagattgttgggtgtctcgtgggctcggagatgtgtataagagacag

SEQ ID NO: 549 - DNA, 66 bp, Artificial
  synthetic
caagcagaagacggcatacgagatggttgggtgtctcgtgggctcggagatgtgtataagagacag

SEQ ID NO: 550 - DNA, 66 bp, Artificial
  synthetic
caagcagaagacggcatacgagattattgggtgtctcgtgggctcggagatgtgtataagagacag

SEQ ID NO: 551 - DNA, 66 bp, Artificial
  synthetic
caagcagaagacggcatacgagatgattgggtgtctcgtgggctcggagatgtgtataagagacag

SEQ ID NO: 552 - DNA, 66 bp, Artificial
  synthetic
caagcagaagacggcatacgagattgctgggtgtctcgtgggctcggagatgtgtataagagacag

SEQ ID NO: 553 - DNA, 66 bp, Artificial
  synthetic
caagcagaagacggcatacgagatggctgggtgtctcgtgggctcggagatgtgtataagagacag

SEQ ID NO: 554 - DNA, 66 bp, Artificial
  synthetic
caagcagaagacggcatacgagattactgggtgtctcgtgggctcggagatgtgtataagagacag

SEQ ID NO: 555 - DNA, 66 bp, Artificial
  synthetic
caagcagaagacggcatacgagatgactgggtgtctcgtgggctcggagatgtgtataagagacag

SEQ ID NO: 556 - DNA, 66 bp, Artificial
  synthetic
  misc_feature (27)..(27): n is a, c, g, or t
caagcagaagacggcatacgagattcntgggtgtctcgtgggctcggagatgtgtataagagacag

SEQ ID NO: 557 - DNA, 66 bp, Artificial
  synthetic
  misc_feature (27)..(27): n is a, c, g, or t
caagcagaagacggcatacgagatgcntgggtgtctcgtgggctcggagatgtgtataagagacag

SEQ ID NO: 558 - DNA, 66 bp, Artificial
  synthetic
caagcagaagacggcatacgagattgatgggtgtctcgtgggctcggagatgtgtataagagacag

SEQ ID NO: 559 - DNA, 66 bp, Artificial
  synthetic
caagcagaagacggcatacgagatggatgggtgtctcgtgggctcggagatgtgtataagagacag

SEQ ID NO: 560 - DNA, 66 bp, Artificial
  synthetic
caagcagaagacggcatacgagattaatgggtgtctcgtgggctcggagatgtgtataagagacag

SEQ ID NO: 561 - DNA, 66 bp, Artificial
  synthetic
caagcagaagacggcatacgagatgaatgggtgtctcgtgggctcggagatgtgtataagagacag

SEQ ID NO: 562 - DNA, 66 bp, Artificial
  synthetic
  misc_feature (27)..(27): n is a, c, g, or t
caagcagaagacggcatacgagattcntcggtgtctcgtgggctcggagatgtgtataagagacag

SEQ ID NO: 563 - DNA, 66 bp, Artificial
  synthetic
  misc_feature (27)..(27): n is a, c, g, or t
caagcagaagacggcatacgagatgcntcggtgtctcgtgggctcggagatgtgtataagagacag

SEQ ID NO: 564 - DNA, 66 bp, Artificial
  synthetic
  misc_feature (26)..(27): n is a, c, g, or t
caagcagaagacggcatacgagattnntaggtgtctcgtgggctcggagatgtgtataagagacag

SEQ ID NO: 565 - DNA, 66 bp, Artificial
  synthetic
  misc_feature (26)..(27): n is a, c, g, or t
caagcagaagacggcatacgagatgnntaggtgtctcgtgggctcggagatgtgtataagagacag

SEQ ID NO: 566 - DNA, 66 bp, Artificial
  synthetic
  misc_feature (27)..(27): n is a, c, g, or t
caagcagaagacggcatacgagatagngaggtgtctcgtgggctcggagatgtgtataagagacag

SEQ ID NO: 567 - DNA, 66 bp, Artificial
  synthetic
  misc_feature (27)..(27): n is a, c, g, or t
caagcagaagacggcatacgagatacngaggtgtctcgtgggctcggagatgtgtataagagacag

SEQ ID NO: 568 - DNA, 66 bp, Artificial
  synthetic
  misc_feature (27)..(27): n is a, c, g, or t
caagcagaagacggcatacgagataangaggtgtctcgtgggctcggagatgtgtataagagacag

SEQ ID NO: 569 - DNA, 66 bp, Artificial
  synthetic
  misc_feature (27)..(27): n is a, c, g, or t
caagcagaagacggcatacgagatagnaaggtgtctcgtgggctcggagatgtgtataagagacag

SEQ ID NO: 570 - DNA, 66 bp, Artificial
  synthetic
  misc_feature (27)..(27): n is a, c, g, or t
caagcagaagacggcatacgagatacnaaggtgtctcgtgggctcggagatgtgtataagagacag

SEQ ID NO: 571 - DNA, 66 bp, Artificial
  synthetic
  misc_feature (27)..(27): n is a, c, g, or t
caagcagaagacggcatacgagataanaaggtgtctcgtgggctcggagatgtgtataagagacag

SEQ ID NO: 572 - DNA, 66 bp, Artificial
  synthetic
  misc_feature (27)..(27): n is a, c, g, or t
caagcagaagacggcatacgagatcgnttcgtgtctcgtgggctcggagatgtgtataagagacag

SEQ ID NO: 573 - DNA, 66 bp, Artificial
  synthetic
  misc_feature (27)..(27): n is a, c, g, or t
caagcagaagacggcatacgagatccnttcgtgtctcgtgggctcggagatgtgtataagagacag

SEQ ID NO: 574 - DNA, 66 bp, Artificial
  synthetic
  misc_feature (26)..(27): n is a, c, g, or t
caagcagaagacggcatacgagattnnttcgtgtctcgtgggctcggagatgtgtataagagacag

SEQ ID NO: 575 - DNA, 66 bp, Artificial
  synthetic
  misc_feature (26)..(27): n is a, c, g, or t
caagcagaagacggcatacgagatgnnttcgtgtctcgtgggctcggagatgtgtataagagacag

SEQ ID NO: 576 - DNA, 66 bp, Artificial
  synthetic
  misc_feature (27)..(27): n is a, c, g, or t
caagcagaagacggcatacgagatcanttcgtgtctcgtgggctcggagatgtgtataagagacag

SEQ ID NO: 577 - DNA, 66 bp, Artificial
  synthetic
  misc_feature (27)..(27): n is a, c, g, or t
caagcagaagacggcatacgagattgngtcgtgtctcgtgggctcggagatgtgtataagagacag

SEQ ID NO: 578 - DNA, 66 bp, Artificial
  synthetic
  misc_feature (27)..(27): n is a, c, g, or t
caagcagaagacggcatacgagatggngtcgtgtctcgtgggctcggagatgtgtataagagacag

SEQ ID NO: 579 - DNA, 66 bp, Artificial
  synthetic
  misc_feature (27)..(27): n is a, c, g, or t
caagcagaagacggcatacgagattcngtcgtgtctcgtgggctcggagatgtgtataagagacag

SEQ ID NO: 580 - DNA, 66 bp, Artificial
  synthetic
  misc_feature (27)..(27): n is a, c, g, or t
caagcagaagacggcatacgagatgcngtcgtgtctcgtgggctcggagatgtgtataagagacag

SEQ ID NO: 581 - DNA, 66 bp, Artificial
  synthetic
  misc_feature (26)..(27): n is a, c, g, or t
caagcagaagacggcatacgagatanngtcgtgtctcgtgggctcggagatgtgtataagagacag

SEQ ID NO: 582 - DNA, 66 bp, Artificial
  synthetic
  misc_feature (27)..(27): n is a, c, g, or t
caagcagaagacggcatacgagattangtcgtgtctcgtgggctcggagatgtgtataagagacag

SEQ ID NO: 583 - DNA, 66 bp, Artificial
  synthetic
  misc_feature (27)..(27): n is a, c, g, or t
caagcagaagacggcatacgagatgangtcgtgtctcgtgggctcggagatgtgtataagagacag

SEQ ID NO: 584 - DNA, 66 bp, Artificial
  synthetic
  misc_feature (27)..(27): n is a, c, g, or t
caagcagaagacggcatacgagatagnctcgtgtctcgtgggctcggagatgtgtataagagacag

SEQ ID NO: 585 - DNA, 66 bp, Artificial
  synthetic
  misc_feature (27)..(27): n is a, c, g, or t
caagcagaagacggcatacgagatacnctcgtgtctcgtgggctcggagatgtgtataagagacag

SEQ ID NO: 586 - DNA, 66 bp, Artificial
  synthetic
  misc_feature (27)..(27): n is a, c, g, or t
caagcagaagacggcatacgagataanctcgtgtctcgtgggctcggagatgtgtataagagacag

SEQ ID NO: 587 - DNA, 66 bp, Artificial
  synthetic
  misc_feature (27)..(27): n is a, c, g, or t
caagcagaagacggcatacgagattgnatcgtgtctcgtgggctcggagatgtgtataagagacag

SEQ ID NO: 588 - DNA, 66 bp, Artificial
  synthetic
  misc_feature (27)..(27): n is a, c, g, or t
caagcagaagacggcatacgagatggnatcgtgtctcgtgggctcggagatgtgtataagagacag

SEQ ID NO: 589 - DNA, 66 bp, Artificial
  synthetic
  misc_feature (27)..(27): n is a, c, g, or t
caagcagaagacggcatacgagattcnatcgtgtctcgtgggctcggagatgtgtataagagacag

SEQ ID NO: 590 - DNA, 66 bp, Artificial
  synthetic
  misc_feature (27)..(27): n is a, c, g, or t
caagcagaagacggcatacgagatgcnatcgtgtctcgtgggctcggagatgtgtataagagacag

SEQ ID NO: 591 - DNA, 66 bp, Artificial
  synthetic
  misc_feature (26)..(27): n is a, c, g, or t
caagcagaagacggcatacgagatannatcgtgtctcgtgggctcggagatgtgtataagagacag

SEQ ID NO: 592 - DNA, 66 bp, Artificial
  synthetic
  misc_feature (27)..(27): n is a, c, g, or t
caagcagaagacggcatacgagattanatcgtgtctcgtgggctcggagatgtgtataagagacag

SEQ ID NO: 593 - DNA, 66 bp, Artificial
  synthetic
  misc_feature (27)..(27): n is a, c, g, or t
caagcagaagacggcatacgagatganatcgtgtctcgtgggctcggagatgtgtataagagacag

SEQ ID NO: 594 - DNA, 66 bp, Artificial
  synthetic
caagcagaagacggcatacgagattcttgcgtgtctcgtgggctcggagatgtgtataagagacag

SEQ ID NO: 595 - DNA, 66 bp, Artificial
  synthetic
caagcagaagacggcatacgagatgcttgcgtgtctcgtgggctcggagatgtgtataagagacag

SEQ ID NO: 596 - DNA, 66 bp, Artificial
  synthetic
caagcagaagacggcatacgagattcctgcgtgtctcgtgggctcggagatgtgtataagagacag

SEQ ID NO: 597 - DNA, 66 bp, Artificial
  synthetic
caagcagaagacggcatacgagatgcctgcgtgtctcgtgggctcggagatgtgtataagagacag

SEQ ID NO: 598 - DNA, 66 bp, Artificial
  synthetic
caagcagaagacggcatacgagattcatgcgtgtctcgtgggctcggagatgtgtataagagacag

SEQ ID NO: 599 - DNA, 66 bp, Artificial
  synthetic
caagcagaagacggcatacgagatgcatgcgtgtctcgtgggctcggagatgtgtataagagacag

SEQ ID NO: 600 - DNA, 66 bp, Artificial
  synthetic
caagcagaagacggcatacgagattcttccgtgtctcgtgggctcggagatgtgtataagagacag

SEQ ID NO: 601 - DNA, 66 bp, Artificial
  synthetic
caagcagaagacggcatacgagatgcttccgtgtctcgtgggctcggagatgtgtataagagacag

SEQ ID NO: 602 - DNA, 66 bp, Artificial
  synthetic
caagcagaagacggcatacgagattcctccgtgtctcgtgggctcggagatgtgtataagagacag

SEQ ID NO: 603 - DNA, 66 bp, Artificial
  synthetic
caagcagaagacggcatacgagatgcctccgtgtctcgtgggctcggagatgtgtataagagacag

SEQ ID NO: 604 - DNA, 66 bp, Artificial
  synthetic
caagcagaagacggcatacgagattcatccgtgtctcgtgggctcggagatgtgtataagagacag

SEQ ID NO: 605 - DNA, 66 bp, Artificial
  synthetic
caagcagaagacggcatacgagatgcatccgtgtctcgtgggctcggagatgtgtataagagacag

SEQ ID NO: 606 - DNA, 66 bp, Artificial
  synthetic
  misc_feature (26)..(27): n is a, c, g, or t
caagcagaagacggcatacgagattnntacgtgtctcgtgggctcggagatgtgtataagagacag

SEQ ID NO: 607 - DNA, 66 bp, Artificial
  synthetic
  misc_feature (26)..(27): n is a, c, g, or t
caagcagaagacggcatacgagatgnntacgtgtctcgtgggctcggagatgtgtataagagacag

SEQ ID NO: 608 - DNA, 66 bp, Artificial
  synthetic
  misc_feature (27)..(27): n is a, c, g, or t
caagcagaagacggcatacgagatagngacgtgtctcgtgggctcggagatgtgtataagagacag

SEQ ID NO: 609 - DNA, 66 bp, Artificial
  synthetic
  misc_feature (27)..(27): n is a, c, g, or t
caagcagaagacggcatacgagatacngacgtgtctcgtgggctcggagatgtgtataagagacag

SEQ ID NO: 610 - DNA, 66 bp, Artificial
  synthetic
  misc_feature (27)..(27): n is a, c, g, or t
caagcagaagacggcatacgagataangacgtgtctcgtgggctcggagatgtgtataagagacag

SEQ ID NO: 611 - DNA, 66 bp, Artificial
  synthetic
  misc_feature (27)..(27): n is a, c, g, or t
caagcagaagacggcatacgagatagnaacgtgtctcgtgggctcggagatgtgtataagagacag

SEQ ID NO: 612 - DNA, 66 bp, Artificial
  synthetic
  misc_feature (27)..(27): n is a, c, g, or t
caagcagaagacggcatacgagatacnaacgtgtctcgtgggctcggagatgtgtataagagacag

SEQ ID NO: 613 - DNA, 66 bp, Artificial
  synthetic
  misc_feature (27)..(27): n is a, c, g, or t
caagcagaagacggcatacgagataanaacgtgtctcgtgggctcggagatgtgtataagagacag

SEQ ID NO: 614 - DNA, 66 bp, Artificial
  synthetic
  misc_feature (26)..(27): n is a, c, g, or t
  misc_feature (29)..(30): n is a, c, g, or t
caagcagaagacggcatacgagatanntnngtgtctcgtgggctcggagatgtgtataagagacag

SEQ ID NO: 615 - DNA, 66 bp, Artificial
  synthetic
  misc_feature (26)..(27): n is a, c, g, or t
caagcagaagacggcatacgagatcnnttagtgtctcgtgggctcggagatgtgtataagagacag

SEQ ID NO: 616 - DNA, 66 bp, Artificial
  synthetic
  misc_feature (27)..(27): n is a, c, g, or t
caagcagaagacggcatacgagatcgngtagtgtctcgtgggctcggagatgtgtataagagacag

SEQ ID NO: 617 - DNA, 66 bp, Artificial
  synthetic
  misc_feature (27)..(27): n is a, c, g, or t
caagcagaagacggcatacgagatccngtagtgtctcgtgggctcggagatgtgtataagagacag

SEQ ID NO: 618 - DNA, 66 bp, Artificial
  synthetic
  misc_feature (26)..(27): n is a, c, g, or t
caagcagaagacggcatacgagattnngtagtgtctcgtgggctcggagatgtgtataagagacag

SEQ ID NO: 619 - DNA, 66 bp, Artificial
  synthetic
  misc_feature (26)..(27): n is a, c, g, or t
caagcagaagacggcatacgagatgnngtagtgtctcgtgggctcggagatgtgtataagagacag

SEQ ID NO: 620 - DNA, 66 bp, Artificial
  synthetic
  misc_feature (26)..(27): n is a, c, g, or t
caagcagaagacggcatacgagatanngtagtgtctcgtgggctcggagatgtgtataagagacag

SEQ ID NO: 621 - DNA, 66 bp, Artificial
  synthetic
  misc_feature (27)..(27): n is a, c, g, or t
caagcagaagacggcatacgagatcangtagtgtctcgtgggctcggagatgtgtataagagacag

SEQ ID NO: 622 - DNA, 66 bp, Artificial
  synthetic
  misc_feature (27)..(27): n is a, c, g, or t
caagcagaagacggcatacgagattgnctagtgtctcgtgggctcggagatgtgtataagagacag

SEQ ID NO: 623 - DNA, 66 bp, Artificial
  synthetic
  misc_feature (27)..(27): n is a, c, g, or t
caagcagaagacggcatacgagatggnctagtgtctcgtgggctcggagatgtgtataagagacag

SEQ ID NO: 624 - DNA, 66 bp, Artificial
  synthetic
  misc_feature (27)..(27): n is a, c, g, or t
caagcagaagacggcatacgagattcnctagtgtctcgtgggctcggagatgtgtataagagacag

SEQ ID NO: 625 - DNA, 66 bp, Artificial
  synthetic
  misc_feature (27)..(27): n is a, c, g, or t
caagcagaagacggcatacgagatgcnctagtgtctcgtgggctcggagatgtgtataagagacag

SEQ ID NO: 626 - DNA, 66 bp, Artificial
  synthetic
  misc_feature (26)..(27): n is a, c, g, or t
caagcagaagacggcatacgagatannctagtgtctcgtgggctcggagatgtgtataagagacag

SEQ ID NO: 627 - DNA, 66 bp, Artificial
  synthetic
  misc_feature (27)..(27): n is a, c, g, or t
caagcagaagacggcatacgagattanctagtgtctcgtgggctcggagatgtgtataagagacag

SEQ ID NO: 628 - DNA, 66 bp, Artificial
  synthetic
  misc_feature (27)..(27): n is a, c, g, or t
caagcagaagacggcatacgagatganctagtgtctcgtgggctcggagatgtgtataagagacag

SEQ ID NO: 629 - DNA, 66 bp, Artificial
  synthetic
  misc_feature (27)..(27): n is a, c, g, or t
caagcagaagacggcatacgagatcgnatagtgtctcgtgggctcggagatgtgtataagagacag

SEQ ID NO: 630 - DNA, 66 bp, Artificial
  synthetic
  misc_feature (27)..(27): n is a, c, g, or t
caagcagaagacggcatacgagatccnatagtgtctcgtgggctcggagatgtgtataagagacag

SEQ ID NO: 631 - DNA, 66 bp, Artificial
  synthetic
  misc_feature (26)..(27): n is a, c, g, or t
caagcagaagacggcatacgagattnnatagtgtctcgtgggctcggagatgtgtataagagacag

SEQ ID NO: 632 - DNA, 66 bp, Artificial
  synthetic
  misc_feature (26)..(27): n is a, c, g, or t
caagcagaagacggcatacgagatgnnatagtgtctcgtgggctcggagatgtgtataagagacag

SEQ ID NO: 633 - DNA, 66 bp, Artificial
  synthetic
  misc_feature (26)..(27): n is a, c, g, or t
caagcagaagacggcatacgagatannatagtgtctcgtgggctcggagatgtgtataagagacag

SEQ ID NO: 634 - DNA, 66 bp, Artificial
  synthetic
  misc_feature (27)..(27): n is a, c, g, or t
caagcagaagacggcatacgagatcanatagtgtctcgtgggctcggagatgtgtataagagacag

SEQ ID NO: 635 - DNA, 66 bp, Artificial
  synthetic
  misc_feature (27)..(27): n is a, c, g, or t
caagcagaagacggcatacgagatagnggagtgtctcgtgggctcggagatgtgtataagagacag

SEQ ID NO: 636 - DNA, 66 bp, Artificial
  synthetic
  misc_feature (27)..(27): n is a, c, g, or t
caagcagaagacggcatacgagatacnggagtgtctcgtgggctcggagatgtgtataagagacag

SEQ ID NO: 637 - DNA, 66 bp, Artificial
  synthetic
  misc_feature (27)..(27): n is a, c, g, or t
caagcagaagacggcatacgagataanggagtgtctcgtgggctcggagatgtgtataagagacag

SEQ ID NO: 638 - DNA, 66 bp, Artificial
  synthetic
  misc_feature (27)..(27): n is a, c, g, or t
caagcagaagacggcatacgagatagnagagtgtctcgtgggctcggagatgtgtataagagacag

SEQ ID NO: 639 - DNA, 66 bp, Artificial
  synthetic
  misc_feature (27)..(27): n is a, c, g, or t
caagcagaagacggcatacgagatacnagagtgtctcgtgggctcggagatgtgtataagagacag

SEQ ID NO: 640 - DNA, 66 bp, Artificial
  synthetic
  misc_feature (27)..(27): n is a, c, g, or t
caagcagaagacggcatacgagataanagagtgtctcgtgggctcggagatgtgtataagagacag

SEQ ID NO: 641 - DNA, 66 bp, Artificial
  synthetic
  misc_feature (27)..(27): n is a, c, g, or t
caagcagaagacggcatacgagatagngcagtgtctcgtgggctcggagatgtgtataagagacag

SEQ ID NO: 642 - DNA, 66 bp, Artificial
  synthetic
  misc_feature (27)..(27): n is a, c, g, or t
caagcagaagacggcatacgagatacngcagtgtctcgtgggctcggagatgtgtataagagacag

SEQ ID NO: 643 - DNA, 66 bp, Artificial
  synthetic
  misc_feature (27)..(27): n is a, c, g, or t
caagcagaagacggcatacgagataangcagtgtctcgtgggctcggagatgtgtataagagacag

SEQ ID NO: 644 - DNA, 66 bp, Artificial
  synthetic
  misc_feature (27)..(27): n is a, c, g, or t
caagcagaagacggcatacgagatagnacagtgtctcgtgggctcggagatgtgtataagagacag

SEQ ID NO: 645 - DNA, 66 bp, Artificial
  synthetic
  misc_feature (27)..(27): n is a, c, g, or t
caagcagaagacggcatacgagatacnacagtgtctcgtgggctcggagatgtgtataagagacag

SEQ ID NO: 646 - DNA, 66 bp, Artificial
  synthetic
  misc_feature (27)..(27): n is a, c, g, or t
caagcagaagacggcatacgagataanacagtgtctcgtgggctcggagatgtgtataagagacag

SEQ ID NO: 647 - DNA, 66 bp, Artificial
  synthetic
  misc_feature (26)..(27): n is a, c, g, or t
  misc_feature (29)..(29): n is a, c, g, or t
caagcagaagacggcatacgagattnntnagtgtctcgtgggctcggagatgtgtataagagacag

SEQ ID NO: 648 - DNA, 66 bp, Artificial
  synthetic
  misc_feature (26)..(27): n is a, c, g, or t
  misc_feature (29)..(29): n is a, c, g, or t
caagcagaagacggcatacgagatgnntnagtgtctcgtgggctcggagatgtgtataagagacag

SEQ ID NO: 649 - DNA, 66 bp, Artificial
  synthetic
  misc_feature (27)..(27): n is a, c, g, or t
caagcagaagacggcatacgagatcgntaagtgtctcgtgggctcggagatgtgtataagagacag

SEQ ID NO: 650 - DNA, 66 bp, Artificial
  synthetic
  misc_feature (27)..(27): n is a, c, g, or t
caagcagaagacggcatacgagatccntaagtgtctcgtgggctcggagatgtgtataagagacag

SEQ ID NO: 651 - DNA, 66 bp, Artificial
  synthetic
  misc_feature (27)..(27): n is a, c, g, or t
caagcagaagacggcatacgagatcantaagtgtctcgtgggctcggagatgtgtataagagacag

SEQ ID NO: 652 - DNA, 66 bp, Artificial
  synthetic
  misc_feature (27)..(27): n is a, c, g, or t
caagcagaagacggcatacgagattgngaagtgtctcgtgggctcggagatgtgtataagagacag

SEQ ID NO: 653 - DNA, 66 bp, Artificial
  synthetic
  misc_feature (27)..(27): n is a, c, g, or t
caagcagaagacggcatacgagatggngaagtgtctcgtgggctcggagatgtgtataagagacag

SEQ ID NO: 654 - DNA, 66 bp, Artificial
  synthetic
  misc_feature (27)..(27): n is a, c, g, or t
caagcagaagacggcatacgagattcngaagtgtctcgtgggctcggagatgtgtataagagacag

SEQ ID NO: 655 - DNA, 66 bp, Artificial
  synthetic
  misc_feature (27)..(27): n is a, c, g, or t
caagcagaagacggcatacgagatgcngaagtgtctcgtgggctcggagatgtgtataagagacag

SEQ ID NO: 656 - DNA, 66 bp, Artificial
  synthetic
  misc_feature (26)..(27): n is a, c, g, or t
caagcagaagacggcatacgagatanngaagtgtctcgtgggctcggagatgtgtataagagacag

SEQ ID NO: 657 - DNA, 66 bp, Artificial
  synthetic
  misc_feature (27)..(27): n is a, c, g, or t
caagcagaagacggcatacgagattangaagtgtctcgtgggctcggagatgtgtataagagacag

SEQ ID NO: 658 - DNA, 66 bp, Artificial
  synthetic
  misc_feature (27)..(27): n is a, c, g, or t
caagcagaagacggcatacgagatgangaagtgtctcgtgggctcggagatgtgtataagagacag

SEQ ID NO: 659 - DNA, 66 bp, Artificial
  synthetic
  misc_feature (27)..(27): n is a, c, g, or t
caagcagaagacggcatacgagatagncaagtgtctcgtgggctcggagatgtgtataagagacag

SEQ ID NO: 660 - DNA, 66 bp, Artificial
  synthetic
  misc_feature (27)..(27): n is a, c, g, or t
caagcagaagacggcatacgagatacncaagtgtctcgtgggctcggagatgtgtataagagacag

SEQ ID NO: 661 - DNA, 66 bp, Artificial
  synthetic
  misc_feature (27)..(27): n is a, c, g, or t
caagcagaagacggcatacgagataancaagtgtctcgtgggctcggagatgtgtataagagacag

SEQ ID NO: 662 - DNA, 66 bp, Artificial
  synthetic
  misc_feature (27)..(27): n is a, c, g, or t
caagcagaagacggcatacgagattgnaaagtgtctcgtgggctcggagatgtgtataagagacag

SEQ ID NO: 663 - DNA, 66 bp, Artificial
  synthetic
  misc_feature (27)..(27): n is a, c, g, or t
caagcagaagacggcatacgagatggnaaagtgtctcgtgggctcggagatgtgtataagagacag

SEQ ID NO: 664 - DNA, 66 bp, Artificial
  synthetic
  misc_feature (27)..(27): n is a, c, g, or t
caagcagaagacggcatacgagattcnaaagtgtctcgtgggctcggagatgtgtataagagacag

SEQ ID NO: 665 - DNA, 66 bp, Artificial
  synthetic
  misc_feature (27)..(27): n is a, c, g, or t
caagcagaagacggcatacgagatgcnaaagtgtctcgtgggctcggagatgtgtataagagacag

SEQ ID NO: 666 - DNA, 66 bp, Artificial
  synthetic
  misc_feature (26)..(27): n is a, c, g, or t
caagcagaagacggcatacgagatannaaagtgtctcgtgggctcggagatgtgtataagagacag

SEQ ID NO: 667 - DNA, 66 bp, Artificial
  synthetic
  misc_feature (27)..(27): n is a, c, g, or t
caagcagaagacggcatacgagattanaaagtgtctcgtgggctcggagatgtgtataagagacag

SEQ ID NO: 668 - DNA, 66 bp, Artificial
  synthetic
  misc_feature (27)..(27): n is a, c, g, or t
caagcagaagacggcatacgagatganaaagtgtctcgtgggctcggagatgtgtataagagacag

SEQ ID NO: 669 - DNA, 66 bp, Artificial
  synthetic
caagcagaagacggcatacgagatctttttctgtctcgtgggctcggagatgtgtataagagacag

SEQ ID NO: 670 - DNA, 66 bp, Artificial
  synthetic
caagcagaagacggcatacgagatctctttctgtctcgtgggctcggagatgtgtataagagacag

SEQ ID NO: 671 - DNA, 66 bp, Artificial
  synthetic
  misc_feature (27)..(27): n is a, c, g, or t
caagcagaagacggcatacgagatcgntttctgtctcgtgggctcggagatgtgtataagagacag

SEQ ID NO: 672 - DNA, 66 bp, Artificial
  synthetic
  misc_feature (27)..(27): n is a, c, g, or t
caagcagaagacggcatacgagatccntttctgtctcgtgggctcggagatgtgtataagagacag

SEQ ID NO: 673 - DNA, 66 bp, Artificial
  synthetic
  misc_feature (26)..(27): n is a, c, g, or t
caagcagaagacggcatacgagattnntttctgtctcgtgggctcggagatgtgtataagagacag

SEQ ID NO: 674 - DNA, 66 bp, Artificial
  synthetic
  misc_feature (26)..(27): n is a, c, g, or t
caagcagaagacggcatacgagatgnntttctgtctcgtgggctcggagatgtgtataagagacag

SEQ ID NO: 675 - DNA, 66 bp, Artificial
  synthetic
  misc_feature (27)..(27): n is a, c, g, or t
caagcagaagacggcatacgagatcantttctgtctcgtgggctcggagatgtgtataagagacag

SEQ ID NO: 676 - DNA, 66 bp, Artificial
  synthetic
caagcagaagacggcatacgagatctatttctgtctcgtgggctcggagatgtgtataagagacag

SEQ ID NO: 677 - DNA, 66 bp, Artificial
  synthetic
  misc_feature (27)..(27): n is a, c, g, or t
caagcagaagacggcatacgagattgngttctgtctcgtgggctcggagatgtgtataagagacag

SEQ ID NO: 678 - DNA, 66 bp, Artificial
  synthetic
  misc_feature (27)..(27): n is a, c, g, or t
caagcagaagacggcatacgagatggngttctgtctcgtgggctcggagatgtgtataagagacag

SEQ ID NO: 679 - DNA, 66 bp, Artificial
  synthetic
  misc_feature (27)..(27): n is a, c, g, or t
caagcagaagacggcatacgagattcngttctgtctcgtgggctcggagatgtgtataagagacag

SEQ ID NO: 680 - DNA, 66 bp, Artificial
  synthetic
  misc_feature (27)..(27): n is a, c, g, or t
caagcagaagacggcatacgagatgcngttctgtctcgtgggctcggagatgtgtataagagacag

SEQ ID NO: 681 - DNA, 66 bp, Artificial
  synthetic
  misc_feature (26)..(27): n is a, c, g, or t
caagcagaagacggcatacgagatanngttctgtctcgtgggctcggagatgtgtataagagacag

SEQ ID NO: 682 - DNA, 66 bp, Artificial
  synthetic
  misc_feature (27)..(27): n is a, c, g, or t
caagcagaagacggcatacgagattangttctgtctcgtgggctcggagatgtgtataagagacag

SEQ ID NO: 683 - DNA, 66 bp, Artificial
  synthetic
  misc_feature (27)..(27): n is a, c, g, or t
caagcagaagacggcatacgagatgangttctgtctcgtgggctcggagatgtgtataagagacag

SEQ ID NO: 684 - DNA, 66 bp, Artificial
  synthetic
  misc_feature (27)..(27): n is a, c, g, or t
caagcagaagacggcatacgagatagncttctgtctcgtgggctcggagatgtgtataagagacag

SEQ ID NO: 685 - DNA, 66 bp, Artificial
  synthetic
  misc_feature (27)..(27): n is a, c, g, or t
caagcagaagacggcatacgagatacncttctgtctcgtgggctcggagatgtgtataagagacag

SEQ ID NO: 686 - DNA, 66 bp, Artificial
  synthetic
  misc_feature (27)..(27): n is a, c, g, or t
caagcagaagacggcatacgagataancttctgtctcgtgggctcggagatgtgtataagagacag

SEQ ID NO: 687 - DNA, 66 bp, Artificial
  synthetic
  misc_feature (27)..(27): n is a, c, g, or t
caagcagaagacggcatacgagattgnattctgtctcgtgggctcggagatgtgtataagagacag

SEQ ID NO: 688 - DNA, 66 bp, Artificial
  synthetic
  misc_feature (27)..(27): n is a, c, g, or t
caagcagaagacggcatacgagatggnattctgtctcgtgggctcggagatgtgtataagagacag

SEQ ID NO: 689 - DNA, 66 bp, Artificial
  synthetic
  misc_feature (27)..(27): n is a, c, g, or t
caagcagaagacggcatacgagattcnattctgtctcgtgggctcggagatgtgtataagagacag

SEQ ID NO: 690 - DNA, 66 bp, Artificial
  synthetic
  misc_feature (27)..(27): n is a, c, g, or t
caagcagaagacggcatacgagatgcnattctgtctcgtgggctcggagatgtgtataagagacag

SEQ ID NO: 691 - DNA, 66 bp, Artificial
  synthetic
  misc_feature (26)..(27): n is a, c, g, or t
caagcagaagacggcatacgagatannattctgtctcgtgggctcggagatgtgtataagagacag

SEQ ID NO: 692 - DNA, 66 bp, Artificial
  synthetic
  misc_feature (27)..(27): n is a, c, g, or t
caagcagaagacggcatacgagattanattctgtctcgtgggctcggagatgtgtataagagacag

SEQ ID NO: 693 - DNA, 66 bp, Artificial
  synthetic
  misc_feature (27)..(27): n is a, c, g, or t
caagcagaagacggcatacgagatganattctgtctcgtgggctcggagatgtgtataagagacag

SEQ ID NO: 694 - DNA, 66 bp, Artificial
  synthetic
  misc_feature (27)..(27): n is a, c, g, or t
caagcagaagacggcatacgagattcntgtctgtctcgtgggctcggagatgtgtataagagacag

SEQ ID NO: 695 - DNA, 66 bp, Artificial
  synthetic
  misc_feature (27)..(27): n is a, c, g, or t
caagcagaagacggcatacgagatgcntgtctgtctcgtgggctcggagatgtgtataagagacag

SEQ ID NO: 696 - DNA, 66 bp, Artificial
  synthetic
caagcagaagacggcatacgagattcttctctgtctcgtgggctcggagatgtgtataagagacag

SEQ ID NO: 697 - DNA, 66 bp, Artificial
  synthetic
caagcagaagacggcatacgagatgcttctctgtctcgtgggctcggagatgtgtataagagacag

SEQ ID NO: 698 - DNA, 66 bp, Artificial
  synthetic
caagcagaagacggcatacgagattcctctctgtctcgtgggctcggagatgtgtataagagacag

SEQ ID NO: 699 - DNA, 66 bp, Artificial
  synthetic
caagcagaagacggcatacgagatgcctctctgtctcgtgggctcggagatgtgtataagagacag

SEQ ID NO: 700 - DNA, 66 bp, Artificial
  synthetic
caagcagaagacggcatacgagattcatctctgtctcgtgggctcggagatgtgtataagagacag

SEQ ID NO: 701 - DNA, 66 bp, Artificial
  synthetic
caagcagaagacggcatacgagatgcatctctgtctcgtgggctcggagatgtgtataagagacag

SEQ ID NO: 702 - DNA, 66 bp, Artificial
  synthetic
  misc_feature (26)..(27): n is a, c, g, or t
  misc_feature (29)..(29): n is a, c, g, or t
caagcagaagacggcatacgagatanntntctgtctcgtgggctcggagatgtgtataagagacag

SEQ ID NO: 703 - DNA, 66 bp, Artificial
  synthetic
  misc_feature (26)..(27): n is a, c, g, or t
caagcagaagacggcatacgagattnntatctgtctcgtgggctcggagatgtgtataagagacag

SEQ ID NO: 704 - DNA, 66 bp, Artificial
  synthetic
  misc_feature (26)..(27): n is a, c, g, or t
caagcagaagacggcatacgagatgnntatctgtctcgtgggctcggagatgtgtataagagacag

SEQ ID NO: 705 - DNA, 66 bp, Artificial
  synthetic
  misc_feature (27)..(27): n is a, c, g, or t
caagcagaagacggcatacgagatagngatctgtctcgtgggctcggagatgtgtataagagacag

SEQ ID NO: 706 - DNA, 66 bp, Artificial
  synthetic
  misc_feature (27)..(27): n is a, c, g, or t
caagcagaagacggcatacgagatacngatctgtctcgtgggctcggagatgtgtataagagacag

SEQ ID NO: 707 - DNA, 66 bp, Artificial
  synthetic
  misc_feature (27)..(27): n is a, c, g, or t
caagcagaagacggcatacgagataangatctgtctcgtgggctcggagatgtgtataagagacag

SEQ ID NO: 708 - DNA, 66 bp, Artificial
  synthetic
  misc_feature (27)..(27): n is a, c, g, or t
caagcagaagacggcatacgagatagnaatctgtctcgtgggctcggagatgtgtataagagacag

SEQ ID NO: 709 - DNA, 66 bp, Artificial
  synthetic
  misc_feature (27)..(27): n is a, c, g, or t
caagcagaagacggcatacgagatacnaatctgtctcgtgggctcggagatgtgtataagagacag

SEQ ID NO: 710 - DNA, 66 bp, Artificial
  synthetic
  misc_feature (27)..(27): n is a, c, g, or t
caagcagaagacggcatacgagataanaatctgtctcgtgggctcggagatgtgtataagagacag

SEQ ID NO: 711 - DNA, 66 bp, Artificial
  synthetic
caagcagaagacggcatacgagattgtttgctgtctcgtgggctcggagatgtgtataagagacag

SEQ ID NO: 712 - DNA, 66 bp, Artificial
  synthetic
caagcagaagacggcatacgagatggtttgctgtctcgtgggctcggagatgtgtataagagacag

SEQ ID NO: 713 - DNA, 66 bp, Artificial
  synthetic
caagcagaagacggcatacgagattatttgctgtctcgtgggctcggagatgtgtataagagacag

SEQ ID NO: 714 - DNA, 66 bp, Artificial
  synthetic
caagcagaagacggcatacgagatgatttgctgtctcgtgggctcggagatgtgtataagagacag

SEQ ID NO: 715 - DNA, 66 bp, Artificial
  synthetic
caagcagaagacggcatacgagattgcttgctgtctcgtgggctcggagatgtgtataagagacag

SEQ ID NO: 716 - DNA, 66 bp, Artificial
  synthetic
caagcagaagacggcatacgagatggcttgctgtctcgtgggctcggagatgtgtataagagacag

SEQ ID NO: 717 - DNA, 66 bp, Artificial
  synthetic
caagcagaagacggcatacgagattacttgctgtctcgtgggctcggagatgtgtataagagacag

SEQ ID NO: 718 - DNA, 66 bp, Artificial
  synthetic
caagcagaagacggcatacgagatgacttgctgtctcgtgggctcggagatgtgtataagagacag

SEQ ID NO: 719 - DNA, 66 bp, Artificial
  synthetic
  misc_feature (27)..(27): n is a, c, g, or t
caagcagaagacggcatacgagattcnttgctgtctcgtgggctcggagatgtgtataagagacag

SEQ ID NO: 720 - DNA, 66 bp, Artificial
  synthetic
  misc_feature (27)..(27): n is a, c, g, or t
caagcagaagacggcatacgagatgcnttgctgtctcgtgggctcggagatgtgtataagagacag

SEQ ID NO: 721 - DNA, 66 bp, Artificial
  synthetic
  misc_feature (26)..(27): n is a, c, g, or t
caagcagaagacggcatacgagatannttgctgtctcgtgggctcggagatgtgtataagagacag

SEQ ID NO: 722 - DNA, 66 bp, Artificial
  synthetic
caagcagaagacggcatacgagattgattgctgtctcgtgggctcggagatgtgtataagagacag

SEQ ID NO: 723 - DNA, 66 bp, Artificial
  synthetic
caagcagaagacggcatacgagatggattgctgtctcgtgggctcggagatgtgtataagagacag

SEQ ID NO: 724 - DNA, 66 bp, Artificial
  synthetic
caagcagaagacggcatacgagattaattgctgtctcgtgggctcggagatgtgtataagagacag

SEQ ID NO: 725 - DNA, 66 bp, Artificial
  synthetic
caagcagaagacggcatacgagatgaattgctgtctcgtgggctcggagatgtgtataagagacag

SEQ ID NO: 726 - DNA, 66 bp, Artificial
  synthetic
  misc_feature (27)..(27): n is a, c, g, or t
caagcagaagacggcatacgagatacntagctgtctcgtgggctcggagatgtgtataagagacag

SEQ ID NO: 727 - DNA, 66 bp, Artificial
  synthetic
  misc_feature (27)..(27): n is a, c, g, or t
caagcagaagacggcatacgagattcnttcctgtctcgtgggctcggagatgtgtataagagacag

SEQ ID NO: 728 - DNA, 66 bp, Artificial
  synthetic
  misc_feature (27)..(27): n is a, c, g, or t
caagcagaagacggcatacgagatgcnttcctgtctcgtgggctcggagatgtgtataagagacag

SEQ ID NO: 729 - DNA, 66 bp, Artificial
  synthetic
  misc_feature (26)..(27): n is a, c, g, or t
caagcagaagacggcatacgagatannttcctgtctcgtgggctcggagatgtgtataagagacag

SEQ ID NO: 730 - DNA, 66 bp, Artificial
  synthetic
caagcagaagacggcatacgagatacttacctgtctcgtgggctcggagatgtgtataagagacag

SEQ ID NO: 731 - DNA, 66 bp, Artificial
  synthetic
caagcagaagacggcatacgagatacctacctgtctcgtgggctcggagatgtgtataagagacag

SEQ ID NO: 732 - DNA, 66 bp, Artificial
  synthetic
caagcagaagacggcatacgagatacatacctgtctcgtgggctcggagatgtgtataagagacag

SEQ ID NO: 733 - DNA, 66 bp, Artificial
  synthetic
  misc_feature (26)..(27): n is a, c, g, or t
caagcagaagacggcatacgagattnnttactgtctcgtgggctcggagatgtgtataagagacag

SEQ ID NO: 734 - DNA, 66 bp, Artificial
  synthetic
  misc_feature (26)..(27): n is a, c, g, or t
caagcagaagacggcatacgagatgnnttactgtctcgtgggctcggagatgtgtataagagacag

SEQ ID NO: 735 - DNA, 66 bp, Artificial
  synthetic
  misc_feature (26)..(27): n is a, c, g, or t
caagcagaagacggcatacgagatannttactgtctcgtgggctcggagatgtgtataagagacag

SEQ ID NO: 736 - DNA, 66 bp, Artificial
  synthetic
  misc_feature (27)..(27): n is a, c, g, or t
caagcagaagacggcatacgagatagngtactgtctcgtgggctcggagatgtgtataagagacag

SEQ ID NO: 737 - DNA, 66 bp, Artificial
  synthetic
  misc_feature (27)..(27): n is a, c, g, or t
caagcagaagacggcatacgagatacngtactgtctcgtgggctcggagatgtgtataagagacag

SEQ ID NO: 738 - DNA, 66 bp, Artificial
  synthetic
  misc_feature (27)..(27): n is a, c, g, or t
caagcagaagacggcatacgagataangtactgtctcgtgggctcggagatgtgtataagagacag

SEQ ID NO: 739 - DNA, 66 bp, Artificial
  synthetic
caagcagaagacggcatacgagatatagtactgtctcgtgggctcggagatgtgtataagagacag

SEQ ID NO: 740 - DNA, 66 bp, Artificial
  synthetic
  misc_feature (27)..(27): n is a, c, g, or t
caagcagaagacggcatacgagatagnatactgtctcgtgggctcggagatgtgtataagagacag

SEQ ID NO: 741 - DNA, 66 bp, Artificial
  synthetic
  misc_feature (27)..(27): n is a, c, g, or t
caagcagaagacggcatacgagatacnatactgtctcgtgggctcggagatgtgtataagagacag

SEQ ID NO: 742 - DNA, 66 bp, Artificial
  synthetic
  misc_feature (27)..(27): n is a, c, g, or t
caagcagaagacggcatacgagataanatactgtctcgtgggctcggagatgtgtataagagacag

SEQ ID NO: 743 - DNA, 66 bp, Artificial
  synthetic
caagcagaagacggcatacgagatataatactgtctcgtgggctcggagatgtgtataagagacag

SEQ ID NO: 744 - DNA, 66 bp, Artificial
  synthetic
caagcagaagacggcatacgagatagttgactgtctcgtgggctcggagatgtgtataagagacag

SEQ ID NO: 745 - DNA, 66 bp, Artificial
  synthetic
caagcagaagacggcatacgagataattgactgtctcgtgggctcggagatgtgtataagagacag

SEQ ID NO: 746 - DNA, 66 bp, Artificial
  synthetic
caagcagaagacggcatacgagatagctgactgtctcgtgggctcggagatgtgtataagagacag

SEQ ID NO: 747 - DNA, 66 bp, Artificial
  synthetic
caagcagaagacggcatacgagataactgactgtctcgtgggctcggagatgtgtataagagacag

SEQ ID NO: 748 - DNA, 66 bp, Artificial
  synthetic
  misc_feature (27)..(27): n is a, c, g, or t
caagcagaagacggcatacgagatacntgactgtctcgtgggctcggagatgtgtataagagacag

SEQ ID NO: 749 - DNA, 66 bp, Artificial
  synthetic
caagcagaagacggcatacgagatagatgactgtctcgtgggctcggagatgtgtataagagacag

SEQ ID NO: 750 - DNA, 66 bp, Artificial
  synthetic
caagcagaagacggcatacgagataaatgactgtctcgtgggctcggagatgtgtataagagacag

SEQ ID NO: 751 - DNA, 66 bp, Artificial
  synthetic
  misc_feature (27)..(27): n is a, c, g, or t
caagcagaagacggcatacgagatacntcactgtctcgtgggctcggagatgtgtataagagacag

SEQ ID NO: 752 - DNA, 66 bp, Artificial
  synthetic
caagcagaagacggcatacgagattcttaactgtctcgtgggctcggagatgtgtataagagacag

SEQ ID NO: 753 - DNA, 66 bp, Artificial
  synthetic
caagcagaagacggcatacgagatgcttaactgtctcgtgggctcggagatgtgtataagagacag

SEQ ID NO: 754 - DNA, 66 bp, Artificial
  synthetic
caagcagaagacggcatacgagattcctaactgtctcgtgggctcggagatgtgtataagagacag

SEQ ID NO: 755 - DNA, 66 bp, Artificial
  synthetic
caagcagaagacggcatacgagatgcctaactgtctcgtgggctcggagatgtgtataagagacag

SEQ ID NO: 756 - DNA, 66 bp, Artificial
  synthetic
  misc_feature (26)..(27): n is a, c, g, or t
caagcagaagacggcatacgagatanntaactgtctcgtgggctcggagatgtgtataagagacag

SEQ ID NO: 757 - DNA, 66 bp, Artificial
  synthetic
caagcagaagacggcatacgagattcataactgtctcgtgggctcggagatgtgtataagagacag

SEQ ID NO: 758 - DNA, 66 bp, Artificial
  synthetic
caagcagaagacggcatacgagatgcataactgtctcgtgggctcggagatgtgtataagagacag

SEQ ID NO: 759 - DNA, 66 bp, Artificial
  synthetic
  misc_feature (26)..(27): n is a, c, g, or t
caagcagaagacggcatacgagatcnncttatgtctcgtgggctcggagatgtgtataagagacag

SEQ ID NO: 760 - DNA, 66 bp, Artificial
  synthetic
  misc_feature (27)..(27): n is a, c, g, or t
caagcagaagacggcatacgagatccncgtatgtctcgtgggctcggagatgtgtataagagacag

SEQ ID NO: 761 - DNA, 66 bp, Artificial
  synthetic
caagcagaagacggcatacgagatcctcctatgtctcgtgggctcggagatgtgtataagagacag

SEQ ID NO: 762 - DNA, 66 bp, Artificial
  synthetic
caagcagaagacggcatacgagatccccctatgtctcgtgggctcggagatgtgtataagagacag

SEQ ID NO: 763 - DNA, 66 bp, Artificial
  synthetic
caagcagaagacggcatacgagatccacctatgtctcgtgggctcggagatgtgtataagagacag

SEQ ID NO: 764 - DNA, 66 bp, Artificial
  synthetic
  misc_feature (25)..(27): n is a, c, g, or t
  misc_feature (29)..(29): n is a, c, g, or t
caagcagaagacggcatacgagatnnntntatgtctcgtgggctcggagatgtgtataagagacag

SEQ ID NO: 765 - DNA, 66 bp, Artificial
  synthetic
  misc_feature (25)..(27): n is a, c, g, or t
  misc_feature (29)..(29): n is a, c, g, or t
caagcagaagacggcatacgagatnnngntatgtctcgtgggctcggagatgtgtataagagacag

SEQ ID NO: 766 - DNA, 66 bp, Artificial
  synthetic
  misc_feature (26)..(27): n is a, c, g, or t
  misc_feature (29)..(29): n is a, c, g, or t
caagcagaagacggcatacgagattnncntatgtctcgtgggctcggagatgtgtataagagacag

SEQ ID NO: 767 - DNA, 66 bp, Artificial
  synthetic
  misc_feature (26)..(27): n is a, c, g, or t
  misc_feature (29)..(29): n is a, c, g, or t
caagcagaagacggcatacgagatgnncntatgtctcgtgggctcggagatgtgtataagagacag

SEQ ID NO: 768 - DNA, 66 bp, Artificial
  synthetic
  misc_feature (26)..(27): n is a, c, g, or t
  misc_feature (29)..(29): n is a, c, g, or t
caagcagaagacggcatacgagatanncntatgtctcgtgggctcggagatgtgtataagagacag

SEQ ID NO: 769 - DNA, 66 bp, Artificial
  synthetic
  misc_feature (25)..(27): n is a, c, g, or t
  misc_feature (29)..(29): n is a, c, g, or t
caagcagaagacggcatacgagatnnnantatgtctcgtgggctcggagatgtgtataagagacag

SEQ ID NO: 770 - DNA, 66 bp, Artificial
  synthetic
  misc_feature (26)..(27): n is a, c, g, or t
caagcagaagacggcatacgagatcnncatatgtctcgtgggctcggagatgtgtataagagacag

SEQ ID NO: 771 - DNA, 66 bp, Artificial
  synthetic
  misc_feature (26)..(27): n is a, c, g, or t
caagcagaagacggcatacgagatcnnttgatgtctcgtgggctcggagatgtgtataagagacag

SEQ ID NO: 772 - DNA, 66 bp, Artificial
  synthetic
  misc_feature (26)..(27): n is a, c, g, or t
caagcagaagacggcatacgagattnngtgatgtctcgtgggctcggagatgtgtataagagacag

SEQ ID NO: 773 - DNA, 66 bp, Artificial
  synthetic
  misc_feature (26)..(27): n is a, c, g, or t
caagcagaagacggcatacgagatgnngtgatgtctcgtgggctcggagatgtgtataagagacag

SEQ ID NO: 774 - DNA, 66 bp, Artificial
  synthetic
  misc_feature (26)..(27): n is a, c, g, or t
caagcagaagacggcatacgagatcnngtgatgtctcgtgggctcggagatgtgtataagagacag

SEQ ID NO: 775 - DNA, 66 bp, Artificial
  synthetic
caagcagaagacggcatacgagatcgtctgatgtctcgtgggctcggagatgtgtataagagacag

SEQ ID NO: 776 - DNA, 66 bp, Artificial
  synthetic
caagcagaagacggcatacgagatcatctgatgtctcgtgggctcggagatgtgtataagagacag

SEQ ID NO: 777 - DNA, 66 bp, Artificial
  synthetic
caagcagaagacggcatacgagatcgcctgatgtctcgtgggctcggagatgtgtataagagacag

SEQ ID NO: 778 - DNA, 66 bp, Artificial
  synthetic
caagcagaagacggcatacgagatcacctgatgtctcgtgggctcggagatgtgtataagagacag

SEQ ID NO: 779 - DNA, 66 bp, Artificial
  synthetic
  misc_feature (27)..(27): n is a, c, g, or t
caagcagaagacggcatacgagatccnctgatgtctcgtgggctcggagatgtgtataagagacag

SEQ ID NO: 780 - DNA, 66 bp, Artificial
  synthetic
  misc_feature (26)..(27): n is a, c, g, or t
caagcagaagacggcatacgagattnnctgatgtctcgtgggctcggagatgtgtataagagacag

SEQ ID NO: 781 - DNA, 66 bp, Artificial
  synthetic
  misc_feature (26)..(27): n is a, c, g, or t
caagcagaagacggcatacgagatgnnctgatgtctcgtgggctcggagatgtgtataagagacag

SEQ ID NO: 782 - DNA, 66 bp, Artificial
  synthetic
  misc_feature (26)..(27): n is a, c, g, or t
caagcagaagacggcatacgagatannctgatgtctcgtgggctcggagatgtgtataagagacag

SEQ ID NO: 783 - DNA, 66 bp, Artificial
  synthetic
caagcagaagacggcatacgagatcgactgatgtctcgtgggctcggagatgtgtataagagacag

SEQ ID NO: 784 - DNA, 66 bp, Artificial
  synthetic
caagcagaagacggcatacgagatcaactgatgtctcgtgggctcggagatgtgtataagagacag

SEQ ID NO: 785 - DNA, 66 bp, Artificial
  synthetic
  misc_feature (26)..(27): n is a, c, g, or t
caagcagaagacggcatacgagattnnatgatgtctcgtgggctcggagatgtgtataagagacag

SEQ ID NO: 786 - DNA, 66 bp, Artificial
  synthetic
  misc_feature (26)..(27): n is a, c, g, or t
caagcagaagacggcatacgagatgnnatgatgtctcgtgggctcggagatgtgtataagagacag

SEQ ID NO: 787 - DNA, 66 bp, Artificial
  synthetic
  misc_feature (26)..(27): n is a, c, g, or t
caagcagaagacggcatacgagatcnnatgatgtctcgtgggctcggagatgtgtataagagacag

SEQ ID NO: 788 - DNA, 66 bp, Artificial
  synthetic
  misc_feature (27)..(27): n is a, c, g, or t
caagcagaagacggcatacgagatcgntggatgtctcgtgggctcggagatgtgtataagagacag

SEQ ID NO: 789 - DNA, 66 bp, Artificial
  synthetic
  misc_feature (27)..(27): n is a, c, g, or t
caagcagaagacggcatacgagatccntggatgtctcgtgggctcggagatgtgtataagagacag

SEQ ID NO: 790 - DNA, 66 bp, Artificial
  synthetic
  misc_feature (27)..(27): n is a, c, g, or t
caagcagaagacggcatacgagatcantggatgtctcgtgggctcggagatgtgtataagagacag

SEQ ID NO: 791 - DNA, 66 bp, Artificial
  synthetic
  misc_feature (27)..(27): n is a, c, g, or t
caagcagaagacggcatacgagattgngggatgtctcgtgggctcggagatgtgtataagagacag

SEQ ID NO: 792 - DNA, 66 bp, Artificial
  synthetic
  misc_feature (27)..(27): n is a, c, g, or t
caagcagaagacggcatacgagatggngggatgtctcgtgggctcggagatgtgtataagagacag

SEQ ID NO: 793 - DNA, 66 bp, Artificial
  synthetic
  misc_feature (27)..(27): n is a, c, g, or t
caagcagaagacggcatacgagattcngggatgtctcgtgggctcggagatgtgtataagagacag

SEQ ID NO: 794 - DNA, 66 bp, Artificial
  synthetic
  misc_feature (27)..(27): n is a, c, g, or t
caagcagaagacggcatacgagatgcngggatgtctcgtgggctcggagatgtgtataagagacag

SEQ ID NO: 795 - DNA, 66 bp, Artificial
  synthetic
  misc_feature (27)..(27): n is a, c, g, or t
caagcagaagacggcatacgagattangggatgtctcgtgggctcggagatgtgtataagagacag

SEQ ID NO: 796 - DNA, 66 bp, Artificial
  synthetic
  misc_feature (27)..(27): n is a, c, g, or t
caagcagaagacggcatacgagatgangggatgtctcgtgggctcggagatgtgtataagagacag

SEQ ID NO: 797 - DNA, 66 bp, Artificial
  synthetic
  misc_feature (27)..(27): n is a, c, g, or t
caagcagaagacggcatacgagatagncggatgtctcgtgggctcggagatgtgtataagagacag

SEQ ID NO: 798 - DNA, 66 bp, Artificial
  synthetic
  misc_feature (27)..(27): n is a, c, g, or t
caagcagaagacggcatacgagatacncggatgtctcgtgggctcggagatgtgtataagagacag

SEQ ID NO: 799 - DNA, 66 bp, Artificial
  synthetic
  misc_feature (27)..(27): n is a, c, g, or t
caagcagaagacggcatacgagataancggatgtctcgtgggctcggagatgtgtataagagacag

SEQ ID NO: 800 - DNA, 66 bp, Artificial
  synthetic
  misc_feature (27)..(27): n is a, c, g, or t
caagcagaagacggcatacgagattgnaggatgtctcgtgggctcggagatgtgtataagagacag

SEQ ID NO: 801 - DNA, 66 bp, Artificial
  synthetic
  misc_feature (27)..(27): n is a, c, g, or t
caagcagaagacggcatacgagatggnaggatgtctcgtgggctcggagatgtgtataagagacag

SEQ ID NO: 802 - DNA, 66 bp, Artificial
  synthetic
  misc_feature (27)..(27): n is a, c, g, or t
caagcagaagacggcatacgagattcnaggatgtctcgtgggctcggagatgtgtataagagacag

SEQ ID NO: 803 - DNA, 66 bp, Artificial
  synthetic
  misc_feature (27)..(27): n is a, c, g, or t
caagcagaagacggcatacgagatgcnaggatgtctcgtgggctcggagatgtgtataagagacag

SEQ ID NO: 804 - DNA, 66 bp, Artificial
  synthetic
  misc_feature (27)..(27): n is a, c, g, or t
caagcagaagacggcatacgagattanaggatgtctcgtgggctcggagatgtgtataagagacag

SEQ ID NO: 805 - DNA, 66 bp, Artificial
  synthetic
  misc_feature (27)..(27): n is a, c, g, or t
caagcagaagacggcatacgagatganaggatgtctcgtgggctcggagatgtgtataagagacag

SEQ ID NO: 806 - DNA, 66 bp, Artificial
  synthetic
  misc_feature (27)..(27): n is a, c, g, or t
caagcagaagacggcatacgagatcgntcgatgtctcgtgggctcggagatgtgtataagagacag

SEQ ID NO: 807 - DNA, 66 bp, Artificial
  synthetic
  misc_feature (27)..(27): n is a, c, g, or t
caagcagaagacggcatacgagatccntcgatgtctcgtgggctcggagatgtgtataagagacag

SEQ ID NO: 808 - DNA, 66 bp, Artificial
  synthetic
  misc_feature (27)..(27): n is a, c, g, or t
caagcagaagacggcatacgagatcantcgatgtctcgtgggctcggagatgtgtataagagacag

SEQ ID NO: 809 - DNA, 66 bp, Artificial
  synthetic
  misc_feature (27)..(27): n is a, c, g, or t
caagcagaagacggcatacgagattgngcgatgtctcgtgggctcggagatgtgtataagagacag

SEQ ID NO: 810 - DNA, 66 bp, Artificial
  synthetic
  misc_feature (27)..(27): n is a, c, g, or t
caagcagaagacggcatacgagatggngcgatgtctcgtgggctcggagatgtgtataagagacag

SEQ ID NO: 811 - DNA, 66 bp, Artificial
  synthetic
  misc_feature (27)..(27): n is a, c, g, or t
caagcagaagacggcatacgagattcngcgatgtctcgtgggctcggagatgtgtataagagacag

SEQ ID NO: 812 - DNA, 66 bp, Artificial
  synthetic
  misc_feature (27)..(27): n is a, c, g, or t
caagcagaagacggcatacgagatgcngcgatgtctcgtgggctcggagatgtgtataagagacag

SEQ ID NO: 813 - DNA, 66 bp, Artificial
  synthetic
  misc_feature (27)..(27): n is a, c, g, or t
caagcagaagacggcatacgagattangcgatgtctcgtgggctcggagatgtgtataagagacag

SEQ ID NO: 814 - DNA, 66 bp, Artificial
  synthetic
  misc_feature (27)..(27): n is a, c, g, or t
caagcagaagacggcatacgagatgangcgatgtctcgtgggctcggagatgtgtataagagacag

SEQ ID NO: 815 - DNA, 66 bp, Artificial
  synthetic
  misc_feature (27)..(27): n is a, c, g, or t
caagcagaagacggcatacgagatagnccgatgtctcgtgggctcggagatgtgtataagagacag

SEQ ID NO: 816 - DNA, 66 bp, Artificial
  synthetic
  misc_feature (27)..(27): n is a, c, g, or t
caagcagaagacggcatacgagatacnccgatgtctcgtgggctcggagatgtgtataagagacag

SEQ ID NO: 817 - DNA, 66 bp, Artificial
  synthetic
  misc_feature (27)..(27): n is a, c, g, or t
caagcagaagacggcatacgagataanccgatgtctcgtgggctcggagatgtgtataagagacag

SEQ ID NO: 818 - DNA, 66 bp, Artificial
  synthetic
  misc_feature (27)..(27): n is a, c, g, or t
caagcagaagacggcatacgagattgnacgatgtctcgtgggctcggagatgtgtataagagacag

SEQ ID NO: 819 - DNA, 66 bp, Artificial
  synthetic
  misc_feature (27)..(27): n is a, c, g, or t
caagcagaagacggcatacgagatggnacgatgtctcgtgggctcggagatgtgtataagagacag

SEQ ID NO: 820 - DNA, 66 bp, Artificial
  synthetic
  misc_feature (27)..(27): n is a, c, g, or t
caagcagaagacggcatacgagattcnacgatgtctcgtgggctcggagatgtgtataagagacag

SEQ ID NO: 821 - DNA, 66 bp, Artificial
  synthetic
  misc_feature (27)..(27): n is a, c, g, or t
caagcagaagacggcatacgagatgcnacgatgtctcgtgggctcggagatgtgtataagagacag

SEQ ID NO: 822 - DNA, 66 bp, Artificial
  synthetic
  misc_feature (27)..(27): n is a, c, g, or t
caagcagaagacggcatacgagattanacgatgtctcgtgggctcggagatgtgtataagagacag

SEQ ID NO: 823 - DNA, 66 bp, Artificial
  synthetic
  misc_feature (27)..(27): n is a, c, g, or t
caagcagaagacggcatacgagatganacgatgtctcgtgggctcggagatgtgtataagagacag

SEQ ID NO: 824 - DNA, 66 bp, Artificial
  synthetic
  misc_feature (26)..(27): n is a, c, g, or t
  misc_feature (29)..(29): n is a, c, g, or t
caagcagaagacggcatacgagattnntngatgtctcgtgggctcggagatgtgtataagagacag

SEQ ID NO: 825 - DNA, 66 bp, Artificial
  synthetic
  misc_feature (26)..(27): n is a, c, g, or t
  misc_feature (29)..(29): n is a, c, g, or t
caagcagaagacggcatacgagatgnntngatgtctcgtgggctcggagatgtgtataagagacag

SEQ ID NO: 826 - DNA, 66 bp, Artificial
  synthetic
  misc_feature (26)..(27): n is a, c, g, or t
  misc_feature (29)..(29): n is a, c, g, or t
caagcagaagacggcatacgagatanntngatgtctcgtgggctcggagatgtgtataagagacag

SEQ ID NO: 827 - DNA, 66 bp, Artificial
  synthetic
  misc_feature (26)..(27): n is a, c, g, or t
  misc_feature (29)..(29): n is a, c, g, or t
caagcagaagacggcatacgagatanngngatgtctcgtgggctcggagatgtgtataagagacag

SEQ ID NO: 828 - DNA, 66 bp, Artificial
  synthetic
  misc_feature (26)..(27): n is a, c, g, or t
  misc_feature (29)..(29): n is a, c, g, or t
caagcagaagacggcatacgagatannangatgtctcgtgggctcggagatgtgtataagagacag

SEQ ID NO: 829 - DNA, 66 bp, Artificial
  synthetic
  misc_feature (26)..(27): n is a, c, g, or t
caagcagaagacggcatacgagatcnntagatgtctcgtgggctcggagatgtgtataagagacag

SEQ ID NO: 830 - DNA, 66 bp, Artificial
  synthetic
  misc_feature (27)..(27): n is a, c, g, or t
caagcagaagacggcatacgagatccngagatgtctcgtgggctcggagatgtgtataagagacag

SEQ ID NO: 831 - DNA, 66 bp, Artificial
  synthetic
  misc_feature (26)..(27): n is a, c, g, or t
caagcagaagacggcatacgagattnngagatgtctcgtgggctcggagatgtgtataagagacag

SEQ ID NO: 832 - DNA, 66 bp, Artificial
  synthetic
  misc_feature (26)..(27): n is a, c, g, or t
caagcagaagacggcatacgagatgnngagatgtctcgtgggctcggagatgtgtataagagacag

SEQ ID NO: 833 - DNA, 66 bp, Artificial
  synthetic
  misc_feature (27)..(27): n is a, c, g, or t
caagcagaagacggcatacgagattgncagatgtctcgtgggctcggagatgtgtataagagacag

SEQ ID NO: 834 - DNA, 66 bp, Artificial
  synthetic
  misc_feature (27)..(27): n is a, c, g, or t
caagcagaagacggcatacgagatggncagatgtctcgtgggctcggagatgtgtataagagacag

SEQ ID NO: 835 - DNA, 66 bp, Artificial
  synthetic
  misc_feature (27)..(27): n is a, c, g, or t
caagcagaagacggcatacgagattcncagatgtctcgtgggctcggagatgtgtataagagacag

SEQ ID NO: 836 - DNA, 66 bp, Artificial
  synthetic
  misc_feature (27)..(27): n is a, c, g, or t
caagcagaagacggcatacgagatgcncagatgtctcgtgggctcggagatgtgtataagagacag

SEQ ID NO: 837 - DNA, 66 bp, Artificial
  synthetic
  misc_feature (26)..(27): n is a, c, g, or t
caagcagaagacggcatacgagatanncagatgtctcgtgggctcggagatgtgtataagagacag

SEQ ID NO: 838 - DNA, 66 bp, Artificial
  synthetic
  misc_feature (27)..(27): n is a, c, g, or t
caagcagaagacggcatacgagattancagatgtctcgtgggctcggagatgtgtataagagacag

SEQ ID NO: 839 - DNA, 66 bp, Artificial
  synthetic
  misc_feature (27)..(27): n is a, c, g, or t
caagcagaagacggcatacgagatgancagatgtctcgtgggctcggagatgtgtataagagacag

SEQ ID NO: 840 - DNA, 66 bp, Artificial
  synthetic
  misc_feature (27)..(27): n is a, c, g, or t
caagcagaagacggcatacgagatccnaagatgtctcgtgggctcggagatgtgtataagagacag

SEQ ID NO: 841 - DNA, 66 bp, Artificial
  synthetic
  misc_feature (26)..(27): n is a, c, g, or t
caagcagaagacggcatacgagattnnaagatgtctcgtgggctcggagatgtgtataagagacag

SEQ ID NO: 842 - DNA, 66 bp, Artificial
  synthetic
  misc_feature (26)..(27): n is a, c, g, or t
caagcagaagacggcatacgagatgnnaagatgtctcgtgggctcggagatgtgtataagagacag

SEQ ID NO: 843 - DNA, 66 bp, Artificial
  synthetic
  misc_feature (26)..(27): n is a, c, g, or t
caagcagaagacggcatacgagatcnnttcatgtctcgtgggctcggagatgtgtataagagacag

SEQ ID NO: 844 - DNA, 66 bp, Artificial
  synthetic
  misc_feature (26)..(27): n is a, c, g, or t
caagcagaagacggcatacgagattnngtcatgtctcgtgggctcggagatgtgtataagagacag

SEQ ID NO: 845 - DNA, 66 bp, Artificial
  synthetic
  misc_feature (26)..(27): n is a, c, g, or t
caagcagaagacggcatacgagatgnngtcatgtctcgtgggctcggagatgtgtataagagacag

SEQ ID NO: 846 - DNA, 66 bp, Artificial
  synthetic
  misc_feature (26)..(27): n is a, c, g, or t
caagcagaagacggcatacgagatcnngtcatgtctcgtgggctcggagatgtgtataagagacag

SEQ ID NO: 847 - DNA, 66 bp, Artificial
  synthetic
  misc_feature (27)..(27): n is a, c, g, or t
caagcagaagacggcatacgagatccnctcatgtctcgtgggctcggagatgtgtataagagacag

SEQ ID NO: 848 - DNA, 66 bp, Artificial
  synthetic
  misc_feature (26)..(27): n is a, c, g, or t
caagcagaagacggcatacgagattnnctcatgtctcgtgggctcggagatgtgtataagagacag

SEQ ID NO: 849 - DNA, 66 bp, Artificial
  synthetic
  misc_feature (26)..(27): n is a, c, g, or t
caagcagaagacggcatacgagatgnnctcatgtctcgtgggctcggagatgtgtataagagacag

SEQ ID NO: 850 - DNA, 66 bp, Artificial
  synthetic
  misc_feature (26)..(27): n is a, c, g, or t
caagcagaagacggcatacgagatannctcatgtctcgtgggctcggagatgtgtataagagacag

SEQ ID NO: 851 - DNA, 66 bp, Artificial
  synthetic
  misc_feature (26)..(27): n is a, c, g, or t
caagcagaagacggcatacgagattnnatcatgtctcgtgggctcggagatgtgtataagagacag

SEQ ID NO: 852 - DNA, 66 bp, Artificial
  synthetic
  misc_feature (26)..(27): n is a, c, g, or t
caagcagaagacggcatacgagatgnnatcatgtctcgtgggctcggagatgtgtataagagacag

SEQ ID NO: 853 - DNA, 66 bp, Artificial
  synthetic
  misc_feature (26)..(27): n is a, c, g, or t
caagcagaagacggcatacgagatcnnatcatgtctcgtgggctcggagatgtgtataagagacag

SEQ ID NO: 854 - DNA, 66 bp, Artificial
  synthetic
  misc_feature (27)..(27): n is a, c, g, or t
caagcagaagacggcatacgagatcgntgcatgtctcgtgggctcggagatgtgtataagagacag

SEQ ID NO: 855 - DNA, 66 bp, Artificial
  synthetic
  misc_feature (27)..(27): n is a, c, g, or t
caagcagaagacggcatacgagatccntgcatgtctcgtgggctcggagatgtgtataagagacag

SEQ ID NO: 856 - DNA, 66 bp, Artificial
  synthetic
  misc_feature (27)..(27): n is a, c, g, or t
caagcagaagacggcatacgagatcantgcatgtctcgtgggctcggagatgtgtataagagacag

SEQ ID NO: 857 - DNA, 66 bp, Artificial
  synthetic
  misc_feature (27)..(27): n is a, c, g, or t
caagcagaagacggcatacgagattgnggcatgtctcgtgggctcggagatgtgtataagagacag

SEQ ID NO: 858 - DNA, 66 bp, Artificial
  synthetic
  misc_feature (27)..(27): n is a, c, g, or t
caagcagaagacggcatacgagatggnggcatgtctcgtgggctcggagatgtgtataagagacag

SEQ ID NO: 859 - DNA, 66 bp, Artificial
  synthetic
  misc_feature (27)..(27): n is a, c, g, or t
caagcagaagacggcatacgagattcnggcatgtctcgtgggctcggagatgtgtataagagacag

SEQ ID NO: 860 - DNA, 66 bp, Artificial
  synthetic
  misc_feature (27)..(27): n is a, c, g, or t
caagcagaagacggcatacgagatgcnggcatgtctcgtgggctcggagatgtgtataagagacag

SEQ ID NO: 861 - DNA, 66 bp, Artificial
  synthetic
  misc_feature (27)..(27): n is a, c, g, or t
caagcagaagacggcatacgagattanggcatgtctcgtgggctcggagatgtgtataagagacag

SEQ ID NO: 862 - DNA, 66 bp, Artificial
  synthetic
  misc_feature (27)..(27): n is a, c, g, or t
caagcagaagacggcatacgagatganggcatgtctcgtgggctcggagatgtgtataagagacag

SEQ ID NO: 863 - DNA, 66 bp, Artificial
  synthetic
  misc_feature (27)..(27): n is a, c, g, or t
caagcagaagacggcatacgagatagncgcatgtctcgtgggctcggagatgtgtataagagacag

SEQ ID NO: 864 - DNA, 66 bp, Artificial
  synthetic
  misc_feature (27)..(27): n is a, c, g, or t
caagcagaagacggcatacgagatacncgcatgtctcgtgggctcggagatgtgtataagagacag

SEQ ID NO: 865 - DNA, 66 bp, Artificial
  synthetic
  misc_feature (27)..(27): n is a, c, g, or t
caagcagaagacggcatacgagataancgcatgtctcgtgggctcggagatgtgtataagagacag

SEQ ID NO: 866 - DNA, 66 bp, Artificial
  synthetic
  misc_feature (27)..(27): n is a, c, g, or t
caagcagaagacggcatacgagattgnagcatgtctcgtgggctcggagatgtgtataagagacag

SEQ ID NO: 867 - DNA, 66 bp, Artificial
  synthetic
  misc_feature (27)..(27): n is a, c, g, or t
caagcagaagacggcatacgagatggnagcatgtctcgtgggctcggagatgtgtataagagacag

SEQ ID NO: 868 - DNA, 66 bp, Artificial
  synthetic
  misc_feature (27)..(27): n is a, c, g, or t
caagcagaagacggcatacgagattcnagcatgtctcgtgggctcggagatgtgtataagagacag

SEQ ID NO: 869 - DNA, 66 bp, Artificial
  synthetic
  misc_feature (27)..(27): n is a, c, g, or t
caagcagaagacggcatacgagatgcnagcatgtctcgtgggctcggagatgtgtataagagacag

SEQ ID NO: 870 - DNA, 66 bp, Artificial
  synthetic
  misc_feature (27)..(27): n is a, c, g, or t
caagcagaagacggcatacgagattanagcatgtctcgtgggctcggagatgtgtataagagacag

SEQ ID NO: 871 - DNA, 66 bp, Artificial
  synthetic
  misc_feature (27)..(27): n is a, c, g, or t
caagcagaagacggcatacgagatganagcatgtctcgtgggctcggagatgtgtataagagacag

SEQ ID NO: 872 - DNA, 66 bp, Artificial
  synthetic
  misc_feature (27)..(27): n is a, c, g, or t
caagcagaagacggcatacgagatcgntccatgtctcgtgggctcggagatgtgtataagagacag

SEQ ID NO: 873 - DNA, 66 bp, Artificial
  synthetic
  misc_feature (27)..(27): n is a, c, g, or t
caagcagaagacggcatacgagatccntccatgtctcgtgggctcggagatgtgtataagagacag

SEQ ID NO: 874 - DNA, 66 bp, Artificial
  synthetic
  misc_feature (27)..(27): n is a, c, g, or t
caagcagaagacggcatacgagatcantccatgtctcgtgggctcggagatgtgtataagagacag

SEQ ID NO: 875 - DNA, 66 bp, Artificial
  synthetic
  misc_feature (27)..(27): n is a, c, g, or t
caagcagaagacggcatacgagattgngccatgtctcgtgggctcggagatgtgtataagagacag

SEQ ID NO: 876 - DNA, 66 bp, Artificial
  synthetic
  misc_feature (27)..(27): n is a, c, g, or t
caagcagaagacggcatacgagatggngccatgtctcgtgggctcggagatgtgtataagagacag

SEQ ID NO: 877 - DNA, 66 bp, Artificial
  synthetic
  misc_feature (27)..(27): n is a, c, g, or t
caagcagaagacggcatacgagattcngccatgtctcgtgggctcggagatgtgtataagagacag

SEQ ID NO: 878 - DNA, 66 bp, Artificial
  synthetic
  misc_feature (27)..(27): n is a, c, g, or t
caagcagaagacggcatacgagatgcngccatgtctcgtgggctcggagatgtgtataagagacag

SEQ ID NO: 879 - DNA, 66 bp, Artificial
  synthetic
  misc_feature (27)..(27): n is a, c, g, or t
caagcagaagacggcatacgagattangccatgtctcgtgggctcggagatgtgtataagagacag

SEQ ID NO: 880 - DNA, 66 bp, Artificial
  synthetic
  misc_feature (27)..(27): n is a, c, g, or t
caagcagaagacggcatacgagatgangccatgtctcgtgggctcggagatgtgtataagagacag

SEQ ID NO: 881 - DNA, 66 bp, Artificial
  synthetic
  misc_feature (27)..(27): n is a, c, g, or t
caagcagaagacggcatacgagatagncccatgtctcgtgggctcggagatgtgtataagagacag

SEQ ID NO: 882 - DNA, 66 bp, Artificial
  synthetic
  misc_feature (27)..(27): n is a, c, g, or t
caagcagaagacggcatacgagatacncccatgtctcgtgggctcggagatgtgtataagagacag

SEQ ID NO: 883 - DNA, 66 bp, Artificial
  synthetic
  misc_feature (27)..(27): n is a, c, g, or t
caagcagaagacggcatacgagataancccatgtctcgtgggctcggagatgtgtataagagacag

SEQ ID NO: 884 - DNA, 66 bp, Artificial
  synthetic
  misc_feature (27)..(27): n is a, c, g, or t
caagcagaagacggcatacgagattgnaccatgtctcgtgggctcggagatgtgtataagagacag

SEQ ID NO: 885 - DNA, 66 bp, Artificial
  synthetic
  misc_feature (27)..(27): n is a, c, g, or t
caagcagaagacggcatacgagatggnaccatgtctcgtgggctcggagatgtgtataagagacag

SEQ ID NO: 886 - DNA, 66 bp, Artificial
  synthetic
  misc_feature (27)..(27): n is a, c, g, or t
caagcagaagacggcatacgagattcnaccatgtctcgtgggctcggagatgtgtataagagacag

SEQ ID NO: 887 - DNA, 66 bp, Artificial
  synthetic
  misc_feature (27)..(27): n is a, c, g, or t
caagcagaagacggcatacgagatgcnaccatgtctcgtgggctcggagatgtgtataagagacag

SEQ ID NO: 888 - DNA, 66 bp, Artificial
  synthetic
  misc_feature (27)..(27): n is a, c, g, or t
caagcagaagacggcatacgagattanaccatgtctcgtgggctcggagatgtgtataagagacag

SEQ ID NO: 889 - DNA, 66 bp, Artificial
  synthetic
  misc_feature (27)..(27): n is a, c, g, or t
caagcagaagacggcatacgagatganaccatgtctcgtgggctcggagatgtgtataagagacag

SEQ ID NO: 890 - DNA, 66 bp, Artificial
  synthetic
  misc_feature (26)..(27): n is a, c, g, or t
  misc_feature (29)..(29): n is a, c, g, or t
caagcagaagacggcatacgagattnntncatgtctcgtgggctcggagatgtgtataagagacag

SEQ ID NO: 891 - DNA, 66 bp, Artificial
  synthetic
  misc_feature (26)..(27): n is a, c, g, or t
  misc_feature (29)..(29): n is a, c, g, or t
caagcagaagacggcatacgagatgnntncatgtctcgtgggctcggagatgtgtataagagacag

SEQ ID NO: 892 - DNA, 66 bp, Artificial
  synthetic
  misc_feature (26)..(27): n is a, c, g, or t
  misc_feature (29)..(29): n is a, c, g, or t
caagcagaagacggcatacgagatanntncatgtctcgtgggctcggagatgtgtataagagacag

SEQ ID NO: 893 - DNA, 66 bp, Artificial
  synthetic
  misc_feature (26)..(27): n is a, c, g, or t
  misc_feature (29)..(29): n is a, c, g, or t
caagcagaagacggcatacgagatanngncatgtctcgtgggctcggagatgtgtataagagacag

SEQ ID NO: 894 - DNA, 66 bp, Artificial
  synthetic
  misc_feature (26)..(27): n is a, c, g, or t
  misc_feature (29)..(29): n is a, c, g, or t
caagcagaagacggcatacgagatannancatgtctcgtgggctcggagatgtgtataagagacag

SEQ ID NO: 895 - DNA, 66 bp, Artificial
  synthetic
  misc_feature (26)..(27): n is a, c, g, or t
caagcagaagacggcatacgagatcnntacatgtctcgtgggctcggagatgtgtataagagacag

SEQ ID NO: 896 - DNA, 66 bp, Artificial
  synthetic
caagcagaagacggcatacgagatcctgacatgtctcgtgggctcggagatgtgtataagagacag

SEQ ID NO: 897 - DNA, 66 bp, Artificial
  synthetic
caagcagaagacggcatacgagatcccgacatgtctcgtgggctcggagatgtgtataagagacag

SEQ ID NO: 898 - DNA, 66 bp, Artificial
  synthetic
  misc_feature (26)..(27): n is a, c, g, or t
caagcagaagacggcatacgagattnngacatgtctcgtgggctcggagatgtgtataagagacag

SEQ ID NO: 899 - DNA, 66 bp, Artificial
  synthetic
  misc_feature (26)..(27): n is a, c, g, or t
caagcagaagacggcatacgagatgnngacatgtctcgtgggctcggagatgtgtataagagacag

SEQ ID NO: 900 - DNA, 66 bp, Artificial
  synthetic
caagcagaagacggcatacgagatccagacatgtctcgtgggctcggagatgtgtataagagacag

SEQ ID NO: 901 - DNA, 66 bp, Artificial
  synthetic
  misc_feature (27)..(27): n is a, c, g, or t
caagcagaagacggcatacgagattgncacatgtctcgtgggctcggagatgtgtataagagacag

SEQ ID NO: 902 - DNA, 66 bp, Artificial
  synthetic
  misc_feature (27)..(27): n is a, c, g, or t
caagcagaagacggcatacgagatggncacatgtctcgtgggctcggagatgtgtataagagacag

SEQ ID NO: 903 - DNA, 66 bp, Artificial
  synthetic
  misc_feature (27)..(27): n is a, c, g, or t
caagcagaagacggcatacgagattcncacatgtctcgtgggctcggagatgtgtataagagacag

SEQ ID NO: 904 - DNA, 66 bp, Artificial
  synthetic
  misc_feature (27)..(27): n is a, c, g, or t
caagcagaagacggcatacgagatgcncacatgtctcgtgggctcggagatgtgtataagagacag

SEQ ID NO: 905 - DNA, 66 bp, Artificial
  synthetic
  misc_feature (26)..(27): n is a, c, g, or t
caagcagaagacggcatacgagatanncacatgtctcgtgggctcggagatgtgtataagagacag

SEQ ID NO: 906 - DNA, 66 bp, Artificial
  synthetic
  misc_feature (27)..(27): n is a, c, g, or t
caagcagaagacggcatacgagattancacatgtctcgtgggctcggagatgtgtataagagacag

SEQ ID NO: 907 - DNA, 66 bp, Artificial
  synthetic
  misc_feature (27)..(27): n is a, c, g, or t
caagcagaagacggcatacgagatgancacatgtctcgtgggctcggagatgtgtataagagacag

SEQ ID NO: 908 - DNA, 66 bp, Artificial
  synthetic
caagcagaagacggcatacgagatcctaacatgtctcgtgggctcggagatgtgtataagagacag

SEQ ID NO: 909 - DNA, 66 bp, Artificial
  synthetic
caagcagaagacggcatacgagatcccaacatgtctcgtgggctcggagatgtgtataagagacag

SEQ ID NO: 910 - DNA, 66 bp, Artificial
  synthetic
  misc_feature (26)..(27): n is a, c, g, or t
caagcagaagacggcatacgagattnnaacatgtctcgtgggctcggagatgtgtataagagacag

SEQ ID NO: 911 - DNA, 66 bp, Artificial
  synthetic
  misc_feature (26)..(27): n is a, c, g, or t
caagcagaagacggcatacgagatgnnaacatgtctcgtgggctcggagatgtgtataagagacag

SEQ ID NO: 912 - DNA, 66 bp, Artificial
  synthetic
caagcagaagacggcatacgagatccaaacatgtctcgtgggctcggagatgtgtataagagacag

SEQ ID NO: 913 - DNA, 66 bp, Artificial
  synthetic
  misc_feature (26)..(27): n is a, c, g, or t
caagcagaagacggcatacgagatcnngtaatgtctcgtgggctcggagatgtgtataagagacag

SEQ ID NO: 914 - DNA, 66 bp, Artificial
  synthetic
  misc_feature (26)..(27): n is a, c, g, or t
caagcagaagacggcatacgagattnnctaatgtctcgtgggctcggagatgtgtataagagacag

SEQ ID NO: 915 - DNA, 66 bp, Artificial
  synthetic
  misc_feature (26)..(27): n is a, c, g, or t
caagcagaagacggcatacgagatgnnctaatgtctcgtgggctcggagatgtgtataagagacag

SEQ ID NO: 916 - DNA, 66 bp, Artificial
  synthetic
  misc_feature (26)..(27): n is a, c, g, or t
caagcagaagacggcatacgagatcnnctaatgtctcgtgggctcggagatgtgtataagagacag

SEQ ID NO: 917 - DNA, 66 bp, Artificial
  synthetic
  misc_feature (26)..(27): n is a, c, g, or t
caagcagaagacggcatacgagatcnnataatgtctcgtgggctcggagatgtgtataagagacag

SEQ ID NO: 918 - DNA, 66 bp, Artificial
  synthetic
caagcagaagacggcatacgagatcgtggaatgtctcgtgggctcggagatgtgtataagagacag

SEQ ID NO: 919 - DNA, 66 bp, Artificial
  synthetic
caagcagaagacggcatacgagatcatggaatgtctcgtgggctcggagatgtgtataagagacag

SEQ ID NO: 920 - DNA, 66 bp, Artificial
  synthetic
caagcagaagacggcatacgagatcgcggaatgtctcgtgggctcggagatgtgtataagagacag

SEQ ID NO: 921 - DNA, 66 bp, Artificial
  synthetic
caagcagaagacggcatacgagatcacggaatgtctcgtgggctcggagatgtgtataagagacag

SEQ ID NO: 922 - DNA, 66 bp, Artificial
  synthetic
  misc_feature (27)..(27): n is a, c, g, or t
caagcagaagacggcatacgagatccnggaatgtctcgtgggctcggagatgtgtataagagacag

SEQ ID NO: 923 - DNA, 66 bp, Artificial
  synthetic
caagcagaagacggcatacgagatcgaggaatgtctcgtgggctcggagatgtgtataagagacag

SEQ ID NO: 924 - DNA, 66 bp, Artificial
  synthetic
caagcagaagacggcatacgagatcaaggaatgtctcgtgggctcggagatgtgtataagagacag

SEQ ID NO: 925 - DNA, 66 bp, Artificial
  synthetic
  misc_feature (27)..(27): n is a, c, g, or t
caagcagaagacggcatacgagattgncgaatgtctcgtgggctcggagatgtgtataagagacag

SEQ ID NO: 926 - DNA, 66 bp, Artificial
  synthetic
  misc_feature (27)..(27): n is a, c, g, or t
caagcagaagacggcatacgagatggncgaatgtctcgtgggctcggagatgtgtataagagacag

SEQ ID NO: 927 - DNA, 66 bp, Artificial
  synthetic
  misc_feature (27)..(27): n is a, c, g, or t
caagcagaagacggcatacgagattcncgaatgtctcgtgggctcggagatgtgtataagagacag

SEQ ID NO: 928 - DNA, 66 bp, Artificial
  synthetic
  misc_feature (27)..(27): n is a, c, g, or t
caagcagaagacggcatacgagatgcncgaatgtctcgtgggctcggagatgtgtataagagacag

SEQ ID NO: 929 - DNA, 66 bp, Artificial
  synthetic
  misc_feature (27)..(27): n is a, c, g, or t
caagcagaagacggcatacgagattancgaatgtctcgtgggctcggagatgtgtataagagacag

SEQ ID NO: 930 - DNA, 66 bp, Artificial
  synthetic
  misc_feature (27)..(27): n is a, c, g, or t
caagcagaagacggcatacgagatgancgaatgtctcgtgggctcggagatgtgtataagagacag

SEQ ID NO: 931 - DNA, 66 bp, Artificial
  synthetic
caagcagaagacggcatacgagatcgtagaatgtctcgtgggctcggagatgtgtataagagacag

SEQ ID NO: 932 - DNA, 66 bp, Artificial
  synthetic
caagcagaagacggcatacgagatcatagaatgtctcgtgggctcggagatgtgtataagagacag

SEQ ID NO: 933 - DNA, 66 bp, Artificial
  synthetic
caagcagaagacggcatacgagatcgcagaatgtctcgtgggctcggagatgtgtataagagacag

SEQ ID NO: 934 - DNA, 66 bp, Artificial
  synthetic
caagcagaagacggcatacgagatcacagaatgtctcgtgggctcggagatgtgtataagagacag

SEQ ID NO: 935 - DNA, 66 bp, Artificial
  synthetic
  misc_feature (27)..(27): n is a, c, g, or t
caagcagaagacggcatacgagatccnagaatgtctcgtgggctcggagatgtgtataagagacag

SEQ ID NO: 936 - DNA, 66 bp, Artificial
  synthetic
caagcagaagacggcatacgagatcgaagaatgtctcgtgggctcggagatgtgtataagagacag

SEQ ID NO: 937 - DNA, 66 bp, Artificial
  synthetic
caagcagaagacggcatacgagatcaaagaatgtctcgtgggctcggagatgtgtataagagacag

SEQ ID NO: 938 - DNA, 66 bp, Artificial
  synthetic
  misc_feature (27)..(27): n is a, c, g, or t
caagcagaagacggcatacgagatccngcaatgtctcgtgggctcggagatgtgtataagagacag

SEQ ID NO: 939 - DNA, 66 bp, Artificial
  synthetic
  misc_feature (27)..(27): n is a, c, g, or t
caagcagaagacggcatacgagattgnccaatgtctcgtgggctcggagatgtgtataagagacag

SEQ ID NO: 940 - DNA, 66 bp, Artificial
  synthetic
  misc_feature (27)..(27): n is a, c, g, or t
caagcagaagacggcatacgagatggnccaatgtctcgtgggctcggagatgtgtataagagacag

SEQ ID NO: 941 - DNA, 66 bp, Artificial
  synthetic
  misc_feature (27)..(27): n is a, c, g, or t
caagcagaagacggcatacgagattcnccaatgtctcgtgggctcggagatgtgtataagagacag

SEQ ID NO: 942 - DNA, 66 bp, Artificial
  synthetic
  misc_feature (27)..(27): n is a, c, g, or t
caagcagaagacggcatacgagatgcnccaatgtctcgtgggctcggagatgtgtataagagacag

SEQ ID NO: 943 - DNA, 66 bp, Artificial
  synthetic
  misc_feature (27)..(27): n is a, c, g, or t
caagcagaagacggcatacgagattanccaatgtctcgtgggctcggagatgtgtataagagacag

SEQ ID NO: 944 - DNA, 66 bp, Artificial
  synthetic
  misc_feature (27)..(27): n is a, c, g, or t
caagcagaagacggcatacgagatganccaatgtctcgtgggctcggagatgtgtataagagacag

SEQ ID NO: 945 - DNA, 66 bp, Artificial
  synthetic
  misc_feature (27)..(27): n is a, c, g, or t
caagcagaagacggcatacgagatccnacaatgtctcgtgggctcggagatgtgtataagagacag

SEQ ID NO: 946 - DNA, 66 bp, Artificial
  synthetic
  misc_feature (25)..(27): n is a, c, g, or t
  misc_feature (29)..(29): n is a, c, g, or t
caagcagaagacggcatacgagatnnntnaatgtctcgtgggctcggagatgtgtataagagacag

SEQ ID NO: 947 - DNA, 66 bp, Artificial
  synthetic
  misc_feature (26)..(27): n is a, c, g, or t
  misc_feature (29)..(29): n is a, c, g, or t
caagcagaagacggcatacgagattnngnaatgtctcgtgggctcggagatgtgtataagagacag

SEQ ID NO: 948 - DNA, 66 bp, Artificial
  synthetic
  misc_feature (26)..(27): n is a, c, g, or t
  misc_feature (29)..(29): n is a, c, g, or t
caagcagaagacggcatacgagatgnngnaatgtctcgtgggctcggagatgtgtataagagacag

SEQ ID NO: 949 - DNA, 66 bp, Artificial
  synthetic
  misc_feature (26)..(27): n is a, c, g, or t
  misc_feature (29)..(29): n is a, c, g, or t
caagcagaagacggcatacgagatanngnaatgtctcgtgggctcggagatgtgtataagagacag

SEQ ID NO: 950 - DNA, 66 bp, Artificial
  synthetic
  misc_feature (26)..(27): n is a, c, g, or t
  misc_feature (29)..(29): n is a, c, g, or t
caagcagaagacggcatacgagatanncnaatgtctcgtgggctcggagatgtgtataagagacag

SEQ ID NO: 951 - DNA, 66 bp, Artificial
  synthetic
  misc_feature (26)..(27): n is a, c, g, or t
  misc_feature (29)..(29): n is a, c, g, or t
caagcagaagacggcatacgagattnnanaatgtctcgtgggctcggagatgtgtataagagacag

SEQ ID NO: 952 - DNA, 66 bp, Artificial
  synthetic
  misc_feature (26)..(27): n is a, c, g, or t
  misc_feature (29)..(29): n is a, c, g, or t
caagcagaagacggcatacgagatgnnanaatgtctcgtgggctcggagatgtgtataagagacag

SEQ ID NO: 953 - DNA, 66 bp, Artificial
  synthetic
  misc_feature (26)..(27): n is a, c, g, or t
  misc_feature (29)..(29): n is a, c, g, or t
caagcagaagacggcatacgagatannanaatgtctcgtgggctcggagatgtgtataagagacag

SEQ ID NO: 954 - DNA, 66 bp, Artificial
  synthetic
  misc_feature (26)..(27): n is a, c, g, or t
caagcagaagacggcatacgagatcnngaaatgtctcgtgggctcggagatgtgtataagagacag

SEQ ID NO: 955 - DNA, 66 bp, Artificial
  synthetic
caagcagaagacggcatacgagatcctcaaatgtctcgtgggctcggagatgtgtataagagacag

SEQ ID NO: 956 - DNA, 66 bp, Artificial
  synthetic
caagcagaagacggcatacgagatccccaaatgtctcgtgggctcggagatgtgtataagagacag

SEQ ID NO: 957 - DNA, 66 bp, Artificial
  synthetic
  misc_feature (26)..(27): n is a, c, g, or t
caagcagaagacggcatacgagattnncaaatgtctcgtgggctcggagatgtgtataagagacag

SEQ ID NO: 958 - DNA, 66 bp, Artificial
  synthetic
  misc_feature (26)..(27): n is a, c, g, or t
caagcagaagacggcatacgagatgnncaaatgtctcgtgggctcggagatgtgtataagagacag

SEQ ID NO: 959 - DNA, 66 bp, Artificial
  synthetic
caagcagaagacggcatacgagatccacaaatgtctcgtgggctcggagatgtgtataagagacag

SEQ ID NO: 960 - DNA, 66 bp, Artificial
  synthetic
  misc_feature (26)..(27): n is a, c, g, or t
caagcagaagacggcatacgagatcnnaaaatgtctcgtgggctcggagatgtgtataagagacag

SEQ ID NO: 961 - DNA, 66 bp, Artificial
  synthetic
  misc_feature (25)..(31): n is a, c, g, or t
caagcagaagacggcatacgagatnnnnnnnggtctcgtgggctcggagatgtgtataagagacag

SEQ ID NO: 962 - DNA, 66 bp, Artificial
  synthetic
  misc_feature (25)..(31): n is a, c, g, or t
caagcagaagacggcatacgagatnnnnnnncgtctcgtgggctcggagatgtgtataagagacag

SEQ ID NO: 963 - DNA, 66 bp, Artificial
  synthetic
  misc_feature (25)..(31): n is a, c, g, or t
caagcagaagacggcatacgagatnnnnnnnagtctcgtgggctcggagatgtgtataagagacag

SEQ ID NO: 964 - DNA, 66 bp, Artificial
  synthetic
  misc_feature (26)..(27): n is a, c, g, or t
caagcagaagacggcatacgagattnntttttgtctcgtgggctcggagatgtgtataagagacag

SEQ ID NO: 965 - DNA, 66 bp, Artificial
  synthetic
  misc_feature (26)..(27): n is a, c, g, or t
caagcagaagacggcatacgagatgnntttttgtctcgtgggctcggagatgtgtataagagacag

SEQ ID NO: 966 - DNA, 66 bp, Artificial
  synthetic
  misc_feature (26)..(27): n is a, c, g, or t
caagcagaagacggcatacgagatanntttttgtctcgtgggctcggagatgtgtataagagacag

SEQ ID NO: 967 - DNA, 66 bp, Artificial
  synthetic
  misc_feature (27)..(27): n is a, c, g, or t
caagcagaagacggcatacgagatagngttttgtctcgtgggctcggagatgtgtataagagacag

SEQ ID NO: 968 - DNA, 66 bp, Artificial
  synthetic
  misc_feature (27)..(27): n is a, c, g, or t
caagcagaagacggcatacgagatacngttttgtctcgtgggctcggagatgtgtataagagacag

SEQ ID NO: 969 - DNA, 66 bp, Artificial
  synthetic
  misc_feature (27)..(27): n is a, c, g, or t
caagcagaagacggcatacgagataangttttgtctcgtgggctcggagatgtgtataagagacag

SEQ ID NO: 970 - DNA, 66 bp, Artificial
  synthetic
  misc_feature (27)..(27): n is a, c, g, or t
caagcagaagacggcatacgagatagnattttgtctcgtgggctcggagatgtgtataagagacag

SEQ ID NO: 971 - DNA, 66 bp, Artificial
  synthetic
  misc_feature (27)..(27): n is a, c, g, or t
caagcagaagacggcatacgagatacnattttgtctcgtgggctcggagatgtgtataagagacag

SEQ ID NO: 972 - DNA, 66 bp, Artificial
  synthetic
  misc_feature (27)..(27): n is a, c, g, or t
caagcagaagacggcatacgagataanattttgtctcgtgggctcggagatgtgtataagagacag

SEQ ID NO: 973 - DNA, 66 bp, Artificial
  synthetic
  misc_feature (27)..(27): n is a, c, g, or t
caagcagaagacggcatacgagatacntgtttgtctcgtgggctcggagatgtgtataagagacag

SEQ ID NO: 974 - DNA, 66 bp, Artificial
  synthetic
caagcagaagacggcatacgagatacttctttgtctcgtgggctcggagatgtgtataagagacag

SEQ ID NO: 975 - DNA, 66 bp, Artificial
  synthetic
caagcagaagacggcatacgagatacctctttgtctcgtgggctcggagatgtgtataagagacag

SEQ ID NO: 976 - DNA, 66 bp, Artificial
  synthetic
caagcagaagacggcatacgagatacatctttgtctcgtgggctcggagatgtgtataagagacag

SEQ ID NO: 977 - DNA, 66 bp, Artificial
  synthetic
caagcagaagacggcatacgagattcttatttgtctcgtgggctcggagatgtgtataagagacag

SEQ ID NO: 978 - DNA, 66 bp, Artificial
  synthetic
caagcagaagacggcatacgagatgcttatttgtctcgtgggctcggagatgtgtataagagacag

SEQ ID NO: 979 - DNA, 66 bp, Artificial
  synthetic
caagcagaagacggcatacgagattcctatttgtctcgtgggctcggagatgtgtataagagacag

SEQ ID NO: 980 - DNA, 66 bp, Artificial
  synthetic
caagcagaagacggcatacgagatgcctatttgtctcgtgggctcggagatgtgtataagagacag

SEQ ID NO: 981 - DNA, 66 bp, Artificial
  synthetic
  misc_feature (26)..(27): n is a, c, g, or t
caagcagaagacggcatacgagatanntatttgtctcgtgggctcggagatgtgtataagagacag

SEQ ID NO: 982 - DNA, 66 bp, Artificial
  synthetic
caagcagaagacggcatacgagattcatatttgtctcgtgggctcggagatgtgtataagagacag

SEQ ID NO: 983 - DNA, 66 bp, Artificial
  synthetic
caagcagaagacggcatacgagatgcatatttgtctcgtgggctcggagatgtgtataagagacag

SEQ ID NO: 984 - DNA, 66 bp, Artificial
  synthetic
caagcagaagacggcatacgagatagtttgttgtctcgtgggctcggagatgtgtataagagacag

SEQ ID NO: 985 - DNA, 66 bp, Artificial
  synthetic
caagcagaagacggcatacgagataatttgttgtctcgtgggctcggagatgtgtataagagacag

SEQ ID NO: 986 - DNA, 66 bp, Artificial
  synthetic
caagcagaagacggcatacgagatagcttgttgtctcgtgggctcggagatgtgtataagagacag

SEQ ID NO: 987 - DNA, 66 bp, Artificial
  synthetic
caagcagaagacggcatacgagataacttgttgtctcgtgggctcggagatgtgtataagagacag

SEQ ID NO: 988 - DNA, 66 bp, Artificial
  synthetic
  misc_feature (27)..(27): n is a, c, g, or t
caagcagaagacggcatacgagatacnttgttgtctcgtgggctcggagatgtgtataagagacag

SEQ ID NO: 989 - DNA, 66 bp, Artificial
  synthetic
caagcagaagacggcatacgagatagattgttgtctcgtgggctcggagatgtgtataagagacag

SEQ ID NO: 990 - DNA, 66 bp, Artificial
  synthetic
caagcagaagacggcatacgagataaattgttgtctcgtgggctcggagatgtgtataagagacag

SEQ ID NO: 991 - DNA, 66 bp, Artificial
  synthetic
  misc_feature (27)..(27): n is a, c, g, or t
caagcagaagacggcatacgagatacnttcttgtctcgtgggctcggagatgtgtataagagacag

SEQ ID NO: 992 - DNA, 66 bp, Artificial
  synthetic
  misc_feature (27)..(27): n is a, c, g, or t
caagcagaagacggcatacgagattcnttattgtctcgtgggctcggagatgtgtataagagacag

SEQ ID NO: 993 - DNA, 66 bp, Artificial
  synthetic
  misc_feature (27)..(27): n is a, c, g, or t
caagcagaagacggcatacgagatgcnttattgtctcgtgggctcggagatgtgtataagagacag

SEQ ID NO: 994 - DNA, 66 bp, Artificial
  synthetic
  misc_feature (26)..(27): n is a, c, g, or t
caagcagaagacggcatacgagatannttattgtctcgtgggctcggagatgtgtataagagacag

SEQ ID NO: 995 - DNA, 66 bp, Artificial
  synthetic
caagcagaagacggcatacgagatacttaattgtctcgtgggctcggagatgtgtataagagacag

SEQ ID NO: 996 - DNA, 66 bp, Artificial
  synthetic
caagcagaagacggcatacgagatacctaattgtctcgtgggctcggagatgtgtataagagacag

SEQ ID NO: 997 - DNA, 66 bp, Artificial
  synthetic
caagcagaagacggcatacgagatacataattgtctcgtgggctcggagatgtgtataagagacag

SEQ ID NO: 998 - DNA, 66 bp, Artificial
  synthetic
  misc_feature (27)..(27): n is a, c, g, or t
caagcagaagacggcatacgagatagntttgtgtctcgtgggctcggagatgtgtataagagacag

SEQ ID NO: 999 - DNA, 66 bp, Artificial
  synthetic
  misc_feature (27)..(27): n is a, c, g, or t
caagcagaagacggcatacgagatacntttgtgtctcgtgggctcggagatgtgtataagagacag

SEQ ID NO: 1000 - DNA, 66 bp, Artificial
  synthetic
  misc_feature (27)..(27): n is a, c, g, or t
caagcagaagacggcatacgagataantttgtgtctcgtgggctcggagatgtgtataagagacag

SEQ ID NO: 1001 - DNA, 66 bp, Artificial
  synthetic
  misc_feature (26)..(27): n is a, c, g, or t
caagcagaagacggcatacgagattnntttatgtctcgtgggctcggagatgtgtataagagacag

SEQ ID NO: 1002 - DNA, 66 bp, Artificial
  synthetic
  misc_feature (26)..(27): n is a, c, g, or t
caagcagaagacggcatacgagatgnntttatgtctcgtgggctcggagatgtgtataagagacag

SEQ ID NO: 1003 - DNA, 66 bp, Artificial
  synthetic
  misc_feature (26)..(27): n is a, c, g, or t
caagcagaagacggcatacgagatanntttatgtctcgtgggctcggagatgtgtataagagacag

SEQ ID NO: 1004 - DNA, 66 bp, Artificial
  synthetic
caagcagaagacggcatacgagatattgttatgtctcgtgggctcggagatgtgtataagagacag

SEQ ID NO: 1005 - DNA, 66 bp, Artificial
  synthetic
caagcagaagacggcatacgagatatcgttatgtctcgtgggctcggagatgtgtataagagacag

SEQ ID NO: 1006 - DNA, 66 bp, Artificial
  synthetic
  misc_feature (27)..(27): n is a, c, g, or t
caagcagaagacggcatacgagatagngttatgtctcgtgggctcggagatgtgtataagagacag

SEQ ID NO: 1007 - DNA, 66 bp, Artificial
  synthetic
  misc_feature (27)..(27): n is a, c, g, or t
caagcagaagacggcatacgagatacngttatgtctcgtgggctcggagatgtgtataagagacag

SEQ ID NO: 1008 - DNA, 66 bp, Artificial
  synthetic
  misc_feature (27)..(27): n is a, c, g, or t
caagcagaagacggcatacgagataangttatgtctcgtgggctcggagatgtgtataagagacag

SEQ ID NO: 1009 - DNA, 66 bp, Artificial
  synthetic
caagcagaagacggcatacgagatatagttatgtctcgtgggctcggagatgtgtataagagacag

SEQ ID NO: 1010 - DNA, 66 bp, Artificial
  synthetic
caagcagaagacggcatacgagatattattatgtctcgtgggctcggagatgtgtataagagacag

SEQ ID NO: 1011 - DNA, 66 bp, Artificial
  synthetic
caagcagaagacggcatacgagatatcattatgtctcgtgggctcggagatgtgtataagagacag

SEQ ID NO: 1012 - DNA, 66 bp, Artificial
  synthetic
  misc_feature (27)..(27): n is a, c, g, or t
caagcagaagacggcatacgagatagnattatgtctcgtgggctcggagatgtgtataagagacag

SEQ ID NO: 1013 - DNA, 66 bp, Artificial
  synthetic
  misc_feature (27)..(27): n is a, c, g, or t
caagcagaagacggcatacgagatacnattatgtctcgtgggctcggagatgtgtataagagacag

SEQ ID NO: 1014 - DNA, 66 bp, Artificial
  synthetic
  misc_feature (27)..(27): n is a, c, g, or t
caagcagaagacggcatacgagataanattatgtctcgtgggctcggagatgtgtataagagacag

SEQ ID NO: 1015 - DNA, 66 bp, Artificial
  synthetic
caagcagaagacggcatacgagatataattatgtctcgtgggctcggagatgtgtataagagacag

SEQ ID NO: 1016 - DNA, 66 bp, Artificial
  synthetic
caagcagaagacggcatacgagatagttgtatgtctcgtgggctcggagatgtgtataagagacag

SEQ ID NO: 1017 - DNA, 66 bp, Artificial
  synthetic
caagcagaagacggcatacgagataattgtatgtctcgtgggctcggagatgtgtataagagacag

SEQ ID NO: 1018 - DNA, 66 bp, Artificial
  synthetic
caagcagaagacggcatacgagatagctgtatgtctcgtgggctcggagatgtgtataagagacag

SEQ ID NO: 1019 - DNA, 66 bp, Artificial
  synthetic
caagcagaagacggcatacgagataactgtatgtctcgtgggctcggagatgtgtataagagacag

SEQ ID NO: 1020 - DNA, 66 bp, Artificial
  synthetic
  misc_feature (27)..(27): n is a, c, g, or t
caagcagaagacggcatacgagatacntgtatgtctcgtgggctcggagatgtgtataagagacag

SEQ ID NO: 1021 - DNA, 66 bp, Artificial
  synthetic
caagcagaagacggcatacgagatagatgtatgtctcgtgggctcggagatgtgtataagagacag

SEQ ID NO: 1022 - DNA, 66 bp, Artificial
  synthetic
caagcagaagacggcatacgagataaatgtatgtctcgtgggctcggagatgtgtataagagacag

SEQ ID NO: 1023 - DNA, 66 bp, Artificial
  synthetic
caagcagaagacggcatacgagatagttctatgtctcgtgggctcggagatgtgtataagagacag

SEQ ID NO: 1024 - DNA, 66 bp, Artificial
  synthetic
caagcagaagacggcatacgagataattctatgtctcgtgggctcggagatgtgtataagagacag

SEQ ID NO: 1025 - DNA, 66 bp, Artificial
  synthetic
caagcagaagacggcatacgagatagctctatgtctcgtgggctcggagatgtgtataagagacag

SEQ ID NO: 1026 - DNA, 66 bp, Artificial
  synthetic
caagcagaagacggcatacgagataactctatgtctcgtgggctcggagatgtgtataagagacag

SEQ ID NO: 1027 - DNA, 66 bp, Artificial
  synthetic
  misc_feature (27)..(27): n is a, c, g, or t
caagcagaagacggcatacgagatacntctatgtctcgtgggctcggagatgtgtataagagacag

SEQ ID NO: 1028 - DNA, 66 bp, Artificial
  synthetic
caagcagaagacggcatacgagatagatctatgtctcgtgggctcggagatgtgtataagagacag

SEQ ID NO: 1029 - DNA, 66 bp, Artificial
  synthetic
caagcagaagacggcatacgagataaatctatgtctcgtgggctcggagatgtgtataagagacag

SEQ ID NO: 1030 - DNA, 66 bp, Artificial
  synthetic
  misc_feature (27)..(27): n is a, c, g, or t
caagcagaagacggcatacgagattcntatatgtctcgtgggctcggagatgtgtataagagacag

SEQ ID NO: 1031 - DNA, 66 bp, Artificial
  synthetic
  misc_feature (27)..(27): n is a, c, g, or t
caagcagaagacggcatacgagatgcntatatgtctcgtgggctcggagatgtgtataagagacag

SEQ ID NO: 1032 - DNA, 66 bp, Artificial
  synthetic
  misc_feature (26)..(27): n is a, c, g, or t
caagcagaagacggcatacgagatanntatatgtctcgtgggctcggagatgtgtataagagacag

SEQ ID NO: 1033 - DNA, 66 bp, Artificial
  synthetic
  misc_feature (27)..(27): n is a, c, g, or t
caagcagaagacggcatacgagatagnttgatgtctcgtgggctcggagatgtgtataagagacag

SEQ ID NO: 1034 - DNA, 66 bp, Artificial
  synthetic
  misc_feature (27)..(27): n is a, c, g, or t
caagcagaagacggcatacgagatacnttgatgtctcgtgggctcggagatgtgtataagagacag

SEQ ID NO: 1035 - DNA, 66 bp, Artificial
  synthetic
  misc_feature (27)..(27): n is a, c, g, or t
caagcagaagacggcatacgagataanttgatgtctcgtgggctcggagatgtgtataagagacag

SEQ ID NO: 1036 - DNA, 66 bp, Artificial
  synthetic
caagcagaagacggcatacgagatagtttcatgtctcgtgggctcggagatgtgtataagagacag

SEQ ID NO: 1037 - DNA, 66 bp, Artificial
  synthetic
caagcagaagacggcatacgagataatttcatgtctcgtgggctcggagatgtgtataagagacag

SEQ ID NO: 1038 - DNA, 66 bp, Artificial
  synthetic
caagcagaagacggcatacgagatagcttcatgtctcgtgggctcggagatgtgtataagagacag

SEQ ID NO: 1039 - DNA, 66 bp, Artificial
  synthetic
caagcagaagacggcatacgagataacttcatgtctcgtgggctcggagatgtgtataagagacag

SEQ ID NO: 1040 - DNA, 66 bp, Artificial
  synthetic
  misc_feature (27)..(27): n is a, c, g, or t
caagcagaagacggcatacgagatacnttcatgtctcgtgggctcggagatgtgtataagagacag

SEQ ID NO: 1041 - DNA, 66 bp, Artificial
  synthetic
caagcagaagacggcatacgagatagattcatgtctcgtgggctcggagatgtgtataagagacag

SEQ ID NO: 1042 - DNA, 66 bp, Artificial
  synthetic
caagcagaagacggcatacgagataaattcatgtctcgtgggctcggagatgtgtataagagacag

SEQ ID NO: 1043 - DNA, 66 bp, Artificial
  synthetic
caagcagaagacggcatacgagattgtttaatgtctcgtgggctcggagatgtgtataagagacag

SEQ ID NO: 1044 - DNA, 66 bp, Artificial
  synthetic
caagcagaagacggcatacgagatggtttaatgtctcgtgggctcggagatgtgtataagagacag

SEQ ID NO: 1045 - DNA, 66 bp, Artificial
  synthetic
caagcagaagacggcatacgagattatttaatgtctcgtgggctcggagatgtgtataagagacag

SEQ ID NO: 1046 - DNA, 66 bp, Artificial
  synthetic
caagcagaagacggcatacgagatgatttaatgtctcgtgggctcggagatgtgtataagagacag

SEQ ID NO: 1047 - DNA, 66 bp, Artificial
  synthetic
caagcagaagacggcatacgagattgcttaatgtctcgtgggctcggagatgtgtataagagacag

SEQ ID NO: 1048 - DNA, 66 bp, Artificial
  synthetic
caagcagaagacggcatacgagatggcttaatgtctcgtgggctcggagatgtgtataagagacag

SEQ ID NO: 1049 - DNA, 66 bp, Artificial
  synthetic
caagcagaagacggcatacgagattacttaatgtctcgtgggctcggagatgtgtataagagacag

SEQ ID NO: 1050 - DNA, 66 bp, Artificial
  synthetic
caagcagaagacggcatacgagatgacttaatgtctcgtgggctcggagatgtgtataagagacag

SEQ ID NO: 1051 - DNA, 66 bp, Artificial
  synthetic
  misc_feature (27)..(27): n is a, c, g, or t
caagcagaagacggcatacgagattcnttaatgtctcgtgggctcggagatgtgtataagagacag

SEQ ID NO: 1052 - DNA, 66 bp, Artificial
  synthetic
  misc_feature (27)..(27): n is a, c, g, or t
caagcagaagacggcatacgagatgcnttaatgtctcgtgggctcggagatgtgtataagagacag

SEQ ID NO: 1053 - DNA, 66 bp, Artificial
  synthetic
  misc_feature (26)..(27): n is a, c, g, or t
caagcagaagacggcatacgagatannttaatgtctcgtgggctcggagatgtgtataagagacag

SEQ ID NO: 1054 - DNA, 66 bp, Artificial
  synthetic
caagcagaagacggcatacgagattgattaatgtctcgtgggctcggagatgtgtataagagacag

SEQ ID NO: 1055 - DNA, 66 bp, Artificial
  synthetic
caagcagaagacggcatacgagatggattaatgtctcgtgggctcggagatgtgtataagagacag

SEQ ID NO: 1056 - DNA, 66 bp, Artificial
  synthetic
caagcagaagacggcatacgagattaattaatgtctcgtgggctcggagatgtgtataagagacag

SEQ ID NO: 1057 - DNA, 66 bp, Artificial
  synthetic
caagcagaagacggcatacgagatgaattaatgtctcgtgggctcggagatgtgtataagagacag

SEQ ID NO: 1058 - DNA, 66 bp, Artificial
  synthetic
caagcagaagacggcatacgagatagttaaatgtctcgtgggctcggagatgtgtataagagacag

SEQ ID NO: 1059 - DNA, 66 bp, Artificial
  synthetic
caagcagaagacggcatacgagataattaaatgtctcgtgggctcggagatgtgtataagagacag

SEQ ID NO: 1060 - DNA, 66 bp, Artificial
  synthetic
caagcagaagacggcatacgagatagctaaatgtctcgtgggctcggagatgtgtataagagacag

SEQ ID NO: 1061 - DNA, 66 bp, Artificial
  synthetic
caagcagaagacggcatacgagataactaaatgtctcgtgggctcggagatgtgtataagagacag

SEQ ID NO: 1062 - DNA, 66 bp, Artificial
  synthetic
  misc_feature (27)..(27): n is a, c, g, or t
caagcagaagacggcatacgagatacntaaatgtctcgtgggctcggagatgtgtataagagacag

SEQ ID NO: 1063 - DNA, 66 bp, Artificial
  synthetic
caagcagaagacggcatacgagatagataaatgtctcgtgggctcggagatgtgtataagagacag

SEQ ID NO: 1064 - DNA, 66 bp, Artificial
  synthetic
caagcagaagacggcatacgagataaataaatgtctcgtgggctcggagatgtgtataagagacag

SEQ ID NO: 1065 - DNA, 66 bp, Artificial
  synthetic
  misc_feature (25)..(30): n is a, c, g, or t
caagcagaagacggcatacgagatnnnnnntggtctcgtgggctcggagatgtgtataagagacag

SEQ ID NO: 1066 - DNA, 66 bp, Artificial
  synthetic
  misc_feature (25)..(30): n is a, c, g, or t
caagcagaagacggcatacgagatnnnnnngggtctcgtgggctcggagatgtgtataagagacag

SEQ ID NO: 1067 - DNA, 66 bp, Artificial
  synthetic
  misc_feature (25)..(29): n is a, c, g, or t
caagcagaagacggcatacgagatnnnnntcggtctcgtgggctcggagatgtgtataagagacag

SEQ ID NO: 1068 - DNA, 66 bp, Artificial
  synthetic
  misc_feature (26)..(27): n is a, c, g, or t
caagcagaagacggcatacgagatcnnctgcggtctcgtgggctcggagatgtgtataagagacag

SEQ ID NO: 1069 - DNA, 66 bp, Artificial
  synthetic
caagcagaagacggcatacgagatcgtcggcggtctcgtgggctcggagatgtgtataagagacag

SEQ ID NO: 1070 - DNA, 66 bp, Artificial
  synthetic
caagcagaagacggcatacgagatcatcggcggtctcgtgggctcggagatgtgtataagagacag

SEQ ID NO: 1071 - DNA, 66 bp, Artificial
  synthetic
caagcagaagacggcatacgagatcgccggcggtctcgtgggctcggagatgtgtataagagacag

SEQ ID NO: 1072 - DNA, 66 bp, Artificial
  synthetic
caagcagaagacggcatacgagatcaccggcggtctcgtgggctcggagatgtgtataagagacag

SEQ ID NO: 1073 - DNA, 66 bp, Artificial
  synthetic
  misc_feature (27)..(27): n is a, c, g, or t
caagcagaagacggcatacgagatccncggcggtctcgtgggctcggagatgtgtataagagacag

SEQ ID NO: 1074 - DNA, 66 bp, Artificial
  synthetic
caagcagaagacggcatacgagatcgacggcggtctcgtgggctcggagatgtgtataagagacag

SEQ ID NO: 1075 - DNA, 66 bp, Artificial
  synthetic
caagcagaagacggcatacgagatcaacggcggtctcgtgggctcggagatgtgtataagagacag

SEQ ID NO: 1076 - DNA, 66 bp, Artificial
  synthetic
  misc_feature (27)..(27): n is a, c, g, or t
caagcagaagacggcatacgagatccnccgcggtctcgtgggctcggagatgtgtataagagacag

SEQ ID NO: 1077 - DNA, 66 bp, Artificial
  synthetic
  misc_feature (25)..(27): n is a, c, g, or t
  misc_feature (29)..(29): n is a, c, g, or t
caagcagaagacggcatacgagatnnntngcggtctcgtgggctcggagatgtgtataagagacag

SEQ ID NO: 1078 - DNA, 66 bp, Artificial
  synthetic
  misc_feature (25)..(27): n is a, c, g, or t
  misc_feature (29)..(29): n is a, c, g, or t
caagcagaagacggcatacgagatnnngngcggtctcgtgggctcggagatgtgtataagagacag

SEQ ID NO: 1079 - DNA, 66 bp, Artificial
  synthetic
  misc_feature (26)..(27): n is a, c, g, or t
  misc_feature (29)..(29): n is a, c, g, or t
caagcagaagacggcatacgagattnncngcggtctcgtgggctcggagatgtgtataagagacag

SEQ ID NO: 1080 - DNA, 66 bp, Artificial
  synthetic
  misc_feature (26)..(27): n is a, c, g, or t
  misc_feature (29)..(29): n is a, c, g, or t
caagcagaagacggcatacgagatgnncngcggtctcgtgggctcggagatgtgtataagagacag

SEQ ID NO: 1081 - DNA, 66 bp, Artificial
  synthetic
  misc_feature (26)..(27): n is a, c, g, or t
  misc_feature (29)..(29): n is a, c, g, or t
caagcagaagacggcatacgagatanncngcggtctcgtgggctcggagatgtgtataagagacag

SEQ ID NO: 1082 - DNA, 66 bp, Artificial
  synthetic
  misc_feature (25)..(27): n is a, c, g, or t
  misc_feature (29)..(29): n is a, c, g, or t
caagcagaagacggcatacgagatnnnangcggtctcgtgggctcggagatgtgtataagagacag

SEQ ID NO: 1083 - DNA, 66 bp, Artificial
  synthetic
  misc_feature (26)..(27): n is a, c, g, or t
caagcagaagacggcatacgagatcnncagcggtctcgtgggctcggagatgtgtataagagacag

SEQ ID NO: 1084 - DNA, 66 bp, Artificial
  synthetic
  misc_feature (26)..(27): n is a, c, g, or t
caagcagaagacggcatacgagatcnnctccggtctcgtgggctcggagatgtgtataagagacag

SEQ ID NO: 1085 - DNA, 66 bp, Artificial
  synthetic
caagcagaagacggcatacgagatcctcgccggtctcgtgggctcggagatgtgtataagagacag

SEQ ID NO: 1086 - DNA, 66 bp, Artificial
  synthetic
caagcagaagacggcatacgagatccccgccggtctcgtgggctcggagatgtgtataagagacag

SEQ ID NO: 1087 - DNA, 66 bp, Artificial
  synthetic
caagcagaagacggcatacgagatccacgccggtctcgtgggctcggagatgtgtataagagacag

SEQ ID NO: 1088 - DNA, 66 bp, Artificial
  synthetic
caagcagaagacggcatacgagatcctccccggtctcgtgggctcggagatgtgtataagagacag

SEQ ID NO: 1089 - DNA, 66 bp, Artificial
  synthetic
caagcagaagacggcatacgagatcccccccggtctcgtgggctcggagatgtgtataagagacag

SEQ ID NO: 1090 - DNA, 66 bp, Artificial
  synthetic
caagcagaagacggcatacgagatccaccccggtctcgtgggctcggagatgtgtataagagacag

SEQ ID NO: 1091 - DNA, 66 bp, Artificial
  synthetic
  misc_feature (25)..(27): n is a, c, g, or t
  misc_feature (29)..(29): n is a, c, g, or t
caagcagaagacggcatacgagatnnntnccggtctcgtgggctcggagatgtgtataagagacag

SEQ ID NO: 1092 - DNA, 66 bp, Artificial
  synthetic
  misc_feature (25)..(27): n is a, c, g, or t
  misc_feature (29)..(29): n is a, c, g, or t
caagcagaagacggcatacgagatnnngnccggtctcgtgggctcggagatgtgtataagagacag

SEQ ID NO: 1093 - DNA, 66 bp, Artificial
  synthetic
  misc_feature (26)..(27): n is a, c, g, or t
  misc_feature (29)..(29): n is a, c, g, or t
caagcagaagacggcatacgagattnncnccggtctcgtgggctcggagatgtgtataagagacag

SEQ ID NO: 1094 - DNA, 66 bp, Artificial
  synthetic
  misc_feature (26)..(27): n is a, c, g, or t
  misc_feature (29)..(29): n is a, c, g, or t
caagcagaagacggcatacgagatgnncnccggtctcgtgggctcggagatgtgtataagagacag

SEQ ID NO: 1095 - DNA, 66 bp, Artificial
  synthetic
  misc_feature (26)..(27): n is a, c, g, or t
  misc_feature (29)..(29): n is a, c, g, or t
caagcagaagacggcatacgagatanncnccggtctcgtgggctcggagatgtgtataagagacag

SEQ ID NO: 1096 - DNA, 66 bp, Artificial
  synthetic
  misc_feature (25)..(27): n is a, c, g, or t
  misc_feature (29)..(29): n is a, c, g, or t
caagcagaagacggcatacgagatnnnanccggtctcgtgggctcggagatgtgtataagagacag

SEQ ID NO: 1097 - DNA, 66 bp, Artificial
  synthetic
  misc_feature (26)..(27): n is a, c, g, or t
caagcagaagacggcatacgagatcnncaccggtctcgtgggctcggagatgtgtataagagacag

SEQ ID NO: 1098 - DNA, 66 bp, Artificial
  synthetic
  misc_feature (25)..(29): n is a, c, g, or t
caagcagaagacggcatacgagatnnnnnacggtctcgtgggctcggagatgtgtataagagacag

SEQ ID NO: 1099 - DNA, 66 bp, Artificial
  synthetic
  misc_feature (25)..(30): n is a, c, g, or t
caagcagaagacggcatacgagatnnnnnnaggtctcgtgggctcggagatgtgtataagagacag

SEQ ID NO: 1100 - DNA, 66 bp, Artificial
  synthetic
  misc_feature (25)..(29): n is a, c, g, or t
caagcagaagacggcatacgagatnnnnnttcgtctcgtgggctcggagatgtgtataagagacag

SEQ ID NO: 1101 - DNA, 66 bp, Artificial
  synthetic
  misc_feature (25)..(29): n is a, c, g, or t
caagcagaagacggcatacgagatnnnnngtcgtctcgtgggctcggagatgtgtataagagacag

SEQ ID NO: 1102 - DNA, 66 bp, Artificial
  synthetic
  misc_feature (26)..(27): n is a, c, g, or t
caagcagaagacggcatacgagatcnnctctcgtctcgtgggctcggagatgtgtataagagacag

SEQ ID NO: 1103 - DNA, 66 bp, Artificial
  synthetic
  misc_feature (26)..(27): n is a, c, g, or t
caagcagaagacggcatacgagatcnncgctcgtctcgtgggctcggagatgtgtataagagacag

SEQ ID NO: 1104 - DNA, 66 bp, Artificial
  synthetic
caagcagaagacggcatacgagatcttccctcgtctcgtgggctcggagatgtgtataagagacag

SEQ ID NO: 1105 - DNA, 66 bp, Artificial
  synthetic
caagcagaagacggcatacgagatctcccctcgtctcgtgggctcggagatgtgtataagagacag

SEQ ID NO: 1106 - DNA, 66 bp, Artificial
  synthetic
  misc_feature (27)..(27): n is a, c, g, or t
caagcagaagacggcatacgagatcgnccctcgtctcgtgggctcggagatgtgtataagagacag

SEQ ID NO: 1107 - DNA, 66 bp, Artificial
  synthetic
  misc_feature (27)..(27): n is a, c, g, or t
caagcagaagacggcatacgagatccnccctcgtctcgtgggctcggagatgtgtataagagacag

SEQ ID NO: 1108 - DNA, 66 bp, Artificial
  synthetic
  misc_feature (27)..(27): n is a, c, g, or t
caagcagaagacggcatacgagatcanccctcgtctcgtgggctcggagatgtgtataagagacag

SEQ ID NO: 1109 - DNA, 66 bp, Artificial
  synthetic
caagcagaagacggcatacgagatctaccctcgtctcgtgggctcggagatgtgtataagagacag

SEQ ID NO: 1110 - DNA, 66 bp, Artificial
  synthetic
  misc_feature (25)..(27): n is a, c, g, or t
  misc_feature (29)..(29): n is a, c, g, or t
caagcagaagacggcatacgagatnnntnctcgtctcgtgggctcggagatgtgtataagagacag

SEQ ID NO: 1111 - DNA, 66 bp, Artificial
  synthetic
  misc_feature (25)..(27): n is a, c, g, or t
  misc_feature (29)..(29): n is a, c, g, or t
caagcagaagacggcatacgagatnnngnctcgtctcgtgggctcggagatgtgtataagagacag

SEQ ID NO: 1112 - DNA, 66 bp, Artificial
  synthetic
  misc_feature (26)..(27): n is a, c, g, or t
  misc_feature (29)..(29): n is a, c, g, or t
caagcagaagacggcatacgagattnncnctcgtctcgtgggctcggagatgtgtataagagacag

SEQ ID NO: 1113 - DNA, 66 bp, Artificial
  synthetic
  misc_feature (26)..(27): n is a, c, g, or t
  misc_feature (29)..(29): n is a, c, g, or t
caagcagaagacggcatacgagatgnncnctcgtctcgtgggctcggagatgtgtataagagacag

SEQ ID NO: 1114 - DNA, 66 bp, Artificial
  synthetic
  misc_feature (26)..(27): n is a, c, g, or t
  misc_feature (29)..(29): n is a, c, g, or t
caagcagaagacggcatacgagatanncnctcgtctcgtgggctcggagatgtgtataagagacag

SEQ ID NO: 1115 - DNA, 66 bp, Artificial
  synthetic
  misc_feature (25)..(27): n is a, c, g, or t
  misc_feature (29)..(29): n is a, c, g, or t
caagcagaagacggcatacgagatnnnanctcgtctcgtgggctcggagatgtgtataagagacag

SEQ ID NO: 1116 - DNA, 66 bp, Artificial
  synthetic
  misc_feature (26)..(27): n is a, c, g, or t
caagcagaagacggcatacgagatcnncactcgtctcgtgggctcggagatgtgtataagagacag

SEQ ID NO: 1117 - DNA, 66 bp, Artificial
  synthetic
  misc_feature (25)..(29): n is a, c, g, or t
caagcagaagacggcatacgagatnnnnnatcgtctcgtgggctcggagatgtgtataagagacag

SEQ ID NO: 1118 - DNA, 66 bp, Artificial
  synthetic
  misc_feature (25)..(29): n is a, c, g, or t
caagcagaagacggcatacgagatnnnnntgcgtctcgtgggctcggagatgtgtataagagacag

SEQ ID NO: 1119 - DNA, 66 bp, Artificial
  synthetic
  misc_feature (26)..(27): n is a, c, g, or t
caagcagaagacggcatacgagatcnngtggcgtctcgtgggctcggagatgtgtataagagacag

SEQ ID NO: 1120 - DNA, 66 bp, Artificial
  synthetic
  misc_feature (26)..(27): n is a, c, g, or t
caagcagaagacggcatacgagattnnctggcgtctcgtgggctcggagatgtgtataagagacag

SEQ ID NO: 1121 - DNA, 66 bp, Artificial
  synthetic
  misc_feature (26)..(27): n is a, c, g, or t
caagcagaagacggcatacgagatgnnctggcgtctcgtgggctcggagatgtgtataagagacag

SEQ ID NO: 1122 - DNA, 66 bp, Artificial
  synthetic
  misc_feature (26)..(27): n is a, c, g, or t
caagcagaagacggcatacgagatcnnctggcgtctcgtgggctcggagatgtgtataagagacag

SEQ ID NO: 1123 - DNA, 66 bp, Artificial
  synthetic
  misc_feature (26)..(27): n is a, c, g, or t
caagcagaagacggcatacgagatcnnatggcgtctcgtgggctcggagatgtgtataagagacag

SEQ ID NO: 1124 - DNA, 66 bp, Artificial
  synthetic
caagcagaagacggcatacgagatcgtggggcgtctcgtgggctcggagatgtgtataagagacag

SEQ ID NO: 1125 - DNA, 66 bp, Artificial
  synthetic
caagcagaagacggcatacgagatcatggggcgtctcgtgggctcggagatgtgtataagagacag

SEQ ID NO: 1126 - DNA, 66 bp, Artificial
  synthetic
caagcagaagacggcatacgagatcgcggggcgtctcgtgggctcggagatgtgtataagagacag

SEQ ID NO: 1127 - DNA, 66 bp, Artificial
  synthetic
caagcagaagacggcatacgagatcacggggcgtctcgtgggctcggagatgtgtataagagacag

SEQ ID NO: 1128 - DNA, 66 bp, Artificial
  synthetic
  misc_feature (27)..(27): n is a, c, g, or t
caagcagaagacggcatacgagatccnggggcgtctcgtgggctcggagatgtgtataagagacag

SEQ ID NO: 1129 - DNA, 66 bp, Artificial
  synthetic
caagcagaagacggcatacgagatcgaggggcgtctcgtgggctcggagatgtgtataagagacag

SEQ ID NO: 1130 - DNA, 66 bp, Artificial
  synthetic
caagcagaagacggcatacgagatcaaggggcgtctcgtgggctcggagatgtgtataagagacag

SEQ ID NO: 1131 - DNA, 66 bp, Artificial
  synthetic
  misc_feature (27)..(27): n is a, c, g, or t
caagcagaagacggcatacgagattgncgggcgtctcgtgggctcggagatgtgtataagagacag

SEQ ID NO: 1132 - DNA, 66 bp, Artificial
  synthetic
  misc_feature (27)..(27): n is a, c, g, or t
caagcagaagacggcatacgagatggncgggcgtctcgtgggctcggagatgtgtataagagacag

SEQ ID NO: 1133 - DNA, 66 bp, Artificial
  synthetic
  misc_feature (27)..(27): n is a, c, g, or t
caagcagaagacggcatacgagattcncgggcgtctcgtgggctcggagatgtgtataagagacag

SEQ ID NO: 1134 - DNA, 66 bp, Artificial
  synthetic
  misc_feature (27)..(27): n is a, c, g, or t
caagcagaagacggcatacgagatgcncgggcgtctcgtgggctcggagatgtgtataagagacag

SEQ ID NO: 1135 - DNA, 66 bp, Artificial
  synthetic
  misc_feature (27)..(27): n is a, c, g, or t
caagcagaagacggcatacgagattancgggcgtctcgtgggctcggagatgtgtataagagacag

SEQ ID NO: 1136 - DNA, 66 bp, Artificial
  synthetic
  misc_feature (27)..(27): n is a, c, g, or t
caagcagaagacggcatacgagatgancgggcgtctcgtgggctcggagatgtgtataagagacag

SEQ ID NO: 1137 - DNA, 66 bp, Artificial
  synthetic
caagcagaagacggcatacgagatcgtagggcgtctcgtgggctcggagatgtgtataagagacag

SEQ ID NO: 1138 - DNA, 66 bp, Artificial
  synthetic
caagcagaagacggcatacgagatcatagggcgtctcgtgggctcggagatgtgtataagagacag

SEQ ID NO: 1139 - DNA, 66 bp, Artificial
  synthetic
caagcagaagacggcatacgagatcgcagggcgtctcgtgggctcggagatgtgtataagagacag

SEQ ID NO: 1140 - DNA, 66 bp, Artificial
  synthetic
caagcagaagacggcatacgagatcacagggcgtctcgtgggctcggagatgtgtataagagacag

SEQ ID NO: 1141 - DNA, 66 bp, Artificial
  synthetic
  misc_feature (27)..(27): n is a, c, g, or t
caagcagaagacggcatacgagatccnagggcgtctcgtgggctcggagatgtgtataagagacag

SEQ ID NO: 1142 - DNA, 66 bp, Artificial
  synthetic
caagcagaagacggcatacgagatcgaagggcgtctcgtgggctcggagatgtgtataagagacag

SEQ ID NO: 1143 - DNA, 66 bp, Artificial
  synthetic
caagcagaagacggcatacgagatcaaagggcgtctcgtgggctcggagatgtgtataagagacag

SEQ ID NO: 1144 - DNA, 66 bp, Artificial
  synthetic
caagcagaagacggcatacgagatcgtgcggcgtctcgtgggctcggagatgtgtataagagacag

SEQ ID NO: 1145 - DNA, 66 bp, Artificial
  synthetic
caagcagaagacggcatacgagatcatgcggcgtctcgtgggctcggagatgtgtataagagacag

SEQ ID NO: 1146 - DNA, 66 bp, Artificial
  synthetic
caagcagaagacggcatacgagatcgcgcggcgtctcgtgggctcggagatgtgtataagagacag

SEQ ID NO: 1147 - DNA, 66 bp, Artificial
  synthetic
caagcagaagacggcatacgagatcacgcggcgtctcgtgggctcggagatgtgtataagagacag

SEQ ID NO: 1148 - DNA, 66 bp, Artificial
  synthetic
  misc_feature (27)..(27): n is a, c, g, or t
caagcagaagacggcatacgagatccngcggcgtctcgtgggctcggagatgtgtataagagacag

SEQ ID NO: 1149 - DNA, 66 bp, Artificial
  synthetic
caagcagaagacggcatacgagatcgagcggcgtctcgtgggctcggagatgtgtataagagacag

SEQ ID NO: 1150 - DNA, 66 bp, Artificial
  synthetic
caagcagaagacggcatacgagatcaagcggcgtctcgtgggctcggagatgtgtataagagacag

SEQ ID NO: 1151 - DNA, 66 bp, Artificial
  synthetic
  misc_feature (27)..(27): n is a, c, g, or t
caagcagaagacggcatacgagattgnccggcgtctcgtgggctcggagatgtgtataagagacag

SEQ ID NO: 1152 - DNA, 66 bp, Artificial
  synthetic
  misc_feature (27)..(27): n is a, c, g, or t
caagcagaagacggcatacgagatggnccggcgtctcgtgggctcggagatgtgtataagagacag

SEQ ID NO: 1153 - DNA, 66 bp, Artificial
  synthetic
  misc_feature (27)..(27): n is a, c, g, or t
caagcagaagacggcatacgagattcnccggcgtctcgtgggctcggagatgtgtataagagacag

SEQ ID NO: 1154 - DNA, 66 bp, Artificial
  synthetic
  misc_feature (27)..(27): n is a, c, g, or t
caagcagaagacggcatacgagatgcnccggcgtctcgtgggctcggagatgtgtataagagacag

SEQ ID NO: 1155 - DNA, 66 bp, Artificial
  synthetic
  misc_feature (27)..(27): n is a, c, g, or t
caagcagaagacggcatacgagattanccggcgtctcgtgggctcggagatgtgtataagagacag

SEQ ID NO: 1156 - DNA, 66 bp, Artificial
  synthetic
  misc_feature (27)..(27): n is a, c, g, or t
caagcagaagacggcatacgagatganccggcgtctcgtgggctcggagatgtgtataagagacag

SEQ ID NO: 1157 - DNA, 66 bp, Artificial
  synthetic
caagcagaagacggcatacgagatcgtacggcgtctcgtgggctcggagatgtgtataagagacag

SEQ ID NO: 1158 - DNA, 66 bp, Artificial
  synthetic
caagcagaagacggcatacgagatcatacggcgtctcgtgggctcggagatgtgtataagagacag

SEQ ID NO: 1159 - DNA, 66 bp, Artificial
  synthetic
caagcagaagacggcatacgagatcgcacggcgtctcgtgggctcggagatgtgtataagagacag

SEQ ID NO: 1160 - DNA, 66 bp, Artificial
  synthetic
caagcagaagacggcatacgagatcacacggcgtctcgtgggctcggagatgtgtataagagacag

SEQ ID NO: 1161 - DNA, 66 bp, Artificial
  synthetic
  misc_feature (27)..(27): n is a, c, g, or t
caagcagaagacggcatacgagatccnacggcgtctcgtgggctcggagatgtgtataagagacag

SEQ ID NO: 1162 - DNA, 66 bp, Artificial
  synthetic
caagcagaagacggcatacgagatcgaacggcgtctcgtgggctcggagatgtgtataagagacag

SEQ ID NO: 1163 - DNA, 66 bp, Artificial
  synthetic
caagcagaagacggcatacgagatcaaacggcgtctcgtgggctcggagatgtgtataagagacag

SEQ ID NO: 1164 - DNA, 66 bp, Artificial
  synthetic
  misc_feature (25)..(27): n is a, c, g, or t
  misc_feature (29)..(29): n is a, c, g, or t
caagcagaagacggcatacgagatnnntnggcgtctcgtgggctcggagatgtgtataagagacag

SEQ ID NO: 1165 - DNA, 66 bp, Artificial
  synthetic
  misc_feature (26)..(27): n is a, c, g, or t
  misc_feature (29)..(29): n is a, c, g, or t
caagcagaagacggcatacgagattnngnggcgtctcgtgggctcggagatgtgtataagagacag

SEQ ID NO: 1166 - DNA, 66 bp, Artificial
  synthetic
  misc_feature (26)..(27): n is a, c, g, or t
  misc_feature (29)..(29): n is a, c, g, or t
caagcagaagacggcatacgagatgnngnggcgtctcgtgggctcggagatgtgtataagagacag

SEQ ID NO: 1167 - DNA, 66 bp, Artificial
  synthetic
  misc_feature (26)..(27): n is a, c, g, or t
  misc_feature (29)..(29): n is a, c, g, or t
caagcagaagacggcatacgagatanngnggcgtctcgtgggctcggagatgtgtataagagacag

SEQ ID NO: 1168 - DNA, 66 bp, Artificial
  synthetic
  misc_feature (26)..(27): n is a, c, g, or t
  misc_feature (29)..(29): n is a, c, g, or t
caagcagaagacggcatacgagatanncnggcgtctcgtgggctcggagatgtgtataagagacag

SEQ ID NO: 1169 - DNA, 66 bp, Artificial
  synthetic
  misc_feature (26)..(27): n is a, c, g, or t
  misc_feature (29)..(29): n is a, c, g, or t
caagcagaagacggcatacgagattnnanggcgtctcgtgggctcggagatgtgtataagagacag

SEQ ID NO: 1170 - DNA, 66 bp, Artificial
  synthetic
  misc_feature (26)..(27): n is a, c, g, or t
  misc_feature (29)..(29): n is a, c, g, or t
caagcagaagacggcatacgagatgnnanggcgtctcgtgggctcggagatgtgtataagagacag

SEQ ID NO: 1171 - DNA, 66 bp, Artificial
  synthetic
  misc_feature (26)..(27): n is a, c, g, or t
  misc_feature (29)..(29): n is a, c, g, or t
caagcagaagacggcatacgagatannanggcgtctcgtgggctcggagatgtgtataagagacag

SEQ ID NO: 1172 - DNA, 66 bp, Artificial
  synthetic
  misc_feature (26)..(27): n is a, c, g, or t
caagcagaagacggcatacgagatcnngaggcgtctcgtgggctcggagatgtgtataagagacag

SEQ ID NO: 1173 - DNA, 66 bp, Artificial
  synthetic
  misc_feature (27)..(27): n is a, c, g, or t
caagcagaagacggcatacgagatccncaggcgtctcgtgggctcggagatgtgtataagagacag

SEQ ID NO: 1174 - DNA, 66 bp, Artificial
  synthetic
  misc_feature (26)..(27): n is a, c, g, or t
caagcagaagacggcatacgagattnncaggcgtctcgtgggctcggagatgtgtataagagacag

SEQ ID NO: 1175 - DNA, 66 bp, Artificial
  synthetic
  misc_feature (26)..(27): n is a, c, g, or t
caagcagaagacggcatacgagatgnncaggcgtctcgtgggctcggagatgtgtataagagacag

SEQ ID NO: 1176 - DNA, 66 bp, Artificial
  synthetic
  misc_feature (26)..(27): n is a, c, g, or t
caagcagaagacggcatacgagatcnnaaggcgtctcgtgggctcggagatgtgtataagagacag

SEQ ID NO: 1177 - DNA, 66 bp, Artificial
  synthetic
  misc_feature (26)..(27): n is a, c, g, or t
caagcagaagacggcatacgagatcnngtcgcgtctcgtgggctcggagatgtgtataagagacag

SEQ ID NO: 1178 - DNA, 66 bp, Artificial
  synthetic
  misc_feature (26)..(27): n is a, c, g, or t
caagcagaagacggcatacgagattnnctcgcgtctcgtgggctcggagatgtgtataagagacag

SEQ ID NO: 1179 - DNA, 66 bp, Artificial
  synthetic
  misc_feature (26)..(27): n is a, c, g, or t
caagcagaagacggcatacgagatgnnctcgcgtctcgtgggctcggagatgtgtataagagacag

SEQ ID NO: 1180 - DNA, 66 bp, Artificial
  synthetic
  misc_feature (26)..(27): n is a, c, g, or t
caagcagaagacggcatacgagatcnnctcgcgtctcgtgggctcggagatgtgtataagagacag

SEQ ID NO: 1181 - DNA, 66 bp, Artificial
  synthetic
  misc_feature (26)..(27): n is a, c, g, or t
caagcagaagacggcatacgagatcnnatcgcgtctcgtgggctcggagatgtgtataagagacag

SEQ ID NO: 1182 - DNA, 66 bp, Artificial
  synthetic
  misc_feature (27)..(27): n is a, c, g, or t
caagcagaagacggcatacgagatccnggcgcgtctcgtgggctcggagatgtgtataagagacag

SEQ ID NO: 1183 - DNA, 66 bp, Artificial
  synthetic
  misc_feature (27)..(27): n is a, c, g, or t
caagcagaagacggcatacgagattgncgcgcgtctcgtgggctcggagatgtgtataagagacag

SEQ ID NO: 1184 - DNA, 66 bp, Artificial
  synthetic
  misc_feature (27)..(27): n is a, c, g, or t
caagcagaagacggcatacgagatggncgcgcgtctcgtgggctcggagatgtgtataagagacag

SEQ ID NO: 1185 - DNA, 66 bp, Artificial
  synthetic
  misc_feature (27)..(27): n is a, c, g, or t
caagcagaagacggcatacgagattcncgcgcgtctcgtgggctcggagatgtgtataagagacag

SEQ ID NO: 1186 - DNA, 66 bp, Artificial
  synthetic
  misc_feature (27)..(27): n is a, c, g, or t
caagcagaagacggcatacgagatgcncgcgcgtctcgtgggctcggagatgtgtataagagacag

SEQ ID NO: 1187 - DNA, 66 bp, Artificial
  synthetic
  misc_feature (27)..(27): n is a, c, g, or t
caagcagaagacggcatacgagattancgcgcgtctcgtgggctcggagatgtgtataagagacag

SEQ ID NO: 1188 - DNA, 66 bp, Artificial
  synthetic
  misc_feature (27)..(27): n is a, c, g, or t
caagcagaagacggcatacgagatgancgcgcgtctcgtgggctcggagatgtgtataagagacag

SEQ ID NO: 1189 - DNA, 66 bp, Artificial
  synthetic
  misc_feature (27)..(27): n is a, c, g, or t
caagcagaagacggcatacgagatccnagcgcgtctcgtgggctcggagatgtgtataagagacag

SEQ ID NO: 1190 - DNA, 66 bp, Artificial
  synthetic
caagcagaagacggcatacgagatcctgccgcgtctcgtgggctcggagatgtgtataagagacag

SEQ ID NO: 1191 - DNA, 66 bp, Artificial
  synthetic
caagcagaagacggcatacgagatcccgccgcgtctcgtgggctcggagatgtgtataagagacag

SEQ ID NO: 1192 - DNA, 66 bp, Artificial
  synthetic
caagcagaagacggcatacgagatccagccgcgtctcgtgggctcggagatgtgtataagagacag

SEQ ID NO: 1193 - DNA, 66 bp, Artificial
  synthetic
  misc_feature (27)..(27): n is a, c, g, or t
caagcagaagacggcatacgagattgncccgcgtctcgtgggctcggagatgtgtataagagacag

SEQ ID NO: 1194 - DNA, 66 bp, Artificial
  synthetic
  misc_feature (27)..(27): n is a, c, g, or t
caagcagaagacggcatacgagatggncccgcgtctcgtgggctcggagatgtgtataagagacag

SEQ ID NO: 1195 - DNA, 66 bp, Artificial
  synthetic
  misc_feature (27)..(27): n is a, c, g, or t
caagcagaagacggcatacgagattcncccgcgtctcgtgggctcggagatgtgtataagagacag

SEQ ID NO: 1196 - DNA, 66 bp, Artificial
  synthetic
  misc_feature (27)..(27): n is a, c, g, or t
caagcagaagacggcatacgagatgcncccgcgtctcgtgggctcggagatgtgtataagagacag

SEQ ID NO: 1197 - DNA, 66 bp, Artificial
  synthetic
  misc_feature (27)..(27): n is a, c, g, or t
caagcagaagacggcatacgagattancccgcgtctcgtgggctcggagatgtgtataagagacag

SEQ ID NO: 1198 - DNA, 66 bp, Artificial
  synthetic
  misc_feature (27)..(27): n is a, c, g, or t
caagcagaagacggcatacgagatgancccgcgtctcgtgggctcggagatgtgtataagagacag

SEQ ID NO: 1199 - DNA, 66 bp, Artificial
  synthetic
caagcagaagacggcatacgagatcctaccgcgtctcgtgggctcggagatgtgtataagagacag

SEQ ID NO: 1200 - DNA, 66 bp, Artificial
  synthetic
caagcagaagacggcatacgagatcccaccgcgtctcgtgggctcggagatgtgtataagagacag

SEQ ID NO: 1201 - DNA, 66 bp, Artificial
  synthetic
caagcagaagacggcatacgagatccaaccgcgtctcgtgggctcggagatgtgtataagagacag

SEQ ID NO: 1202 - DNA, 66 bp, Artificial
  synthetic
  misc_feature (25)..(27): n is a, c, g, or t
  misc_feature (29)..(29): n is a, c, g, or t
caagcagaagacggcatacgagatnnntncgcgtctcgtgggctcggagatgtgtataagagacag

SEQ ID NO: 1203 - DNA, 66 bp, Artificial
  synthetic
  misc_feature (26)..(27): n is a, c, g, or t
  misc_feature (29)..(29): n is a, c, g, or t
caagcagaagacggcatacgagattnngncgcgtctcgtgggctcggagatgtgtataagagacag

SEQ ID NO: 1204 - DNA, 66 bp, Artificial
  synthetic
  misc_feature (26)..(27): n is a, c, g, or t
  misc_feature (29)..(29): n is a, c, g, or t
caagcagaagacggcatacgagatgnngncgcgtctcgtgggctcggagatgtgtataagagacag

SEQ ID NO: 1205 - DNA, 66 bp, Artificial
  synthetic
  misc_feature (26)..(27): n is a, c, g, or t
  misc_feature (29)..(29): n is a, c, g, or t
caagcagaagacggcatacgagatanngncgcgtctcgtgggctcggagatgtgtataagagacag

SEQ ID NO: 1206 - DNA, 66 bp, Artificial
  synthetic
  misc_feature (26)..(27): n is a, c, g, or t
  misc_feature (29)..(29): n is a, c, g, or t
caagcagaagacggcatacgagatanncncgcgtctcgtgggctcggagatgtgtataagagacag

SEQ ID NO: 1207 - DNA, 66 bp, Artificial
  synthetic
  misc_feature (26)..(27): n is a, c, g, or t
  misc_feature (29)..(29): n is a, c, g, or t
caagcagaagacggcatacgagattnnancgcgtctcgtgggctcggagatgtgtataagagacag

SEQ ID NO: 1208 - DNA, 66 bp, Artificial
  synthetic
  misc_feature (26)..(27): n is a, c, g, or t
  misc_feature (29)..(29): n is a, c, g, or t
caagcagaagacggcatacgagatgnnancgcgtctcgtgggctcggagatgtgtataagagacag

SEQ ID NO: 1209 - DNA, 66 bp, Artificial
  synthetic
  misc_feature (26)..(27): n is a, c, g, or t
  misc_feature (29)..(29): n is a, c, g, or t
caagcagaagacggcatacgagatannancgcgtctcgtgggctcggagatgtgtataagagacag

SEQ ID NO: 1210 - DNA, 66 bp, Artificial
  synthetic
  misc_feature (26)..(27): n is a, c, g, or t
caagcagaagacggcatacgagatcnngacgcgtctcgtgggctcggagatgtgtataagagacag

SEQ ID NO: 1211 - DNA, 66 bp, Artificial
  synthetic
caagcagaagacggcatacgagatcctcacgcgtctcgtgggctcggagatgtgtataagagacag

SEQ ID NO: 1212 - DNA, 66 bp, Artificial
  synthetic
caagcagaagacggcatacgagatccccacgcgtctcgtgggctcggagatgtgtataagagacag

SEQ ID NO: 1213 - DNA, 66 bp, Artificial
  synthetic
  misc_feature (26)..(27): n is a, c, g, or t
caagcagaagacggcatacgagattnncacgcgtctcgtgggctcggagatgtgtataagagacag

SEQ ID NO: 1214 - DNA, 66 bp, Artificial
  synthetic
  misc_feature (26)..(27): n is a, c, g, or t
caagcagaagacggcatacgagatgnncacgcgtctcgtgggctcggagatgtgtataagagacag

SEQ ID NO: 1215 - DNA, 66 bp, Artificial
  synthetic
caagcagaagacggcatacgagatccacacgcgtctcgtgggctcggagatgtgtataagagacag

SEQ ID NO: 1216 - DNA, 66 bp, Artificial
  synthetic
  misc_feature (26)..(27): n is a, c, g, or t
caagcagaagacggcatacgagatcnnaacgcgtctcgtgggctcggagatgtgtataagagacag

SEQ ID NO: 1217 - DNA, 66 bp, Artificial
  synthetic
  misc_feature (26)..(27): n is a, c, g, or t
caagcagaagacggcatacgagatcnnctagcgtctcgtgggctcggagatgtgtataagagacag

SEQ ID NO: 1218 - DNA, 66 bp, Artificial
  synthetic
caagcagaagacggcatacgagatcgtcgagcgtctcgtgggctcggagatgtgtataagagacag

SEQ ID NO: 1219 - DNA, 66 bp, Artificial
  synthetic
caagcagaagacggcatacgagatcatcgagcgtctcgtgggctcggagatgtgtataagagacag

SEQ ID NO: 1220 - DNA, 66 bp, Artificial
  synthetic
caagcagaagacggcatacgagatcgccgagcgtctcgtgggctcggagatgtgtataagagacag

SEQ ID NO: 1221 - DNA, 66 bp, Artificial
  synthetic
caagcagaagacggcatacgagatcaccgagcgtctcgtgggctcggagatgtgtataagagacag

SEQ ID NO: 1222 - DNA, 66 bp, Artificial
  synthetic
  misc_feature (27)..(27): n is a, c, g, or t
caagcagaagacggcatacgagatccncgagcgtctcgtgggctcggagatgtgtataagagacag

SEQ ID NO: 1223 - DNA, 66 bp, Artificial
  synthetic
caagcagaagacggcatacgagatcgacgagcgtctcgtgggctcggagatgtgtataagagacag

SEQ ID NO: 1224 - DNA, 66 bp, Artificial
  synthetic
caagcagaagacggcatacgagatcaacgagcgtctcgtgggctcggagatgtgtataagagacag

SEQ ID NO: 1225 - DNA, 66 bp, Artificial
  synthetic
  misc_feature (27)..(27): n is a, c, g, or t
caagcagaagacggcatacgagatccnccagcgtctcgtgggctcggagatgtgtataagagacag

SEQ ID NO: 1226 - DNA, 66 bp, Artificial
  synthetic
  misc_feature (25)..(27): n is a, c, g, or t
  misc_feature (29)..(29): n is a, c, g, or t
caagcagaagacggcatacgagatnnntnagcgtctcgtgggctcggagatgtgtataagagacag

SEQ ID NO: 1227 - DNA, 66 bp, Artificial
  synthetic
  misc_feature (25)..(27): n is a, c, g, or t
  misc_feature (29)..(29): n is a, c, g, or t
caagcagaagacggcatacgagatnnngnagcgtctcgtgggctcggagatgtgtataagagacag

SEQ ID NO: 1228 - DNA, 66 bp, Artificial
  synthetic
  misc_feature (26)..(27): n is a, c, g, or t
  misc_feature (29)..(29): n is a, c, g, or t
caagcagaagacggcatacgagattnncnagcgtctcgtgggctcggagatgtgtataagagacag

SEQ ID NO: 1229 - DNA, 66 bp, Artificial
  synthetic
  misc_feature (26)..(27): n is a, c, g, or t
  misc_feature (29)..(29): n is a, c, g, or t
caagcagaagacggcatacgagatgnncnagcgtctcgtgggctcggagatgtgtataagagacag

SEQ ID NO: 1230 - DNA, 66 bp, Artificial
  synthetic
  misc_feature (26)..(27): n is a, c, g, or t
  misc_feature (29)..(29): n is a, c, g, or t
caagcagaagacggcatacgagatanncnagcgtctcgtgggctcggagatgtgtataagagacag

SEQ ID NO: 1231 - DNA, 66 bp, Artificial
  synthetic
  misc_feature (25)..(27): n is a, c, g, or t
  misc_feature (29)..(29): n is a, c, g, or t
caagcagaagacggcatacgagatnnnanagcgtctcgtgggctcggagatgtgtataagagacag

SEQ ID NO: 1232 - DNA, 66 bp, Artificial
  synthetic
  misc_feature (26)..(27): n is a, c, g, or t
caagcagaagacggcatacgagatcnncaagcgtctcgtgggctcggagatgtgtataagagacag

SEQ ID NO: 1233 - DNA, 66 bp, Artificial
  synthetic
  misc_feature (26)..(27): n is a, c, g, or t
caagcagaagacggcatacgagatcnngttccgtctcgtgggctcggagatgtgtataagagacag

SEQ ID NO: 1234 - DNA, 66 bp, Artificial
  synthetic
  misc_feature (26)..(27): n is a, c, g, or t
caagcagaagacggcatacgagattnncttccgtctcgtgggctcggagatgtgtataagagacag

SEQ ID NO: 1235 - DNA, 66 bp, Artificial
  synthetic
  misc_feature (26)..(27): n is a, c, g, or t
caagcagaagacggcatacgagatgnncttccgtctcgtgggctcggagatgtgtataagagacag

SEQ ID NO: 1236 - DNA, 66 bp, Artificial
  synthetic
  misc_feature (26)..(27): n is a, c, g, or t
caagcagaagacggcatacgagatcnncttccgtctcgtgggctcggagatgtgtataagagacag

SEQ ID NO: 1237 - DNA, 66 bp, Artificial
  synthetic
  misc_feature (26)..(27): n is a, c, g, or t
caagcagaagacggcatacgagatcnnattccgtctcgtgggctcggagatgtgtataagagacag

SEQ ID NO: 1238 - DNA, 66 bp, Artificial
  synthetic
caagcagaagacggcatacgagatcgtggtccgtctcgtgggctcggagatgtgtataagagacag

SEQ ID NO: 1239 - DNA, 66 bp, Artificial
  synthetic
caagcagaagacggcatacgagatcatggtccgtctcgtgggctcggagatgtgtataagagacag

SEQ ID NO: 1240 - DNA, 66 bp, Artificial
  synthetic
caagcagaagacggcatacgagatcgcggtccgtctcgtgggctcggagatgtgtataagagacag

SEQ ID NO: 1241 - DNA, 66 bp, Artificial
  synthetic
caagcagaagacggcatacgagatcacggtccgtctcgtgggctcggagatgtgtataagagacag

SEQ ID NO: 1242 - DNA, 66 bp, Artificial
  synthetic
  misc_feature (27)..(27): n is a, c, g, or t
caagcagaagacggcatacgagatccnggtccgtctcgtgggctcggagatgtgtataagagacag

SEQ ID NO: 1243 - DNA, 66 bp, Artificial
  synthetic
caagcagaagacggcatacgagatcgaggtccgtctcgtgggctcggagatgtgtataagagacag

SEQ ID NO: 1244 - DNA, 66 bp, Artificial
  synthetic
caagcagaagacggcatacgagatcaaggtccgtctcgtgggctcggagatgtgtataagagacag

SEQ ID NO: 1245 - DNA, 66 bp, Artificial
  synthetic
  misc_feature (27)..(27): n is a, c, g, or t
caagcagaagacggcatacgagattgncgtccgtctcgtgggctcggagatgtgtataagagacag

SEQ ID NO: 1246 - DNA, 66 bp, Artificial
  synthetic
  misc_feature (27)..(27): n is a, c, g, or t
caagcagaagacggcatacgagatggncgtccgtctcgtgggctcggagatgtgtataagagacag

SEQ ID NO: 1247 - DNA, 66 bp, Artificial
  synthetic
  misc_feature (27)..(27): n is a, c, g, or t
caagcagaagacggcatacgagattcncgtccgtctcgtgggctcggagatgtgtataagagacag

SEQ ID NO: 1248 - DNA, 66 bp, Artificial
  synthetic
  misc_feature (27)..(27): n is a, c, g, or t
caagcagaagacggcatacgagatgcncgtccgtctcgtgggctcggagatgtgtataagagacag

SEQ ID NO: 1249 - DNA, 66 bp, Artificial
  synthetic
  misc_feature (27)..(27): n is a, c, g, or t
caagcagaagacggcatacgagattancgtccgtctcgtgggctcggagatgtgtataagagacag

SEQ ID NO: 1250 - DNA, 66 bp, Artificial
  synthetic
  misc_feature (27)..(27): n is a, c, g, or t
caagcagaagacggcatacgagatgancgtccgtctcgtgggctcggagatgtgtataagagacag

SEQ ID NO: 1251 - DNA, 66 bp, Artificial
  synthetic
caagcagaagacggcatacgagatcgtagtccgtctcgtgggctcggagatgtgtataagagacag

SEQ ID NO: 1252 - DNA, 66 bp, Artificial
  synthetic
caagcagaagacggcatacgagatcatagtccgtctcgtgggctcggagatgtgtataagagacag

SEQ ID NO: 1253 - DNA, 66 bp, Artificial
  synthetic
caagcagaagacggcatacgagatcgcagtccgtctcgtgggctcggagatgtgtataagagacag

SEQ ID NO: 1254 - DNA, 66 bp, Artificial
  synthetic
caagcagaagacggcatacgagatcacagtccgtctcgtgggctcggagatgtgtataagagacag

SEQ ID NO: 1255 - DNA, 66 bp, Artificial
  synthetic
  misc_feature (27)..(27): n is a, c, g, or t
caagcagaagacggcatacgagatccnagtccgtctcgtgggctcggagatgtgtataagagacag

SEQ ID NO: 1256 - DNA, 66 bp, Artificial
  synthetic
caagcagaagacggcatacgagatcgaagtccgtctcgtgggctcggagatgtgtataagagacag

SEQ ID NO: 1257 - DNA, 66 bp, Artificial
  synthetic
caagcagaagacggcatacgagatcaaagtccgtctcgtgggctcggagatgtgtataagagacag

SEQ ID NO: 1258 - DNA, 66 bp, Artificial
  synthetic
  misc_feature (27)..(27): n is a, c, g, or t
caagcagaagacggcatacgagatccngctccgtctcgtgggctcggagatgtgtataagagacag

SEQ ID NO: 1259 - DNA, 66 bp, Artificial
  synthetic
  misc_feature (27)..(27): n is a, c, g, or t
caagcagaagacggcatacgagattgncctccgtctcgtgggctcggagatgtgtataagagacag

SEQ ID NO: 1260 - DNA, 66 bp, Artificial
  synthetic
  misc_feature (27)..(27): n is a, c, g, or t
caagcagaagacggcatacgagatggncctccgtctcgtgggctcggagatgtgtataagagacag

SEQ ID NO: 1261 - DNA, 66 bp, Artificial
  synthetic
  misc_feature (27)..(27): n is a, c, g, or t
caagcagaagacggcatacgagattcncctccgtctcgtgggctcggagatgtgtataagagacag

SEQ ID NO: 1262 - DNA, 66 bp, Artificial
  synthetic
  misc_feature (27)..(27): n is a, c, g, or t
caagcagaagacggcatacgagatgcncctccgtctcgtgggctcggagatgtgtataagagacag

SEQ ID NO: 1263 - DNA, 66 bp, Artificial
  synthetic
  misc_feature (27)..(27): n is a, c, g, or t
caagcagaagacggcatacgagattancctccgtctcgtgggctcggagatgtgtataagagacag

SEQ ID NO: 1264 - DNA, 66 bp, Artificial
  synthetic
  misc_feature (27)..(27): n is a, c, g, or t
caagcagaagacggcatacgagatgancctccgtctcgtgggctcggagatgtgtataagagacag

SEQ ID NO: 1265 - DNA, 66 bp, Artificial
  synthetic
  misc_feature (27)..(27): n is a, c, g, or t
caagcagaagacggcatacgagatccnactccgtctcgtgggctcggagatgtgtataagagacag

SEQ ID NO: 1266 - DNA, 66 bp, Artificial
  synthetic
  misc_feature (25)..(27): n is a, c, g, or t
  misc_feature (29)..(29): n is a, c, g, or t
caagcagaagacggcatacgagatnnntntccgtctcgtgggctcggagatgtgtataagagacag

SEQ ID NO: 1267 - DNA, 66 bp, Artificial
  synthetic
  misc_feature (26)..(27): n is a, c, g, or t
  misc_feature (29)..(29): n is a, c, g, or t
caagcagaagacggcatacgagattnngntccgtctcgtgggctcggagatgtgtataagagacag

SEQ ID NO: 1268 - DNA, 66 bp, Artificial
  synthetic
  misc_feature (26)..(27): n is a, c, g, or t
  misc_feature (29)..(29): n is a, c, g, or t
caagcagaagacggcatacgagatgnngntccgtctcgtgggctcggagatgtgtataagagacag

SEQ ID NO: 1269 - DNA, 66 bp, Artificial
  synthetic
  misc_feature (26)..(27): n is a, c, g, or t
  misc_feature (29)..(29): n is a, c, g, or t
caagcagaagacggcatacgagatanngntccgtctcgtgggctcggagatgtgtataagagacag

SEQ ID NO: 1270 - DNA, 66 bp, Artificial
  synthetic
  misc_feature (26)..(27): n is a, c, g, or t
  misc_feature (29)..(29): n is a, c, g, or t
caagcagaagacggcatacgagatanncntccgtctcgtgggctcggagatgtgtataagagacag

SEQ ID NO: 1271 - DNA, 66 bp, Artificial
  synthetic
  misc_feature (26)..(27): n is a, c, g, or t
  misc_feature (29)..(29): n is a, c, g, or t
caagcagaagacggcatacgagattnnantccgtctcgtgggctcggagatgtgtataagagacag

SEQ ID NO: 1272 - DNA, 66 bp, Artificial
  synthetic
  misc_feature (26)..(27): n is a, c, g, or t
  misc_feature (29)..(29): n is a, c, g, or t
caagcagaagacggcatacgagatgnnantccgtctcgtgggctcggagatgtgtataagagacag

SEQ ID NO: 1273 - DNA, 66 bp, Artificial
  synthetic
  misc_feature (26)..(27): n is a, c, g, or t
  misc_feature (29)..(29): n is a, c, g, or t
caagcagaagacggcatacgagatannantccgtctcgtgggctcggagatgtgtataagagacag

SEQ ID NO: 1274 - DNA, 66 bp, Artificial
  synthetic
  misc_feature (26)..(27): n is a, c, g, or t
caagcagaagacggcatacgagatcnngatccgtctcgtgggctcggagatgtgtataagagacag

SEQ ID NO: 1275 - DNA, 66 bp, Artificial
  synthetic
caagcagaagacggcatacgagatcctcatccgtctcgtgggctcggagatgtgtataagagacag

SEQ ID NO: 1276 - DNA, 66 bp, Artificial
  synthetic
caagcagaagacggcatacgagatccccatccgtctcgtgggctcggagatgtgtataagagacag

SEQ ID NO: 1277 - DNA, 66 bp, Artificial
  synthetic
  misc_feature (26)..(27): n is a, c, g, or t
caagcagaagacggcatacgagattnncatccgtctcgtgggctcggagatgtgtataagagacag

SEQ ID NO: 1278 - DNA, 66 bp, Artificial
  synthetic
  misc_feature (26)..(27): n is a, c, g, or t
caagcagaagacggcatacgagatgnncatccgtctcgtgggctcggagatgtgtataagagacag

SEQ ID NO: 1279 - DNA, 66 bp, Artificial
  synthetic
caagcagaagacggcatacgagatccacatccgtctcgtgggctcggagatgtgtataagagacag

SEQ ID NO: 1280 - DNA, 66 bp, Artificial
  synthetic
  misc_feature (26)..(27): n is a, c, g, or t
caagcagaagacggcatacgagatcnnaatccgtctcgtgggctcggagatgtgtataagagacag

SEQ ID NO: 1281 - DNA, 66 bp, Artificial
  synthetic
  misc_feature (26)..(27): n is a, c, g, or t
caagcagaagacggcatacgagatcnnttgccgtctcgtgggctcggagatgtgtataagagacag

SEQ ID NO: 1282 - DNA, 66 bp, Artificial
  synthetic
caagcagaagacggcatacgagatcgtgtgccgtctcgtgggctcggagatgtgtataagagacag

SEQ ID NO: 1283 - DNA, 66 bp, Artificial
  synthetic
caagcagaagacggcatacgagatcatgtgccgtctcgtgggctcggagatgtgtataagagacag

SEQ ID NO: 1284 - DNA, 66 bp, Artificial
  synthetic
caagcagaagacggcatacgagatcgcgtgccgtctcgtgggctcggagatgtgtataagagacag

SEQ ID NO: 1285 - DNA, 66 bp, Artificial
  synthetic
caagcagaagacggcatacgagatcacgtgccgtctcgtgggctcggagatgtgtataagagacag

SEQ ID NO: 1286 - DNA, 66 bp, Artificial
  synthetic
  misc_feature (27)..(27): n is a, c, g, or t
caagcagaagacggcatacgagatccngtgccgtctcgtgggctcggagatgtgtataagagacag

SEQ ID NO: 1287 - DNA, 66 bp, Artificial
  synthetic
  misc_feature (26)..(27): n is a, c, g, or t
caagcagaagacggcatacgagattnngtgccgtctcgtgggctcggagatgtgtataagagacag

SEQ ID NO: 1288 - DNA, 66 bp, Artificial
  synthetic
  misc_feature (26)..(27): n is a, c, g, or t
caagcagaagacggcatacgagatgnngtgccgtctcgtgggctcggagatgtgtataagagacag

SEQ ID NO: 1289 - DNA, 66 bp, Artificial
  synthetic
  misc_feature (26)..(27): n is a, c, g, or t
caagcagaagacggcatacgagatanngtgccgtctcgtgggctcggagatgtgtataagagacag

SEQ ID NO: 1290 - DNA, 66 bp, Artificial
  synthetic
caagcagaagacggcatacgagatcgagtgccgtctcgtgggctcggagatgtgtataagagacag

SEQ ID NO: 1291 - DNA, 66 bp, Artificial
  synthetic
caagcagaagacggcatacgagatcaagtgccgtctcgtgggctcggagatgtgtataagagacag

SEQ ID NO: 1292 - DNA, 66 bp, Artificial
  synthetic
  misc_feature (27)..(27): n is a, c, g, or t
caagcagaagacggcatacgagattgnctgccgtctcgtgggctcggagatgtgtataagagacag

SEQ ID NO: 1293 - DNA, 66 bp, Artificial
  synthetic
  misc_feature (27)..(27): n is a, c, g, or t
caagcagaagacggcatacgagatggnctgccgtctcgtgggctcggagatgtgtataagagacag

SEQ ID NO: 1294 - DNA, 66 bp, Artificial
  synthetic
  misc_feature (27)..(27): n is a, c, g, or t
caagcagaagacggcatacgagattcnctgccgtctcgtgggctcggagatgtgtataagagacag

SEQ ID NO: 1295 - DNA, 66 bp, Artificial
  synthetic
  misc_feature (27)..(27): n is a, c, g, or t
caagcagaagacggcatacgagatgcnctgccgtctcgtgggctcggagatgtgtataagagacag

SEQ ID NO: 1296 - DNA, 66 bp, Artificial
  synthetic
  misc_feature (26)..(27): n is a, c, g, or t
caagcagaagacggcatacgagatannctgccgtctcgtgggctcggagatgtgtataagagacag

SEQ ID NO: 1297 - DNA, 66 bp, Artificial
  synthetic
  misc_feature (27)..(27): n is a, c, g, or t
caagcagaagacggcatacgagattanctgccgtctcgtgggctcggagatgtgtataagagacag

SEQ ID NO: 1298 - DNA, 66 bp, Artificial
  synthetic
  misc_feature (27)..(27): n is a, c, g, or t
caagcagaagacggcatacgagatganctgccgtctcgtgggctcggagatgtgtataagagacag

SEQ ID NO: 1299 - DNA, 66 bp, Artificial
  synthetic
caagcagaagacggcatacgagatcgtatgccgtctcgtgggctcggagatgtgtataagagacag

SEQ ID NO: 1300 - DNA, 66 bp, Artificial
  synthetic
caagcagaagacggcatacgagatcatatgccgtctcgtgggctcggagatgtgtataagagacag

SEQ ID NO: 1301 - DNA, 66 bp, Artificial
  synthetic
caagcagaagacggcatacgagatcgcatgccgtctcgtgggctcggagatgtgtataagagacag

SEQ ID NO: 1302 - DNA, 66 bp, Artificial
  synthetic
caagcagaagacggcatacgagatcacatgccgtctcgtgggctcggagatgtgtataagagacag

SEQ ID NO: 1303 - DNA, 66 bp, Artificial
  synthetic
  misc_feature (27)..(27): n is a, c, g, or t
caagcagaagacggcatacgagatccnatgccgtctcgtgggctcggagatgtgtataagagacag

SEQ ID NO: 1304 - DNA, 66 bp, Artificial
  synthetic
  misc_feature (26)..(27): n is a, c, g, or t
caagcagaagacggcatacgagattnnatgccgtctcgtgggctcggagatgtgtataagagacag

SEQ ID NO: 1305 - DNA, 66 bp, Artificial
  synthetic
  misc_feature (26)..(27): n is a, c, g, or t
caagcagaagacggcatacgagatgnnatgccgtctcgtgggctcggagatgtgtataagagacag

SEQ ID NO: 1306 - DNA, 66 bp, Artificial
  synthetic
  misc_feature (26)..(27): n is a, c, g, or t
caagcagaagacggcatacgagatannatgccgtctcgtgggctcggagatgtgtataagagacag

SEQ ID NO: 1307 - DNA, 66 bp, Artificial
  synthetic
caagcagaagacggcatacgagatcgaatgccgtctcgtgggctcggagatgtgtataagagacag

SEQ ID NO: 1308 - DNA, 66 bp, Artificial
  synthetic
caagcagaagacggcatacgagatcaaatgccgtctcgtgggctcggagatgtgtataagagacag

SEQ ID NO: 1309 - DNA, 66 bp, Artificial
  synthetic
  misc_feature (27)..(27): n is a, c, g, or t
caagcagaagacggcatacgagatagngggccgtctcgtgggctcggagatgtgtataagagacag

SEQ ID NO: 1310 - DNA, 66 bp, Artificial
  synthetic
  misc_feature (27)..(27): n is a, c, g, or t
caagcagaagacggcatacgagatacngggccgtctcgtgggctcggagatgtgtataagagacag

SEQ ID NO: 1311 - DNA, 66 bp, Artificial
  synthetic
  misc_feature (27)..(27): n is a, c, g, or t
caagcagaagacggcatacgagataangggccgtctcgtgggctcggagatgtgtataagagacag

SEQ ID NO: 1312 - DNA, 66 bp, Artificial
  synthetic
  misc_feature (27)..(27): n is a, c, g, or t
caagcagaagacggcatacgagatagnaggccgtctcgtgggctcggagatgtgtataagagacag

SEQ ID NO: 1313 - DNA, 66 bp, Artificial
  synthetic
  misc_feature (27)..(27): n is a, c, g, or t
caagcagaagacggcatacgagatacnaggccgtctcgtgggctcggagatgtgtataagagacag

SEQ ID NO: 1314 - DNA, 66 bp, Artificial
  synthetic
  misc_feature (27)..(27): n is a, c, g, or t
caagcagaagacggcatacgagataanaggccgtctcgtgggctcggagatgtgtataagagacag

SEQ ID NO: 1315 - DNA, 66 bp, Artificial
  synthetic
  misc_feature (27)..(27): n is a, c, g, or t
caagcagaagacggcatacgagatagngcgccgtctcgtgggctcggagatgtgtataagagacag

SEQ ID NO: 1316 - DNA, 66 bp, Artificial
  synthetic
  misc_feature (27)..(27): n is a, c, g, or t
caagcagaagacggcatacgagatacngcgccgtctcgtgggctcggagatgtgtataagagacag

SEQ ID NO: 1317 - DNA, 66 bp, Artificial
  synthetic
  misc_feature (27)..(27): n is a, c, g, or t
caagcagaagacggcatacgagataangcgccgtctcgtgggctcggagatgtgtataagagacag

SEQ ID NO: 1318 - DNA, 66 bp, Artificial
  synthetic
  misc_feature (27)..(27): n is a, c, g, or t
caagcagaagacggcatacgagatagnacgccgtctcgtgggctcggagatgtgtataagagacag

SEQ ID NO: 1319 - DNA, 66 bp, Artificial
  synthetic
  misc_feature (27)..(27): n is a, c, g, or t
caagcagaagacggcatacgagatacnacgccgtctcgtgggctcggagatgtgtataagagacag

SEQ ID NO: 1320 - DNA, 66 bp, Artificial
  synthetic
  misc_feature (27)..(27): n is a, c, g, or t
caagcagaagacggcatacgagataanacgccgtctcgtgggctcggagatgtgtataagagacag

SEQ ID NO: 1321 - DNA, 66 bp, Artificial
  synthetic
  misc_feature (26)..(27): n is a, c, g, or t
  misc_feature (29)..(29): n is a, c, g, or t
caagcagaagacggcatacgagattnntngccgtctcgtgggctcggagatgtgtataagagacag

SEQ ID NO: 1322 - DNA, 66 bp, Artificial
  synthetic
  misc_feature (26)..(27): n is a, c, g, or t
  misc_feature (29)..(29): n is a, c, g, or t
caagcagaagacggcatacgagatgnntngccgtctcgtgggctcggagatgtgtataagagacag

SEQ ID NO: 1323 - DNA, 66 bp, Artificial
  synthetic
  misc_feature (26)..(27): n is a, c, g, or t
  misc_feature (29)..(29): n is a, c, g, or t
caagcagaagacggcatacgagatanntngccgtctcgtgggctcggagatgtgtataagagacag

SEQ ID NO: 1324 - DNA, 66 bp, Artificial
  synthetic
  misc_feature (27)..(27): n is a, c, g, or t
caagcagaagacggcatacgagatcgntagccgtctcgtgggctcggagatgtgtataagagacag

SEQ ID NO: 1325 - DNA, 66 bp, Artificial
  synthetic
  misc_feature (27)..(27): n is a, c, g, or t
caagcagaagacggcatacgagatccntagccgtctcgtgggctcggagatgtgtataagagacag

SEQ ID NO: 1326 - DNA, 66 bp, Artificial
  synthetic
  misc_feature (27)..(27): n is a, c, g, or t
caagcagaagacggcatacgagatcantagccgtctcgtgggctcggagatgtgtataagagacag

SEQ ID NO: 1327 - DNA, 66 bp, Artificial
  synthetic
  misc_feature (27)..(27): n is a, c, g, or t
caagcagaagacggcatacgagattgngagccgtctcgtgggctcggagatgtgtataagagacag

SEQ ID NO: 1328 - DNA, 66 bp, Artificial
  synthetic
  misc_feature (27)..(27): n is a, c, g, or t
caagcagaagacggcatacgagatggngagccgtctcgtgggctcggagatgtgtataagagacag

SEQ ID NO: 1329 - DNA, 66 bp, Artificial
  synthetic
  misc_feature (27)..(27): n is a, c, g, or t
caagcagaagacggcatacgagattcngagccgtctcgtgggctcggagatgtgtataagagacag

SEQ ID NO: 1330 - DNA, 66 bp, Artificial
  synthetic
  misc_feature (27)..(27): n is a, c, g, or t
caagcagaagacggcatacgagatgcngagccgtctcgtgggctcggagatgtgtataagagacag

SEQ ID NO: 1331 - DNA, 66 bp, Artificial
  synthetic
  misc_feature (26)..(27): n is a, c, g, or t
caagcagaagacggcatacgagatanngagccgtctcgtgggctcggagatgtgtataagagacag

SEQ ID NO: 1332 - DNA, 66 bp, Artificial
  synthetic
  misc_feature (27)..(27): n is a, c, g, or t
caagcagaagacggcatacgagattangagccgtctcgtgggctcggagatgtgtataagagacag

SEQ ID NO: 1333 - DNA, 66 bp, Artificial
  synthetic
  misc_feature (27)..(27): n is a, c, g, or t
caagcagaagacggcatacgagatgangagccgtctcgtgggctcggagatgtgtataagagacag

SEQ ID NO: 1334 - DNA, 66 bp, Artificial
  synthetic
  misc_feature (27)..(27): n is a, c, g, or t
caagcagaagacggcatacgagatagncagccgtctcgtgggctcggagatgtgtataagagacag

SEQ ID NO: 1335 - DNA, 66 bp, Artificial
  synthetic
  misc_feature (27)..(27): n is a, c, g, or t
caagcagaagacggcatacgagatacncagccgtctcgtgggctcggagatgtgtataagagacag

SEQ ID NO: 1336 - DNA, 66 bp, Artificial
  synthetic
  misc_feature (27)..(27): n is a, c, g, or t
caagcagaagacggcatacgagataancagccgtctcgtgggctcggagatgtgtataagagacag

SEQ ID NO: 1337 - DNA, 66 bp, Artificial
  synthetic
  misc_feature (27)..(27): n is a, c, g, or t
caagcagaagacggcatacgagattgnaagccgtctcgtgggctcggagatgtgtataagagacag

SEQ ID NO: 1338 - DNA, 66 bp, Artificial
  synthetic
  misc_feature (27)..(27): n is a, c, g, or t
caagcagaagacggcatacgagatggnaagccgtctcgtgggctcggagatgtgtataagagacag

SEQ ID NO: 1339 - DNA, 66 bp, Artificial
  synthetic
  misc_feature (27)..(27): n is a, c, g, or t
caagcagaagacggcatacgagattcnaagccgtctcgtgggctcggagatgtgtataagagacag

SEQ ID NO: 1340 - DNA, 66 bp, Artificial
  synthetic
  misc_feature (27)..(27): n is a, c, g, or t
caagcagaagacggcatacgagatgcnaagccgtctcgtgggctcggagatgtgtataagagacag

SEQ ID NO: 1341 - DNA, 66 bp, Artificial
  synthetic
  misc_feature (26)..(27): n is a, c, g, or t
caagcagaagacggcatacgagatannaagccgtctcgtgggctcggagatgtgtataagagacag

SEQ ID NO: 1342 - DNA, 66 bp, Artificial
  synthetic
  misc_feature (27)..(27): n is a, c, g, or t
caagcagaagacggcatacgagattanaagccgtctcgtgggctcggagatgtgtataagagacag

SEQ ID NO: 1343 - DNA, 66 bp, Artificial
  synthetic
  misc_feature (27)..(27): n is a, c, g, or t
caagcagaagacggcatacgagatganaagccgtctcgtgggctcggagatgtgtataagagacag

SEQ ID NO: 1344 - DNA, 66 bp, Artificial
  synthetic
  misc_feature (26)..(27): n is a, c, g, or t
caagcagaagacggcatacgagatcnnttcccgtctcgtgggctcggagatgtgtataagagacag

SEQ ID NO: 1345 - DNA, 66 bp, Artificial
  synthetic
  misc_feature (27)..(27): n is a, c, g, or t
caagcagaagacggcatacgagatccngtcccgtctcgtgggctcggagatgtgtataagagacag

SEQ ID NO: 1346 - DNA, 66 bp, Artificial
  synthetic
  misc_feature (26)..(27): n is a, c, g, or t
caagcagaagacggcatacgagattnngtcccgtctcgtgggctcggagatgtgtataagagacag

SEQ ID NO: 1347 - DNA, 66 bp, Artificial
  synthetic
  misc_feature (26)..(27): n is a, c, g, or t
caagcagaagacggcatacgagatgnngtcccgtctcgtgggctcggagatgtgtataagagacag

SEQ ID NO: 1348 - DNA, 66 bp, Artificial
  synthetic
  misc_feature (26)..(27): n is a, c, g, or t
caagcagaagacggcatacgagatanngtcccgtctcgtgggctcggagatgtgtataagagacag

SEQ ID NO: 1349 - DNA, 66 bp, Artificial
  synthetic
  misc_feature (27)..(27): n is a, c, g, or t
caagcagaagacggcatacgagattgnctcccgtctcgtgggctcggagatgtgtataagagacag

SEQ ID NO: 1350 - DNA, 66 bp, Artificial
  synthetic
  misc_feature (27)..(27): n is a, c, g, or t
caagcagaagacggcatacgagatggnctcccgtctcgtgggctcggagatgtgtataagagacag

SEQ ID NO: 1351 - DNA, 66 bp, Artificial
  synthetic
  misc_feature (27)..(27): n is a, c, g, or t
caagcagaagacggcatacgagattcnctcccgtctcgtgggctcggagatgtgtataagagacag

SEQ ID NO: 1352 - DNA, 66 bp, Artificial
  synthetic
  misc_feature (27)..(27): n is a, c, g, or t
caagcagaagacggcatacgagatgcnctcccgtctcgtgggctcggagatgtgtataagagacag

SEQ ID NO: 1353 - DNA, 66 bp, Artificial
  synthetic
  misc_feature (26)..(27): n is a, c, g, or t
caagcagaagacggcatacgagatannctcccgtctcgtgggctcggagatgtgtataagagacag

SEQ ID NO: 1354 - DNA, 66 bp, Artificial
  synthetic
  misc_feature (27)..(27): n is a, c, g, or t
caagcagaagacggcatacgagattanctcccgtctcgtgggctcggagatgtgtataagagacag

SEQ ID NO: 1355 - DNA, 66 bp, Artificial
  synthetic
  misc_feature (27)..(27): n is a, c, g, or t
caagcagaagacggcatacgagatganctcccgtctcgtgggctcggagatgtgtataagagacag

SEQ ID NO: 1356 - DNA, 66 bp, Artificial
  synthetic
  misc_feature (27)..(27): n is a, c, g, or t
caagcagaagacggcatacgagatccnatcccgtctcgtgggctcggagatgtgtataagagacag

SEQ ID NO: 1357 - DNA, 66 bp, Artificial
  synthetic
  misc_feature (26)..(27): n is a, c, g, or t
caagcagaagacggcatacgagattnnatcccgtctcgtgggctcggagatgtgtataagagacag

SEQ ID NO: 1358 - DNA, 66 bp, Artificial
  synthetic
  misc_feature (26)..(27): n is a, c, g, or t
caagcagaagacggcatacgagatgnnatcccgtctcgtgggctcggagatgtgtataagagacag

SEQ ID NO: 1359 - DNA, 66 bp, Artificial
  synthetic
  misc_feature (26)..(27): n is a, c, g, or t
caagcagaagacggcatacgagatannatcccgtctcgtgggctcggagatgtgtataagagacag

SEQ ID NO: 1360 - DNA, 66 bp, Artificial
  synthetic
  misc_feature (27)..(27): n is a, c, g, or t
caagcagaagacggcatacgagatagnggcccgtctcgtgggctcggagatgtgtataagagacag

SEQ ID NO: 1361 - DNA, 66 bp, Artificial
  synthetic
  misc_feature (27)..(27): n is a, c, g, or t
caagcagaagacggcatacgagatacnggcccgtctcgtgggctcggagatgtgtataagagacag

SEQ ID NO: 1362 - DNA, 66 bp, Artificial
  synthetic
  misc_feature (27)..(27): n is a, c, g, or t
caagcagaagacggcatacgagataanggcccgtctcgtgggctcggagatgtgtataagagacag

SEQ ID NO: 1363 - DNA, 66 bp, Artificial
  synthetic
  misc_feature (27)..(27): n is a, c, g, or t
caagcagaagacggcatacgagatagnagcccgtctcgtgggctcggagatgtgtataagagacag

SEQ ID NO: 1364 - DNA, 66 bp, Artificial
  synthetic
  misc_feature (27)..(27): n is a, c, g, or t
caagcagaagacggcatacgagatacnagcccgtctcgtgggctcggagatgtgtataagagacag

SEQ ID NO: 1365 - DNA, 66 bp, Artificial
  synthetic
  misc_feature (27)..(27): n is a, c, g, or t
caagcagaagacggcatacgagataanagcccgtctcgtgggctcggagatgtgtataagagacag

SEQ ID NO: 1366 - DNA, 66 bp, Artificial
  synthetic
  misc_feature (27)..(27): n is a, c, g, or t
caagcagaagacggcatacgagatagngccccgtctcgtgggctcggagatgtgtataagagacag

SEQ ID NO: 1367 - DNA, 66 bp, Artificial
  synthetic
  misc_feature (27)..(27): n is a, c, g, or t
caagcagaagacggcatacgagatacngccccgtctcgtgggctcggagatgtgtataagagacag

SEQ ID NO: 1368 - DNA, 66 bp, Artificial
  synthetic
  misc_feature (27)..(27): n is a, c, g, or t
caagcagaagacggcatacgagataangccccgtctcgtgggctcggagatgtgtataagagacag

SEQ ID NO: 1369 - DNA, 66 bp, Artificial
  synthetic
  misc_feature (27)..(27): n is a, c, g, or t
caagcagaagacggcatacgagatagnaccccgtctcgtgggctcggagatgtgtataagagacag

SEQ ID NO: 1370 - DNA, 66 bp, Artificial
  synthetic
  misc_feature (27)..(27): n is a, c, g, or t
caagcagaagacggcatacgagatacnaccccgtctcgtgggctcggagatgtgtataagagacag

SEQ ID NO: 1371 - DNA, 66 bp, Artificial
  synthetic
  misc_feature (27)..(27): n is a, c, g, or t
caagcagaagacggcatacgagataanaccccgtctcgtgggctcggagatgtgtataagagacag

SEQ ID NO: 1372 - DNA, 66 bp, Artificial
  synthetic
  misc_feature (26)..(27): n is a, c, g, or t
  misc_feature (29)..(29): n is a, c, g, or t
caagcagaagacggcatacgagattnntncccgtctcgtgggctcggagatgtgtataagagacag

SEQ ID NO: 1373 - DNA, 66 bp, Artificial
  synthetic
  misc_feature (26)..(27): n is a, c, g, or t
  misc_feature (29)..(29): n is a, c, g, or t
caagcagaagacggcatacgagatgnntncccgtctcgtgggctcggagatgtgtataagagacag

SEQ ID NO: 1374 - DNA, 66 bp, Artificial
  synthetic
  misc_feature (26)..(27): n is a, c, g, or t
  misc_feature (29)..(29): n is a, c, g, or t
caagcagaagacggcatacgagatanntncccgtctcgtgggctcggagatgtgtataagagacag

SEQ ID NO: 1375 - DNA, 66 bp, Artificial
  synthetic
  misc_feature (27)..(27): n is a, c, g, or t
caagcagaagacggcatacgagatcgntacccgtctcgtgggctcggagatgtgtataagagacag

SEQ ID NO: 1376 - DNA, 66 bp, Artificial
  synthetic
  misc_feature (27)..(27): n is a, c, g, or t
caagcagaagacggcatacgagatccntacccgtctcgtgggctcggagatgtgtataagagacag

SEQ ID NO: 1377 - DNA, 66 bp, Artificial
  synthetic
  misc_feature (27)..(27): n is a, c, g, or t
caagcagaagacggcatacgagatcantacccgtctcgtgggctcggagatgtgtataagagacag

SEQ ID NO: 1378 - DNA, 66 bp, Artificial
  synthetic
  misc_feature (27)..(27): n is a, c, g, or t
caagcagaagacggcatacgagattgngacccgtctcgtgggctcggagatgtgtataagagacag

SEQ ID NO: 1379 - DNA, 66 bp, Artificial
  synthetic
  misc_feature (27)..(27): n is a, c, g, or t
caagcagaagacggcatacgagatggngacccgtctcgtgggctcggagatgtgtataagagacag

SEQ ID NO: 1380 - DNA, 66 bp, Artificial
  synthetic
  misc_feature (27)..(27): n is a, c, g, or t
caagcagaagacggcatacgagattcngacccgtctcgtgggctcggagatgtgtataagagacag

SEQ ID NO: 1381 - DNA, 66 bp, Artificial
  synthetic
  misc_feature (27)..(27): n is a, c, g, or t
caagcagaagacggcatacgagatgcngacccgtctcgtgggctcggagatgtgtataagagacag

SEQ ID NO: 1382 - DNA, 66 bp, Artificial
  synthetic
  misc_feature (26)..(27): n is a, c, g, or t
caagcagaagacggcatacgagatanngacccgtctcgtgggctcggagatgtgtataagagacag

SEQ ID NO: 1383 - DNA, 66 bp, Artificial
  synthetic
  misc_feature (27)..(27): n is a, c, g, or t
caagcagaagacggcatacgagattangacccgtctcgtgggctcggagatgtgtataagagacag

SEQ ID NO: 1384 - DNA, 66 bp, Artificial
  synthetic
  misc_feature (27)..(27): n is a, c, g, or t
caagcagaagacggcatacgagatgangacccgtctcgtgggctcggagatgtgtataagagacag

SEQ ID NO: 1385 - DNA, 66 bp, Artificial
  synthetic
  misc_feature (27)..(27): n is a, c, g, or t
caagcagaagacggcatacgagatagncacccgtctcgtgggctcggagatgtgtataagagacag

SEQ ID NO: 1386 - DNA, 66 bp, Artificial
  synthetic
  misc_feature (27)..(27): n is a, c, g, or t
caagcagaagacggcatacgagatacncacccgtctcgtgggctcggagatgtgtataagagacag

SEQ ID NO: 1387 - DNA, 66 bp, Artificial
  synthetic
  misc_feature (27)..(27): n is a, c, g, or t
caagcagaagacggcatacgagataancacccgtctcgtgggctcggagatgtgtataagagacag

SEQ ID NO: 1388 - DNA, 66 bp, Artificial
  synthetic
  misc_feature (27)..(27): n is a, c, g, or t
caagcagaagacggcatacgagattgnaacccgtctcgtgggctcggagatgtgtataagagacag

SEQ ID NO: 1389 - DNA, 66 bp, Artificial
  synthetic
  misc_feature (27)..(27): n is a, c, g, or t
caagcagaagacggcatacgagatggnaacccgtctcgtgggctcggagatgtgtataagagacag

SEQ ID NO: 1390 - DNA, 66 bp, Artificial
  synthetic
  misc_feature (27)..(27): n is a, c, g, or t
caagcagaagacggcatacgagattcnaacccgtctcgtgggctcggagatgtgtataagagacag

SEQ ID NO: 1391 - DNA, 66 bp, Artificial
  synthetic
  misc_feature (27)..(27): n is a, c, g, or t
caagcagaagacggcatacgagatgcnaacccgtctcgtgggctcggagatgtgtataagagacag

SEQ ID NO: 1392 - DNA, 66 bp, Artificial
  synthetic
  misc_feature (26)..(27): n is a, c, g, or t
caagcagaagacggcatacgagatannaacccgtctcgtgggctcggagatgtgtataagagacag

SEQ ID NO: 1393 - DNA, 66 bp, Artificial
  synthetic
  misc_feature (27)..(27): n is a, c, g, or t
caagcagaagacggcatacgagattanaacccgtctcgtgggctcggagatgtgtataagagacag

SEQ ID NO: 1394 - DNA, 66 bp, Artificial
  synthetic
  misc_feature (27)..(27): n is a, c, g, or t
caagcagaagacggcatacgagatganaacccgtctcgtgggctcggagatgtgtataagagacag

SEQ ID NO: 1395 - DNA, 66 bp, Artificial
  synthetic
  misc_feature (26)..(27): n is a, c, g, or t
caagcagaagacggcatacgagatcnnttaccgtctcgtgggctcggagatgtgtataagagacag

SEQ ID NO: 1396 - DNA, 66 bp, Artificial
  synthetic
  misc_feature (26)..(27): n is a, c, g, or t
caagcagaagacggcatacgagattnngtaccgtctcgtgggctcggagatgtgtataagagacag

SEQ ID NO: 1397 - DNA, 66 bp, Artificial
  synthetic
  misc_feature (26)..(27): n is a, c, g, or t
caagcagaagacggcatacgagatgnngtaccgtctcgtgggctcggagatgtgtataagagacag

SEQ ID NO: 1398 - DNA, 66 bp, Artificial
  synthetic
  misc_feature (26)..(27): n is a, c, g, or t
caagcagaagacggcatacgagatcnngtaccgtctcgtgggctcggagatgtgtataagagacag

SEQ ID NO: 1399 - DNA, 66 bp, Artificial
  synthetic
caagcagaagacggcatacgagatcgtctaccgtctcgtgggctcggagatgtgtataagagacag

SEQ ID NO: 1400 - DNA, 66 bp, Artificial
  synthetic
caagcagaagacggcatacgagatcatctaccgtctcgtgggctcggagatgtgtataagagacag

SEQ ID NO: 1401 - DNA, 66 bp, Artificial
  synthetic
caagcagaagacggcatacgagatcgcctaccgtctcgtgggctcggagatgtgtataagagacag

SEQ ID NO: 1402 - DNA, 66 bp, Artificial
  synthetic
caagcagaagacggcatacgagatcacctaccgtctcgtgggctcggagatgtgtataagagacag

SEQ ID NO: 1403 - DNA, 66 bp, Artificial
  synthetic
  misc_feature (27)..(27): n is a, c, g, or t
caagcagaagacggcatacgagatccnctaccgtctcgtgggctcggagatgtgtataagagacag

SEQ ID NO: 1404 - DNA, 66 bp, Artificial
  synthetic
  misc_feature (26)..(27): n is a, c, g, or t
caagcagaagacggcatacgagattnnctaccgtctcgtgggctcggagatgtgtataagagacag

SEQ ID NO: 1405 - DNA, 66 bp, Artificial
  synthetic
  misc_feature (26)..(27): n is a, c, g, or t
caagcagaagacggcatacgagatgnnctaccgtctcgtgggctcggagatgtgtataagagacag

SEQ ID NO: 1406 - DNA, 66 bp, Artificial
  synthetic
  misc_feature (26)..(27): n is a, c, g, or t
caagcagaagacggcatacgagatannctaccgtctcgtgggctcggagatgtgtataagagacag

SEQ ID NO: 1407 - DNA, 66 bp, Artificial
  synthetic
caagcagaagacggcatacgagatcgactaccgtctcgtgggctcggagatgtgtataagagacag

SEQ ID NO: 1408 - DNA, 66 bp, Artificial
  synthetic
caagcagaagacggcatacgagatcaactaccgtctcgtgggctcggagatgtgtataagagacag

SEQ ID NO: 1409 - DNA, 66 bp, Artificial
  synthetic
  misc_feature (26)..(27): n is a, c, g, or t
caagcagaagacggcatacgagattnnataccgtctcgtgggctcggagatgtgtataagagacag

SEQ ID NO: 1410 - DNA, 66 bp, Artificial
  synthetic
  misc_feature (26)..(27): n is a, c, g, or t
caagcagaagacggcatacgagatgnnataccgtctcgtgggctcggagatgtgtataagagacag

SEQ ID NO: 1411 - DNA, 66 bp, Artificial
  synthetic
  misc_feature (26)..(27): n is a, c, g, or t
caagcagaagacggcatacgagatcnnataccgtctcgtgggctcggagatgtgtataagagacag

SEQ ID NO: 1412 - DNA, 66 bp, Artificial
  synthetic
  misc_feature (27)..(27): n is a, c, g, or t
caagcagaagacggcatacgagatcgntgaccgtctcgtgggctcggagatgtgtataagagacag

SEQ ID NO: 1413 - DNA, 66 bp, Artificial
  synthetic
  misc_feature (27)..(27): n is a, c, g, or t
caagcagaagacggcatacgagatccntgaccgtctcgtgggctcggagatgtgtataagagacag

SEQ ID NO: 1414 - DNA, 66 bp, Artificial
  synthetic
  misc_feature (27)..(27): n is a, c, g, or t
caagcagaagacggcatacgagatcantgaccgtctcgtgggctcggagatgtgtataagagacag

SEQ ID NO: 1415 - DNA, 66 bp, Artificial
  synthetic
  misc_feature (27)..(27): n is a, c, g, or t
caagcagaagacggcatacgagattgnggaccgtctcgtgggctcggagatgtgtataagagacag

SEQ ID NO: 1416 - DNA, 66 bp, Artificial
  synthetic
  misc_feature (27)..(27): n is a, c, g, or t
caagcagaagacggcatacgagatggnggaccgtctcgtgggctcggagatgtgtataagagacag

SEQ ID NO: 1417 - DNA, 66 bp, Artificial
  synthetic
  misc_feature (27)..(27): n is a, c, g, or t
caagcagaagacggcatacgagattcnggaccgtctcgtgggctcggagatgtgtataagagacag

SEQ ID NO: 1418 - DNA, 66 bp, Artificial
  synthetic
  misc_feature (27)..(27): n is a, c, g, or t
caagcagaagacggcatacgagatgcnggaccgtctcgtgggctcggagatgtgtataagagacag

SEQ ID NO: 1419 - DNA, 66 bp, Artificial
  synthetic
  misc_feature (27)..(27): n is a, c, g, or t
caagcagaagacggcatacgagattanggaccgtctcgtgggctcggagatgtgtataagagacag

SEQ ID NO: 1420 - DNA, 66 bp, Artificial
  synthetic
  misc_feature (27)..(27): n is a, c, g, or t
caagcagaagacggcatacgagatganggaccgtctcgtgggctcggagatgtgtataagagacag

SEQ ID NO: 1421 - DNA, 66 bp, Artificial
  synthetic
  misc_feature (27)..(27): n is a, c, g, or t
caagcagaagacggcatacgagatagncgaccgtctcgtgggctcggagatgtgtataagagacag

SEQ ID NO: 1422 - DNA, 66 bp, Artificial
  synthetic
  misc_feature (27)..(27): n is a, c, g, or t
caagcagaagacggcatacgagatacncgaccgtctcgtgggctcggagatgtgtataagagacag

SEQ ID NO: 1423 - DNA, 66 bp, Artificial
  synthetic
  misc_feature (27)..(27): n is a, c, g, or t
caagcagaagacggcatacgagataancgaccgtctcgtgggctcggagatgtgtataagagacag

SEQ ID NO: 1424 - DNA, 66 bp, Artificial
  synthetic
  misc_feature (27)..(27): n is a, c, g, or t
caagcagaagacggcatacgagattgnagaccgtctcgtgggctcggagatgtgtataagagacag

SEQ ID NO: 1425 - DNA, 66 bp, Artificial
  synthetic
  misc_feature (27)..(27): n is a, c, g, or t
caagcagaagacggcatacgagatggnagaccgtctcgtgggctcggagatgtgtataagagacag

SEQ ID NO: 1426 - DNA, 66 bp, Artificial
  synthetic
  misc_feature (27)..(27): n is a, c, g, or t
caagcagaagacggcatacgagattcnagaccgtctcgtgggctcggagatgtgtataagagacag

SEQ ID NO: 1427 - DNA, 66 bp, Artificial
  synthetic
  misc_feature (27)..(27): n is a, c, g, or t
caagcagaagacggcatacgagatgcnagaccgtctcgtgggctcggagatgtgtataagagacag

SEQ ID NO: 1428 - DNA, 66 bp, Artificial
  synthetic
  misc_feature (27)..(27): n is a, c, g, or t
caagcagaagacggcatacgagattanagaccgtctcgtgggctcggagatgtgtataagagacag

SEQ ID NO: 1429 - DNA, 66 bp, Artificial
  synthetic
  misc_feature (27)..(27): n is a, c, g, or t
caagcagaagacggcatacgagatganagaccgtctcgtgggctcggagatgtgtataagagacag

SEQ ID NO: 1430 - DNA, 66 bp, Artificial
  synthetic
  misc_feature (27)..(27): n is a, c, g, or t
caagcagaagacggcatacgagatcgntcaccgtctcgtgggctcggagatgtgtataagagacag

SEQ ID NO: 1431 - DNA, 66 bp, Artificial
  synthetic
  misc_feature (27)..(27): n is a, c, g, or t
caagcagaagacggcatacgagatccntcaccgtctcgtgggctcggagatgtgtataagagacag

SEQ ID NO: 1432 - DNA, 66 bp, Artificial
  synthetic
  misc_feature (27)..(27): n is a, c, g, or t
caagcagaagacggcatacgagatcantcaccgtctcgtgggctcggagatgtgtataagagacag

SEQ ID NO: 1433 - DNA, 66 bp, Artificial
  synthetic
  misc_feature (27)..(27): n is a, c, g, or t
caagcagaagacggcatacgagattgngcaccgtctcgtgggctcggagatgtgtataagagacag

SEQ ID NO: 1434 - DNA, 66 bp, Artificial
  synthetic
  misc_feature (27)..(27): n is a, c, g, or t
caagcagaagacggcatacgagatggngcaccgtctcgtgggctcggagatgtgtataagagacag

SEQ ID NO: 1435 - DNA, 66 bp, Artificial
  synthetic
  misc_feature (27)..(27): n is a, c, g, or t
caagcagaagacggcatacgagattcngcaccgtctcgtgggctcggagatgtgtataagagacag

SEQ ID NO: 1436 - DNA, 66 bp, Artificial
  synthetic
  misc_feature (27)..(27): n is a, c, g, or t
caagcagaagacggcatacgagatgcngcaccgtctcgtgggctcggagatgtgtataagagacag

SEQ ID NO: 1437 - DNA, 66 bp, Artificial
  synthetic
  misc_feature (27)..(27): n is a, c, g, or t
caagcagaagacggcatacgagattangcaccgtctcgtgggctcggagatgtgtataagagacag

SEQ ID NO: 1438 - DNA, 66 bp, Artificial
  synthetic
  misc_feature (27)..(27): n is a, c, g, or t
caagcagaagacggcatacgagatgangcaccgtctcgtgggctcggagatgtgtataagagacag

SEQ ID NO: 1439 - DNA, 66 bp, Artificial
  synthetic
  misc_feature (27)..(27): n is a, c, g, or t
caagcagaagacggcatacgagatagnccaccgtctcgtgggctcggagatgtgtataagagacag

SEQ ID NO: 1440 - DNA, 66 bp, Artificial
  synthetic
  misc_feature (27)..(27): n is a, c, g, or t
caagcagaagacggcatacgagatacnccaccgtctcgtgggctcggagatgtgtataagagacag

SEQ ID NO: 1441 - DNA, 66 bp, Artificial
  synthetic
  misc_feature (27)..(27): n is a, c, g, or t
caagcagaagacggcatacgagataanccaccgtctcgtgggctcggagatgtgtataagagacag

SEQ ID NO: 1442 - DNA, 66 bp, Artificial
  synthetic
  misc_feature (27)..(27): n is a, c, g, or t
caagcagaagacggcatacgagattgnacaccgtctcgtgggctcggagatgtgtataagagacag

SEQ ID NO: 1443 - DNA, 66 bp, Artificial
  synthetic
  misc_feature (27)..(27): n is a, c, g, or t
caagcagaagacggcatacgagatggnacaccgtctcgtgggctcggagatgtgtataagagacag

SEQ ID NO: 1444 - DNA, 66 bp, Artificial
  synthetic
  misc_feature (27)..(27): n is a, c, g, or t
caagcagaagacggcatacgagattcnacaccgtctcgtgggctcggagatgtgtataagagacag

SEQ ID NO: 1445 - DNA, 66 bp, Artificial
  synthetic
  misc_feature (27)..(27): n is a, c, g, or t
caagcagaagacggcatacgagatgcnacaccgtctcgtgggctcggagatgtgtataagagacag

SEQ ID NO: 1446 - DNA, 66 bp, Artificial
  synthetic
  misc_feature (27)..(27): n is a, c, g, or t
caagcagaagacggcatacgagattanacaccgtctcgtgggctcggagatgtgtataagagacag

SEQ ID NO: 1447 - DNA, 66 bp, Artificial
  synthetic
  misc_feature (27)..(27): n is a, c, g, or t
caagcagaagacggcatacgagatganacaccgtctcgtgggctcggagatgtgtataagagacag

SEQ ID NO: 1448 - DNA, 66 bp, Artificial
  synthetic
  misc_feature (26)..(27): n is a, c, g, or t
  misc_feature (29)..(29): n is a, c, g, or t
caagcagaagacggcatacgagattnntnaccgtctcgtgggctcggagatgtgtataagagacag

SEQ ID NO: 1449 - DNA, 66 bp, Artificial
  synthetic
  misc_feature (26)..(27): n is a, c, g, or t
  misc_feature (29)..(29): n is a, c, g, or t
caagcagaagacggcatacgagatgnntnaccgtctcgtgggctcggagatgtgtataagagacag

SEQ ID NO: 1450 - DNA, 66 bp, Artificial
  synthetic
  misc_feature (26)..(27): n is a, c, g, or t
  misc_feature (29)..(29): n is a, c, g, or t
caagcagaagacggcatacgagatanntnaccgtctcgtgggctcggagatgtgtataagagacag

SEQ ID NO: 1451 - DNA, 66 bp, Artificial
  synthetic
  misc_feature (26)..(27): n is a, c, g, or t
  misc_feature (29)..(29): n is a, c, g, or t
caagcagaagacggcatacgagatanngnaccgtctcgtgggctcggagatgtgtataagagacag

SEQ ID NO: 1452 - DNA, 66 bp, Artificial
  synthetic
  misc_feature (26)..(27): n is a, c, g, or t
  misc_feature (29)..(29): n is a, c, g, or t
caagcagaagacggcatacgagatannanaccgtctcgtgggctcggagatgtgtataagagacag

SEQ ID NO: 1453 - DNA, 66 bp, Artificial
  synthetic
  misc_feature (26)..(27): n is a, c, g, or t
caagcagaagacggcatacgagatcnntaaccgtctcgtgggctcggagatgtgtataagagacag

SEQ ID NO: 1454 - DNA, 66 bp, Artificial
  synthetic
  misc_feature (27)..(27): n is a, c, g, or t
caagcagaagacggcatacgagatccngaaccgtctcgtgggctcggagatgtgtataagagacag

SEQ ID NO: 1455 - DNA, 66 bp, Artificial
  synthetic
  misc_feature (26)..(27): n is a, c, g, or t
caagcagaagacggcatacgagattnngaaccgtctcgtgggctcggagatgtgtataagagacag

SEQ ID NO: 1456 - DNA, 66 bp, Artificial
  synthetic
  misc_feature (26)..(27): n is a, c, g, or t
caagcagaagacggcatacgagatgnngaaccgtctcgtgggctcggagatgtgtataagagacag

SEQ ID NO: 1457 - DNA, 66 bp, Artificial
  synthetic
  misc_feature (27)..(27): n is a, c, g, or t
caagcagaagacggcatacgagattgncaaccgtctcgtgggctcggagatgtgtataagagacag

SEQ ID NO: 1458 - DNA, 66 bp, Artificial
  synthetic
  misc_feature (27)..(27): n is a, c, g, or t
caagcagaagacggcatacgagatggncaaccgtctcgtgggctcggagatgtgtataagagacag

SEQ ID NO: 1459 - DNA, 66 bp, Artificial
  synthetic
  misc_feature (27)..(27): n is a, c, g, or t
caagcagaagacggcatacgagattcncaaccgtctcgtgggctcggagatgtgtataagagacag

SEQ ID NO: 1460 - DNA, 66 bp, Artificial
  synthetic
  misc_feature (27)..(27): n is a, c, g, or t
caagcagaagacggcatacgagatgcncaaccgtctcgtgggctcggagatgtgtataagagacag

SEQ ID NO: 1461 - DNA, 66 bp, Artificial
  synthetic
  misc_feature (26)..(27): n is a, c, g, or t
caagcagaagacggcatacgagatanncaaccgtctcgtgggctcggagatgtgtataagagacag

SEQ ID NO: 1462 - DNA, 66 bp, Artificial
  synthetic
  misc_feature (27)..(27): n is a, c, g, or t
caagcagaagacggcatacgagattancaaccgtctcgtgggctcggagatgtgtataagagacag

SEQ ID NO: 1463 - DNA, 66 bp, Artificial
  synthetic
  misc_feature (27)..(27): n is a, c, g, or t
caagcagaagacggcatacgagatgancaaccgtctcgtgggctcggagatgtgtataagagacag

SEQ ID NO: 1464 - DNA, 66 bp, Artificial
  synthetic
  misc_feature (27)..(27): n is a, c, g, or t
caagcagaagacggcatacgagatccnaaaccgtctcgtgggctcggagatgtgtataagagacag

SEQ ID NO: 1465 - DNA, 66 bp, Artificial
  synthetic
  misc_feature (26)..(27): n is a, c, g, or t
caagcagaagacggcatacgagattnnaaaccgtctcgtgggctcggagatgtgtataagagacag

SEQ ID NO: 1466 - DNA, 66 bp, Artificial
  synthetic
  misc_feature (26)..(27): n is a, c, g, or t
caagcagaagacggcatacgagatgnnaaaccgtctcgtgggctcggagatgtgtataagagacag

SEQ ID NO: 1467 - DNA, 66 bp, Artificial
  synthetic
  misc_feature (25)..(30): n is a, c, g, or t
caagcagaagacggcatacgagatnnnnnnacgtctcgtgggctcggagatgtgtataagagacag

SEQ ID NO: 1468 - DNA, 66 bp, Artificial
  synthetic
  misc_feature (25)..(30): n is a, c, g, or t
caagcagaagacggcatacgagatnnnnnntagtctcgtgggctcggagatgtgtataagagacag

SEQ ID NO: 1469 - DNA, 66 bp, Artificial
  synthetic
  misc_feature (25)..(30): n is a, c, g, or t
caagcagaagacggcatacgagatnnnnnngagtctcgtgggctcggagatgtgtataagagacag

SEQ ID NO: 1470 - DNA, 66 bp, Artificial
  synthetic
  misc_feature (25)..(29): n is a, c, g, or t
caagcagaagacggcatacgagatnnnnntcagtctcgtgggctcggagatgtgtataagagacag

SEQ ID NO: 1471 - DNA, 66 bp, Artificial
  synthetic
  misc_feature (26)..(27): n is a, c, g, or t
caagcagaagacggcatacgagatcnnctgcagtctcgtgggctcggagatgtgtataagagacag

SEQ ID NO: 1472 - DNA, 66 bp, Artificial
  synthetic
  misc_feature (25)..(27): n is a, c, g, or t
  misc_feature (29)..(29): n is a, c, g, or t
caagcagaagacggcatacgagatnnntngcagtctcgtgggctcggagatgtgtataagagacag

SEQ ID NO: 1473 - DNA, 66 bp, Artificial
  synthetic
  misc_feature (25)..(27): n is a, c, g, or t
  misc_feature (29)..(29): n is a, c, g, or t
caagcagaagacggcatacgagatnnngngcagtctcgtgggctcggagatgtgtataagagacag

SEQ ID NO: 1474 - DNA, 66 bp, Artificial
  synthetic
  misc_feature (26)..(27): n is a, c, g, or t
  misc_feature (29)..(29): n is a, c, g, or t
caagcagaagacggcatacgagattnncngcagtctcgtgggctcggagatgtgtataagagacag

SEQ ID NO: 1475 - DNA, 66 bp, Artificial
  synthetic
  misc_feature (26)..(27): n is a, c, g, or t
  misc_feature (29)..(29): n is a, c, g, or t
caagcagaagacggcatacgagatgnncngcagtctcgtgggctcggagatgtgtataagagacag

SEQ ID NO: 1476 - DNA, 66 bp, Artificial
  synthetic
  misc_feature (26)..(27): n is a, c, g, or t
  misc_feature (29)..(29): n is a, c, g, or t
caagcagaagacggcatacgagatanncngcagtctcgtgggctcggagatgtgtataagagacag

SEQ ID NO: 1477 - DNA, 66 bp, Artificial
  synthetic
  misc_feature (25)..(27): n is a, c, g, or t
  misc_feature (29)..(29): n is a, c, g, or t
caagcagaagacggcatacgagatnnnangcagtctcgtgggctcggagatgtgtataagagacag

SEQ ID NO: 1478 - DNA, 66 bp, Artificial
  synthetic
  misc_feature (26)..(27): n is a, c, g, or t
caagcagaagacggcatacgagatcnncagcagtctcgtgggctcggagatgtgtataagagacag

SEQ ID NO: 1479 - DNA, 66 bp, Artificial
  synthetic
  misc_feature (26)..(27): n is a, c, g, or t
caagcagaagacggcatacgagatcnngtccagtctcgtgggctcggagatgtgtataagagacag

SEQ ID NO: 1480 - DNA, 66 bp, Artificial
  synthetic
  misc_feature (26)..(27): n is a, c, g, or t
caagcagaagacggcatacgagatcnnctccagtctcgtgggctcggagatgtgtataagagacag

SEQ ID NO: 1481 - DNA, 66 bp, Artificial
  synthetic
  misc_feature (26)..(27): n is a, c, g, or t
caagcagaagacggcatacgagatcnnatccagtctcgtgggctcggagatgtgtataagagacag

SEQ ID NO: 1482 - DNA, 66 bp, Artificial
  synthetic
  misc_feature (26)..(27): n is a, c, g, or t
caagcagaagacggcatacgagatcnnggccagtctcgtgggctcggagatgtgtataagagacag

SEQ ID NO: 1483 - DNA, 66 bp, Artificial
  synthetic
  misc_feature (26)..(27): n is a, c, g, or t
caagcagaagacggcatacgagatcnnagccagtctcgtgggctcggagatgtgtataagagacag

SEQ ID NO: 1484 - DNA, 66 bp, Artificial
  synthetic
caagcagaagacggcatacgagatcttgcccagtctcgtgggctcggagatgtgtataagagacag

SEQ ID NO: 1485 - DNA, 66 bp, Artificial
  synthetic
caagcagaagacggcatacgagatctcgcccagtctcgtgggctcggagatgtgtataagagacag

SEQ ID NO: 1486 - DNA, 66 bp, Artificial
  synthetic
  misc_feature (27)..(27): n is a, c, g, or t
caagcagaagacggcatacgagatcgngcccagtctcgtgggctcggagatgtgtataagagacag

SEQ ID NO: 1487 - DNA, 66 bp, Artificial
  synthetic
  misc_feature (27)..(27): n is a, c, g, or t
caagcagaagacggcatacgagatccngcccagtctcgtgggctcggagatgtgtataagagacag

SEQ ID NO: 1488 - DNA, 66 bp, Artificial
  synthetic
  misc_feature (27)..(27): n is a, c, g, or t
caagcagaagacggcatacgagatcangcccagtctcgtgggctcggagatgtgtataagagacag

SEQ ID NO: 1489 - DNA, 66 bp, Artificial
  synthetic
caagcagaagacggcatacgagatctagcccagtctcgtgggctcggagatgtgtataagagacag

SEQ ID NO: 1490 - DNA, 66 bp, Artificial
  synthetic
caagcagaagacggcatacgagatcttacccagtctcgtgggctcggagatgtgtataagagacag

SEQ ID NO: 1491 - DNA, 66 bp, Artificial
  synthetic
caagcagaagacggcatacgagatctcacccagtctcgtgggctcggagatgtgtataagagacag

SEQ ID NO: 1492 - DNA, 66 bp, Artificial
  synthetic
  misc_feature (27)..(27): n is a, c, g, or t
caagcagaagacggcatacgagatcgnacccagtctcgtgggctcggagatgtgtataagagacag

SEQ ID NO: 1493 - DNA, 66 bp, Artificial
  synthetic
  misc_feature (27)..(27): n is a, c, g, or t
caagcagaagacggcatacgagatccnacccagtctcgtgggctcggagatgtgtataagagacag

SEQ ID NO: 1494 - DNA, 66 bp, Artificial
  synthetic
  misc_feature (27)..(27): n is a, c, g, or t
caagcagaagacggcatacgagatcanacccagtctcgtgggctcggagatgtgtataagagacag

SEQ ID NO: 1495 - DNA, 66 bp, Artificial
  synthetic
caagcagaagacggcatacgagatctaacccagtctcgtgggctcggagatgtgtataagagacag

SEQ ID NO: 1496 - DNA, 66 bp, Artificial
  synthetic
  misc_feature (25)..(27): n is a, c, g, or t
  misc_feature (29)..(29): n is a, c, g, or t
caagcagaagacggcatacgagatnnntnccagtctcgtgggctcggagatgtgtataagagacag

SEQ ID NO: 1497 - DNA, 66 bp, Artificial
  synthetic
  misc_feature (26)..(27): n is a, c, g, or t
  misc_feature (29)..(29): n is a, c, g, or t
caagcagaagacggcatacgagattnngnccagtctcgtgggctcggagatgtgtataagagacag

SEQ ID NO: 1498 - DNA, 66 bp, Artificial
  synthetic
  misc_feature (26)..(27): n is a, c, g, or t
  misc_feature (29)..(29): n is a, c, g, or t
caagcagaagacggcatacgagatgnngnccagtctcgtgggctcggagatgtgtataagagacag

SEQ ID NO: 1499 - DNA, 66 bp, Artificial
  synthetic
  misc_feature (26)..(27): n is a, c, g, or t
  misc_feature (29)..(29): n is a, c, g, or t
caagcagaagacggcatacgagatanngnccagtctcgtgggctcggagatgtgtataagagacag

SEQ ID NO: 1500 - DNA, 66 bp, Artificial
  synthetic
  misc_feature (26)..(27): n is a, c, g, or t
  misc_feature (29)..(29): n is a, c, g, or t
caagcagaagacggcatacgagattnncnccagtctcgtgggctcggagatgtgtataagagacag

SEQ ID NO: 1501 - DNA, 66 bp, Artificial
  synthetic
  misc_feature (26)..(27): n is a, c, g, or t
  misc_feature (29)..(29): n is a, c, g, or t
caagcagaagacggcatacgagatgnncnccagtctcgtgggctcggagatgtgtataagagacag

SEQ ID NO: 1502 - DNA, 66 bp, Artificial
  synthetic
  misc_feature (26)..(27): n is a, c, g, or t
  misc_feature (29)..(29): n is a, c, g, or t
caagcagaagacggcatacgagatanncnccagtctcgtgggctcggagatgtgtataagagacag

SEQ ID NO: 1503 - DNA, 66 bp, Artificial
  synthetic
  misc_feature (26)..(27): n is a, c, g, or t
  misc_feature (29)..(29): n is a, c, g, or t
caagcagaagacggcatacgagattnnanccagtctcgtgggctcggagatgtgtataagagacag

SEQ ID NO: 1504 - DNA, 66 bp, Artificial
  synthetic
  misc_feature (26)..(27): n is a, c, g, or t
  misc_feature (29)..(29): n is a, c, g, or t
caagcagaagacggcatacgagatgnnanccagtctcgtgggctcggagatgtgtataagagacag

SEQ ID NO: 1505 - DNA, 66 bp, Artificial
  synthetic
  misc_feature (26)..(27): n is a, c, g, or t
  misc_feature (29)..(29): n is a, c, g, or t
caagcagaagacggcatacgagatannanccagtctcgtgggctcggagatgtgtataagagacag

SEQ ID NO: 1506 - DNA, 66 bp, Artificial
  synthetic
  misc_feature (26)..(27): n is a, c, g, or t
caagcagaagacggcatacgagatcnngaccagtctcgtgggctcggagatgtgtataagagacag

SEQ ID NO: 1507 - DNA, 66 bp, Artificial
  synthetic
caagcagaagacggcatacgagatcttcaccagtctcgtgggctcggagatgtgtataagagacag

SEQ ID NO: 1508 - DNA, 66 bp, Artificial
  synthetic
caagcagaagacggcatacgagatctccaccagtctcgtgggctcggagatgtgtataagagacag

SEQ ID NO: 1509 - DNA, 66 bp, Artificial
  synthetic
  misc_feature (27)..(27): n is a, c, g, or t
caagcagaagacggcatacgagatcgncaccagtctcgtgggctcggagatgtgtataagagacag

SEQ ID NO: 1510 - DNA, 66 bp, Artificial
  synthetic
  misc_feature (27)..(27): n is a, c, g, or t
caagcagaagacggcatacgagatccncaccagtctcgtgggctcggagatgtgtataagagacag

SEQ ID NO: 1511 - DNA, 66 bp, Artificial
  synthetic
  misc_feature (27)..(27): n is a, c, g, or t
caagcagaagacggcatacgagatcancaccagtctcgtgggctcggagatgtgtataagagacag

SEQ ID NO: 1512 - DNA, 66 bp, Artificial
  synthetic
caagcagaagacggcatacgagatctacaccagtctcgtgggctcggagatgtgtataagagacag

SEQ ID NO: 1513 - DNA, 66 bp, Artificial
  synthetic
  misc_feature (26)..(27): n is a, c, g, or t
caagcagaagacggcatacgagatcnnaaccagtctcgtgggctcggagatgtgtataagagacag

SEQ ID NO: 1514 - DNA, 66 bp, Artificial
  synthetic
  misc_feature (25)..(29): n is a, c, g, or t
caagcagaagacggcatacgagatnnnnnacagtctcgtgggctcggagatgtgtataagagacag

SEQ ID NO: 1515 - DNA, 66 bp, Artificial
  synthetic
  misc_feature (25)..(30): n is a, c, g, or t
caagcagaagacggcatacgagatnnnnnnaagtctcgtgggctcggagatgtgtataagagacag